European Patent Application EP 4 741 507 A1, published May 13, 2026. Title: Modified Bacteria with Anti-tumor Activity and Improved Safety. Applicant: Shenzhen Synthetica Pioneering Co., Ltd. The sequence listing filed with the application follows.

SEQUENCE LISTING (483 sequences)

SEQ ID NO: 1 - DNA, 3977 bp, synthetic construct
  source 1..3977: mol_type = other DNA
ttcacagaaaagtgttgcccccttccatggcggaagggggacaaaggtgaatttgtcctactcaggagagcgttcaccgacaaacaacagataaaacgaaaggcccagtctttcgactgagcctttcgttttatttgatgcactagtgccgatcatattcaataacccttaatataacttcgtataatgtatgctatacgaagttattaggtctgaagaggagtttacgtcccatatggagtcccgctcagaagaactcgtcaagaaggcgatagaaggcgatgcgctgcgaatcgggagcggcgataccgtaaagcacgaggaagcggtcagcccattcgccgccaagctcttcagcaatatcacgggtagccaacgctatgtcctgatagcggtccgccacacccagccggccacagtcgatgaatccagaaaagcggccattttccaccatgatattcggcaagcaggcatcgccatgggtcacgacgagatcctcgccgtcgggcatgcgcgccttgagcctggcgaacagttcggccggcgcgagcccctgatgctcttcgtccagatcatcctgatcgacaagaccggcttccatccgagtacgtgctcgctcgatgcgatgtttcgcttggtggtcgaatgggcaggtagccggatcaagcgtatgcagccgccgcattgcatcagccatgatggatactttctcggcaggagcaaggtgagatgacaggagatcctgccccggcacttcgcccaatagcagccagtcccttcccgcttcagtgacaacgtcgagcacagctgcgcaaggaacgcccgtcgtggccagccacgatagccgcgctgcctcgtcctgcagttcattcagggcaccggacaggtcggtcttgacaaaaagaaccgggcgcccctgcgctgacagccggaacacggcggcatcagagcagccgattgtctgttgtgcccagtcatagccgaatagcctctccacccaagcggccggagaacctgcgtgcaatccatcttgttcaatcatgcgaaacgatcctcatcctgtctcttgatcagatcctgatcccctgcgccatcagatccttggcggcaagaaagccatccagtttactttgcagggcttcccaaccttaccagagggcgccccagctggcaattccgacgtcattgcgttgctagccaagcttaggatccggaacccttaatataacttcgtataatgtatgctatacgaagttattaggtccctcgaagaggttcactagctatctagagcttggactcctgttgatagatccagtaatgacctcagaactccatctggatttgttcagaacgctcggttgccgccgggcgttttttattggtgagaatccaagcccgggaaacgggatcctgatcttgatcaggctgtgggtcaggccactcttggcatcgacaccaatgtgggccttcatgccaaagtgccactgattgcctttcttggtctgatgcatctccggatcgcgttgctgctctttgttcttggtcgagctgggtgcctcaatgatggtggcatcgaccaaggtgccttgagtcatcatgacgcctgcttcggccagccagcgattgatggtcttgaacaattggcgggccagttgatgctgctccagcaggtggcggaaattcatgatggtggtgcggtccggcaaggcgctatccagggataaccgggcaaacagacgcatggaggcgatttcgtacagagcatcttccatcgcgccatcgctcaggttgtaccaatgctgcatgcagtgaatgcgtagcatggtttccagcggataaggtcgccggccattaccagccttggggtaaaacggctcgatgacttccaccatgttttgccatggcagaatctgctccatgcgggacaagaaaatctcttttctggtctgacggcgcttactgctgaattcactgtcggcgaaggtaagttgatgactcatgatgaaccctgttctatggctccagatgacaaacatgatctcatatcagggacttgttcgcaccttccttagcacgttaattatctatcgtgtatatggaggggatctagaatgaaaaaaataatgctagtttttattacacttatattagttagtctaccaattgcgcaacaaactgaagcaaaggatgcatctgcattcaataaagaaaattcaatttcatccatggcaccaccagcatctccgcctgcaagtcctaagacgccaatcgaaaagaaacacgcggatgaaatcgataagtatatacaaggattggactacaataaaaacaatgtattagtataccacggagatgcagtgacaaatgtgccgccaagaaaaggttacaaagatggaaatgaatatattgttgtggagaaaaagaagaaatccatcaatcaaaataatgcagacattcaagttgtgaatgcaatttcgagcctaacctatccaggtgctctcgtaaaagcgaattcggaattagtagaaaatcaaccagatgttctccctgtaaaacgtgattcattaacactcagcattgatttgccaggtatgactaatcaagacaataaaatcgttgtaaaaaatgccactaaatcaaacgttaacaacgcagtaaatacattagtggaaagatggaatgaaaaatatgctcaagcttatccaaatgtaagtgcaaaaattgattatgatgacgaaatggcttacagtgaatcacaattaattgcgaaatttggtacagcatttaaagctgtaaataatagcttgaatgtaaacttcggcgcaatcagtgaagggaaaatgcaagaagaagtcattagttttaaacaaatttactataacgtgaatgttaatgaacctacaagaccttccagatttttcggcaaagctgttactaaagagcagttgcaagcgcttggagtgaatgcagaaaatcctcctgcatatatctcaagtgtggcgtatggccgtcaagtttatttgaaattatcaactaattcccatagtactaaagtaaaagctgcttttgatgctgccgtaagcggaaaatctgtctcaggtgatgtagaactaacaaatatcatcaaaaattcttccttcaaagccgtaatttacggaggttccgcaaaagatgaagttcaaatcatcgacggcaacctcggagacttacgagatattttgaaaaaaggcgctacttttaatcgagaaacaccaggagttcccattgcttatacaacaaacttcctaaaagacaatgaattagctgttattaaaaacaactcagaatatattgaaacaacttcaaaagcttatacagatggaaaaattaacatcgatcactctggaggatacgttgctcaattcaacatttcttgggatgaagtaaattatgatcctgaaggtaacgaaattgttcaacataaaaactggagcgaaaacaataaaagtaagctagctcatttcacatcgtccatctatttgccaggtaacgcgagaaatattaatgtttacgctaaagaatgcactggtttagcttgggaatggtggagaacggtaattgatgaccggaacttaccacttgtgaaaaatagaaatatctccatctggggcaccacgctttatccgaaatatagtaataaagtagataatccaatcgaataagtcgacctcgaggactagtgaacctcttcgagggacctaataacttcgtatagcatacattatacgaagttatattaagggttattgaatatgatcggctcgagattacttcgcattgcaatcagctacggactcaagcttacgtcaggtcatacgatgaaggcgataagtcgcgtaagttgctagcccacgcggctcaccttcacgggtgggcctttcttcggtgtttcaatctcgattaacaggtaacgcaaaattgctgtgtacgtcaga

SEQ ID NO: 2 - DNA, 2716 bp, synthetic construct
  source 1..2716: mol_type = other DNA
ttggtttcagtgaatcccgttatcagcagttttttgatgaggtgtagtctatttgtcctactcaggagagcgttcaccgacaaacaacagataaaacgaaaggcccagtctttcgactgagcctttcgttttatttgatgcactagtgccgatcatattcaataacccttaatataacttcgtataatgtatgctatacgaagttattaggtctgaagaggagtttacgtcccatatggagtcccgcttacgccccgccctgccactcatcgcagtactgttgtaattcattaagcattctgccgacatggaagccatcacagacggcatgatgaacctgaatcgccagcggcatcagcaccttgtcgccttgcgtataatatttgcccatggtgaaaacgggggcgaagaagttgtccatattggccacgtttaaatcaaaactggtgaaactcacccagggattggctgagacgaaaaacatattctcaataaaccctttagggaaataggccaggttttcaccgtaacacgccacatcttgcgaatatatgtgtagaaactgccggaaatcgtcgtggtattcactccagagcgatgaaaacgtttcagtttgctcatggaaaacggtgtaacaagggtgaacactatcccatatcaccagctcaccgtctttcattgccatacgaaattccggatgagcattcatcaggcgggcaagaatgtgaataaaggccggataaaacttgtgcttatttttctttacggtctttaaaaaggccgtaatatccagctgaacggtctggttataggtacattgagcaactgactgaaatgcctcaaaatgttctttacgatgccattgggatatatcaacggtggtatatccagtgatttttttctccatgcgaaacgatcctcatcctgtctcttgatcagatcctgatcccctgcgccatcagatccttggcggcaagaaagccatccagtttactttgcagggcttcccaaccttaccagagggcgccccagctggcaattccgacgtcattgcgttgctagccaagcttaggatccggaacccttaatataacttcgtataatgtatgctatacgaagttattaggtccctcgaagaggttcactagctatctagagcttggactcctgttgatagatccagtaatgacctcagaactccatctggatttgttcagaacgctcggttgccgccgggcgttttttattggtgagaatccaagcccgggaaacgggatcctgatcttgatcaaccgaggtcacaacatagtaaaagcgctattggtaatggtacaatcgcgcgtttacacttattcagaacgatttttttcaggagggcctacttgtcacacaggacggtaatgtcgtgcccggttattgagctgacacagcaacttattcgtcgcccctccctgagtccggatgacgcaggctgtcaggcattaatgattgaacgcctgcgtaaaatcggttttaccattgagcatatggattttggcgacacgcaaaatttttgggcatggcgtgggcgtggcgaaacgctggcgttcgccgggcatactgacgtcgtaccggctggcgatgtcgatcgctggatcaatccgccgtttgagcctacgattcgcgacggaatgttgttcggtcgcggcgcggcggatatgaaaggttcactggcggccatggtggtggctgctgaacgttttgttgcgcagcatcctcatcaccggggccgcctcgcatttttgattacctctgatgaggaagccagcgcaaaaaatggcaccgtaaaggtggttgaagcgctgatggcccgtaacgagcggctggattactgtctggtcggcgaaccttccagtactgaaattgtgggcgatgtcgtcaaaaacgggcgtcgcggttctctcacctgtaacctcactatccatggcgttcaggggcacgtcgcctatccgcatctggcggataaccctgttcatcgcgccgcgccttttcttaatgaactggtcgctatcgagtgggatcggggcaatgactttttcccggccaccagtatgcaggtagccaatatccaggcaggcaccggcagcaataatgtcattcccggcgaactgttcgtgcagtttaacttccgtttcagcacggaactgaccgatgagatgatcaaagagcgggtacatgcgctgcttgaaaagcatcagctacgctataccgtagactggtggctttccgggcagccgttcctgaccgcacgcggcaagctggtggacgcggtggtaaacgccattgagcactataatgaaattaaaccgcaattactgacgacgggcggtacgtccgacggacgttttatcgcccgtatgggagcgcaggtggtagaactggggccggtgaacgccaccattcataaaattaatgaatgtgtgaatgccgccgatctccagctactggcccgtatgtatcaacgcattatggaacagctcgtcgcccatcaccatcaccatcactaagattacttcgcattgcaatcagctacggactcaagcttacgtcaggtcatacgatgaaggcgataagtcgcgtaagttgctagcccacgcggctcaccttcacgggtgggcctttcttcgtgagcgttccggtaagaggaaataagcatggactggctggcaaaatattg

SEQ ID NO: 3 - DNA, 6750 bp, synthetic construct
  source 1..6750: mol_type = other DNA
catggtcatagctgtttcctttaatgcccatggcgtttaccaatgcttaatcagtgaggcacctatctcagcgatctgtctatttcgttcatccatagttgcctgactccccgtcgtgtagataactacgatacgggagggcttaccatctggccccagtgctgcaatgataccgcgacttccacgctcaccggctccagatttatcagcaataaaccagccagccggaagggccgagcgcagaagtggtcctgcaactttatccgcctccatccagtctattaattgttgccgggaagctagagtaagtagttcgccagttaatagtttgcgcaacgttgttgccattgctacaggcatcgtggtgtcacgctcgtcgtttggtatggcttcattcagctccggttcccaacgatcaaggcgagttacatgatcccccatgttgtgcaaaaaagcggttagctccttcggtcctccgatcgttgtcagaagtaagttggccgcagtgttatcactcatggttatggcagcactgcataattctcttactgtcatgccatccgtaagatgcttttctgtgactggtgagtactcaaccaagtcattctgagaatagtgtatgcggcgaccgagttgctcttgcccggcgtcaatacgggataataccgcgccacatagcagaactttaaaagtgctcatcattggaaaacgttcttcggggcgaaaactctcaaggatcttaccgctgttgagatccagttcgatgtaacccactcgtgcacccaactgatcttcagcatcttttactttcaccagcgtttctgggtgagcaaaaacaggaaggcaaaatgccgcaaaaaagggaataagggcgacacggaaatgttgaatactcatactcttcctttttcaatattattgaagcatttatcagggttattgtctcatgagcggatacatatttgaatgtatttagaaaaataaacaaataggggttccgcgcacatttccccgaaaagtgccacctgacgtctaagaaaccattattatcatgacattaacctataaaaataggcgtatcacgaggcccttaggccaaataggccgttcagatccttccgtatttagccagtatgttctctagtgtggttcgttgtttttgcgtgagccatgagaacgaaccattgagatcatgcttactttgcatgtcactcaaaaattttgcctcaaaactggtgagctgaatttttgcagttaaagcatcgtgtagtgtttttcttagtccgttacgtaggtaggaatctgatgtaatggttgttggtattttgtcaccattcatttttatctggttgttctcaagttcggttacgagatccatttgtctatctagttcaacttggaaaatcaacgtatcagtcgggcggcctcgcttatcaaccaccaatttcatattgctgtaagtgtttaaatctttacttattggtttcaaaacccattggttaagccttttaaactcatggtagttattttcaagcattaacatgaacttaaattcatcaaggctaatctctatatttgccttgtgagttttcttttgtgttagttcttttaataaccactcataaatcctcatagagtatttgttttcaaaagacttaacatgttccagattatattttatgaatttttttaactggaaaagataaggcaatatctcttcactaaaaactaattctaatttttcgcttgagaacttggcatagtttgtccactggaaaatctcaaagcctttaaccaaaggattcctgatttccacagttctcgtcatcagctctctggttgctttagctaatacaccataagcattttccctactgatgttcatcatctgagcgtattggttataagtgaacgataccgtccgttctttccttgtagggttttcaatcgtggggttgagtagtgccacacagcataaaattagcttggtttcatgctccgttaagtcatagcgactaatcgctagttcatttgctttgaaaacaactaattcagacatacatctcaattggtctaggtgattttaatcactataccaattgagatgggctagtcaatgataattactagtccttttcctttgagttgtgggtatctgtaaattctgctagacctttgctggaaaacttgtaaattctgctagaccctctgtaaattccgctagacctttgtgtgttttttttgtttatattcaagtggttataatttatagaataaagaaagaataaaaaaagataaaaagaatagatcccagccctgtgtataactcactactttagtcagttccgcagtattacaaaaggatgtcgcaaacgctgtttgctcctctacaaaacagaccttaaaaccctaaaggcttaagtagcaccctcgcaagctcgggcaaatcgctgaatattccttttgtctccgaccatcaggcacctgagtcgctgtctttttcgtgacattcagttcgctgcgctcacggctctggcagtgaatgggggtaaatggcactacaggcgccttttatggattcatgcaaggaaactacccataatacaagaaaagcccgtcacgggcttctcagggcgttttatggcgggtctgctatgtggtgctatctgactttttgctgttcagcagttcctgccctctgattttccagtctgaccacttcggattatcccgtgacaggtcattcagactggctaatgcacccagtaaggcagcggtatcatcaacaggcttacccgtcttactgtcaagaggacatccggtcagataaccgtcatcttcggctactgtctagggcggcggatttgtcctactcaggagagcgttcaccgacaaacaacagataaaacgaaaggcccagtctttcgactgagcctttcgttttatttgatgcactagtgccgatcatattcaataacccttaatataacttcgtataatgtatgctatacgaagttattaggtctgaagaggagtttacgtcccatatggagtcccgctcagaagaactcgtcaagaaggcgatagaaggcgatgcgctgcgaatcgggagcggcgataccgtaaagcacgaggaagcggtcagcccattcgccgccaagctcttcagcaatatcacgggtagccaacgctatgtcctgatagcggtccgccacacccagccggccacagtcgatgaatccagaaaagcggccattttccaccatgatattcggcaagcaggcatcgccatgggtcacgacgagatcctcgccgtcgggcatgcgcgccttgagcctggcgaacagttcggccggcgcgagcccctgatgctcttcgtccagatcatcctgatcgacaagaccggcttccatccgagtacgtgctcgctcgatgcgatgtttcgcttggtggtcgaatgggcaggtagccggatcaagcgtatgcagccgccgcattgcatcagccatgatggatactttctcggcaggagcaaggtgagatgacaggagatcctgccccggcacttcgcccaatagcagccagtcccttcccgcttcagtgacaacgtcgagcacagctgcgcaaggaacgcccgtcgtggccagccacgatagccgcgctgcctcgtcctgcagttcattcagggcaccggacaggtcggtcttgacaaaaagaaccgggcgcccctgcgctgacagccggaacacggcggcatcagagcagccgattgtctgttgtgcccagtcatagccgaatagcctctccacccaagcggccggagaacctgcgtgcaatccatcttgttcaatcatgcgaaacgatcctcatcctgtctcttgatcagatcctgatcccctgcgccatcagatccttggcggcaagaaagccatccagtttactttgcagggcttcccaaccttaccagagggcgccccagctggcaattccgacgtcattgcgttgctagccaagcttaggatccggaacccttaatataacttcgtataatgtatgctatacgaagttattaggtccctcgaagaggttcactagctatctagagcttggactcctgttgatagatccagtaatgacctcagaactccatctggatttgttcagaacgctcggttgccgccgggcgttttttattggtgagaatccaagcccgggaaacgggatcctgatcttgatcaggctgtgggtcaggccactcttggcatcgacaccaatgtgggccttcatgccaaagtgccactgattgcctttcttggtctgatgcatctccggatcgcgttgctgctctttgttcttggtcgagctgggtgcctcaatgatggtggcatcgaccaaggtgccttgagtcatcatgacgcctgcttcggccagccagcgattgatggtcttgaacaattggcgggccagttgatgctgctccagcaggtggcggaaattcatgatggtggtgcggtccggcaaggcgctatccagggataaccgggcaaacagacgcatggaggcgatttcgtacagagcatcttccatcgcgccatcgctcaggttgtaccaatgctgcatgcagtgaatgcgtagcatggtttccagcggataaggtcgccggccattaccagccttggggtaaaacggctcgatgacttccaccatgttttgccatggcagaatctgctccatgcgggacaagaaaatctcttttctggtctgacggcgcttactgctgaattcactgtcggcgaaggtaagttgatgactcatgatgaaccctgttctatggctccagatgacaaacatgatctcatatcagggacttgttcgcaccttccttagcacgttaattatctatcgtgtatatggaggggatctagaatgaaaaaaataatgctagtttttattacacttatattagttagtctaccaattgcgcaacaaactgaagcaaaggatgcatctgcattcaataaagaaaattcaatttcatccatggcaccaccagcatctccgcctgcaagtcctaagacgccaatcgaaaagaaacacgcggatgaaatcgataagtatatacaaggattggactacaataaaaacaatgtattagtataccacggagatgcagtgacaaatgtgccgccaagaaaaggttacaaagatggaaatgaatatattgttgtggagaaaaagaagaaatccatcaatcaaaataatgcagacattcaagttgtgaatgcaatttcgagcctaacctatccaggtgctctcgtaaaagcgaattcggaattagtagaaaatcaaccagatgttctccctgtaaaacgtgattcattaacactcagcattgatttgccaggtatgactaatcaagacaataaaatcgttgtaaaaaatgccactaaatcaaacgttaacaacgcagtaaatacattagtggaaagatggaatgaaaaatatgctcaagcttatccaaatgtaagtgcaaaaattgattatgatgacgaaatggcttacagtgaatcacaattaattgcgaaatttggtacagcatttaaagctgtaaataatagcttgaatgtaaacttcggcgcaatcagtgaagggaaaatgcaagaagaagtcattagttttaaacaaatttactataacgtgaatgttaatgaacctacaagaccttccagatttttcggcaaagctgttactaaagagcagttgcaagcgcttggagtgaatgcagaaaatcctcctgcatatatctcaagtgtggcgtatggccgtcaagtttatttgaaattatcaactaattcccatagtactaaagtaaaagctgcttttgatgctgccgtaagcggaaaatctgtctcaggtgatgtagaactaacaaatatcatcaaaaattcttccttcaaagccgtaatttacggaggttccgcaaaagatgaagttcaaatcatcgacggcaacctcggagacttacgagatattttgaaaaaaggcgctacttttaatcgagaaacaccaggagttcccattgcttatacaacaaacttcctaaaagacaatgaattagctgttattaaaaacaactcagaatatattgaaacaacttcaaaagcttatacagatggaaaaattaacatcgatcactctggaggatacgttgctcaattcaacatttcttgggatgaagtaaattatgatcctgaaggtaacgaaattgttcaacataaaaactggagcgaaaacaataaaagtaagctagctcatttcacatcgtccatctatttgccaggtaacgcgagaaatattaatgtttacgctaaagaatgcactggtttagcttgggaatggtggagaacggtaattgatgaccggaacttaccacttgtgaaaaatagaaatatctccatctggggcaccacgctttatccgaaatatagtaataaagtagataatccaatcgaataagtcgacctcgaggactagtgaacctcttcgagggacctaataacttcgtatagcatacattatacgaagttatattaagggttattgaatatgatcggctcgagattacttcgcattgcaatcagctacggactcaagcttacgtcaggtcatacgatgaaggcgataagtcgcgtaagttgctagcccacgcggctcaccttcacgggtgggcctttcttcgcgatccacatg

SEQ ID NO: 4 - DNA, 5456 bp, synthetic construct
  source 1..5456: mol_type = other DNA
catggtcatagctgtttcctttaatgcccatggcgtttaccaatgcttaatcagtgaggcacctatctcagcgatctgtctatttcgttcatccatagttgcctgactccccgtcgtgtagataactacgatacgggagggcttaccatctggccccagtgctgcaatgataccgcgacttccacgctcaccggctccagatttatcagcaataaaccagccagccggaagggccgagcgcagaagtggtcctgcaactttatccgcctccatccagtctattaattgttgccgggaagctagagtaagtagttcgccagttaatagtttgcgcaacgttgttgccattgctacaggcatcgtggtgtcacgctcgtcgtttggtatggcttcattcagctccggttcccaacgatcaaggcgagttacatgatcccccatgttgtgcaaaaaagcggttagctccttcggtcctccgatcgttgtcagaagtaagttggccgcagtgttatcactcatggttatggcagcactgcataattctcttactgtcatgccatccgtaagatgcttttctgtgactggtgagtactcaaccaagtcattctgagaatagtgtatgcggcgaccgagttgctcttgcccggcgtcaatacgggataataccgcgccacatagcagaactttaaaagtgctcatcattggaaaacgttcttcggggcgaaaactctcaaggatcttaccgctgttgagatccagttcgatgtaacccactcgtgcacccaactgatcttcagcatcttttactttcaccagcgtttctgggtgagcaaaaacaggaaggcaaaatgccgcaaaaaagggaataagggcgacacggaaatgttgaatactcatactcttcctttttcaatattattgaagcatttatcagggttattgtctcatgagcggatacatatttgaatgtatttagaaaaataaacaaataggggttccgcgcacatttccccgaaaagtgccacctgacgtctaagaaaccattattatcatgacattaacctataaaaataggcgtatcacgaggcccttaggccaaataggccgttcagatccttccgtatttagccagtatgttctctagtgtggttcgttgtttttgcgtgagccatgagaacgaaccattgagatcatgcttactttgcatgtcactcaaaaattttgcctcaaaactggtgagctgaatttttgcagttaaagcatcgtgtagtgtttttcttagtccgttacgtaggtaggaatctgatgtaatggttgttggtattttgtcaccattcatttttatctggttgttctcaagttcggttacgagatccatttgtctatctagttcaacttggaaaatcaacgtatcagtcgggcggcctcgcttatcaaccaccaatttcatattgctgtaagtgtttaaatctttacttattggtttcaaaacccattggttaagccttttaaactcatggtagttattttcaagcattaacatgaacttaaattcatcaaggctaatctctatatttgccttgtgagttttcttttgtgttagttcttttaataaccactcataaatcctcatagagtatttgttttcaaaagacttaacatgttccagattatattttatgaatttttttaactggaaaagataaggcaatatctcttcactaaaaactaattctaatttttcgcttgagaacttggcatagtttgtccactggaaaatctcaaagcctttaaccaaaggattcctgatttccacagttctcgtcatcagctctctggttgctttagctaatacaccataagcattttccctactgatgttcatcatctgagcgtattggttataagtgaacgataccgtccgttctttccttgtagggttttcaatcgtggggttgagtagtgccacacagcataaaattagcttggtttcatgctccgttaagtcatagcgactaatcgctagttcatttgctttgaaaacaactaattcagacatacatctcaattggtctaggtgattttaatcactataccaattgagatgggctagtcaatgataattactagtccttttcctttgagttgtgggtatctgtaaattctgctagacctttgctggaaaacttgtaaattctgctagaccctctgtaaattccgctagacctttgtgtgttttttttgtttatattcaagtggttataatttatagaataaagaaagaataaaaaaagataaaaagaatagatcccagccctgtgtataactcactactttagtcagttccgcagtattacaaaaggatgtcgcaaacgctgtttgctcctctacaaaacagaccttaaaaccctaaaggcttaagtagcaccctcgcaagctcgggcaaatcgctgaatattccttttgtctccgaccatcaggcacctgagtcgctgtctttttcgtgacattcagttcgctgcgctcacggctctggcagtgaatgggggtaaatggcactacaggcgccttttatggattcatgcaaggaaactacccataatacaagaaaagcccgtcacgggcttctcagggcgttttatggcgggtctgctatgtggtgctatctgactttttgctgttcagcagttcctgccctctgattttccagtctgaccacttcggattatcccgtgacaggtcattcagactggctaatgcacccagtaaggcagcggtatcatcaacaggcttacccgtcttactgtcaagaggacatccggtcagataaccgtcatcttcggctactgtctagggcggcggatttgtcctactcaggagagcgttcaccgacaaacaacagataaaacgaaaggcccagtctttcgactgagcctttcgttttatttgatgcactagtgccgatcatattcaataacccttaatataacttcgtataatgtatgctatacgaagttattaggtctgaagaggagtttacgtcccatatggagtcccgcttacgccccgccctgccactcatcgcagtactgttgtaattcattaagcattctgccgacatggaagccatcacagacggcatgatgaacctgaatcgccagcggcatcagcaccttgtcgccttgcgtataatatttgcccatggtgaaaacgggggcgaagaagttgtccatattggccacgtttaaatcaaaactggtgaaactcacccagggattggctgagacgaaaaacatattctcaataaaccctttagggaaataggccaggttttcaccgtaacacgccacatcttgcgaatatatgtgtagaaactgccggaaatcgtcgtggtattcactccagagcgatgaaaacgtttcagtttgctcatggaaaacggtgtaacaagggtgaacactatcccatatcaccagctcaccgtctttcattgccatacgaaattccggatgagcattcatcaggcgggcaagaatgtgaataaaggccggataaaacttgtgcttatttttctttacggtctttaaaaaggccgtaatatccagctgaacggtctggttataggtacattgagcaactgactgaaatgcctcaaaatgttctttacgatgccattgggatatatcaacggtggtatatccagtgatttttttctccattttagcttccttagctcctgaaaatctcgataactcaaaaaatacgcccggtagtgatcttatttcattatggtgaaagttggaacctcttacgtgccgatcagacgtcattgcgttgctagccaagcttaggatccggaacccttaatataacttcgtataatgtatgctatacgaagttattaggtccctcgaagaggttcactagctatctagagcttggactcctgttgatagatccagtaatgacctcagaactccatctggatttgttcagaacgctcggttgccgccgggcgttttttattggtgagaatccaagcccgggaaacgggatcctgatcttgatcaaccgaggtcacaacatagtaaaagcgctattggtaatggtacaatcgcgcgtttacacttattcagaacgatttttttcaggagggcctacttgtcacacaggacggtaatgtcgtgcccggttattgagctgacacagcaacttattcgtcgcccctccctgagtccggatgacgcaggctgtcaggcattaatgattgaacgcctgcgtaaaatcggttttaccattgagcatatggattttggcgacacgcaaaatttttgggcatggcgtgggcgtggcgaaacgctggcgttcgccgggcatactgacgtcgtaccggctggcgatgtcgatcgctggatcaatccgccgtttgagcctacgattcgcgacggaatgttgttcggtcgcggcgcggcggatatgaaaggttcactggcggccatggtggtggctgctgaacgttttgttgcgcagcatcctcatcaccggggccgcctcgcatttttgattacctctgatgaggaagccagcgcaaaaaatggcaccgtaaaggtggttgaagcgctgatggcccgtaacgagcggctggattactgtctggtcggcgaaccttccagtactgaaattgtgggcgatgtcgtcaaaaacgggcgtcgcggttctctcacctgtaacctcactatccatggcgttcaggggcacgtcgcctatccgcatctggcggataaccctgttcatcgcgccgcgccttttcttaatgaactggtcgctatcgagtgggatcggggcaatgactttttcccggccaccagtatgcaggtagccaatatccaggcaggcaccggcagcaataatgtcattcccggcgaactgttcgtgcagtttaacttccgtttcagcacggaactgaccgatgagatgatcaaagagcgggtacatgcgctgcttgaaaagcatcagctacgctataccgtagactggtggctttccgggcagccgttcctgaccgcacgcggcaagctggtggacgcggtggtaaacgccattgagcactataatgaaattaaaccgcaattactgacgacgggcggtacgtccgacggacgttttatcgcccgtatgggagcgcaggtggtagaactggggccggtgaacgccaccattcataaaattaatgaatgtgtgaatgccgccgatctccagctactggcccgtatgtatcaacgcattatggaacagctcgtcgcccatcaccatcaccatcactaagattacttcgcattgcaatcagctacggactcaagcttacgtcaggtcatacgatgaaggcgataagtcgcgtaagttgctagcccacgcggctcaccttcacgggtgggcctttcttcgcgatccacatg

SEQ ID NO: 5 - DNA, 76 bp, synthetic construct
  source 1..76: mol_type = other DNA
ttcacagaaaagtgttgcccccttccatggcggaagggggacaaaggtgaatttgtcctactcaggagagcgttca

SEQ ID NO: 6 - DNA, 68 bp, synthetic construct
  source 1..68: mol_type = other DNA
tctgacgtacacagcaattttgcgttacctgttaatcgagattgaaacaccgaagaaaggcccacccg

SEQ ID NO: 7 - DNA, 72 bp, synthetic construct
  source 1..72: mol_type = other DNA
ttggtttcagtgaatcccgttatcagcagttttttgatgaggtgtagtctatttgtcctactcaggagagcg

SEQ ID NO: 8 - DNA, 68 bp, synthetic construct
  source 1..68: mol_type = other DNA
caatattttgccagccagtccatgcttatttcctcttaccggaacgctcacgaagaaaggcccacccg

SEQ ID NO: 9 - DNA, 85 bp, synthetic construct
  source 1..85: mol_type = other DNA
gcaggggtaaaagtgacctgacgcaatatttgtcttttcttgcttcttaataatgttgtcacaaaaagtgagggtgactacatgg

SEQ ID NO: 10 - DNA, 85 bp, synthetic construct
  source 1..85: mol_type = other DNA
cgccgcaaagtttgagcgaagtcaataaactctctacccattcagggcaatatctctcttgcaggtgaatgcaacgtcaagcgat

SEQ ID NO: 11 - DNA, 85 bp, synthetic construct
  source 1..85: mol_type = other DNA
tcagaagaagcaaaaagacactttaccgaagggtttaacattttttcgtgatactcatcaccatgacgcaaatgcgttgcataaa

SEQ ID NO: 12 - DNA, 85 bp, synthetic construct
  source 1..85: mol_type = other DNA
aaccgaggtcacaacatagtaaaagcgctattggtaatggtacaatcgcgcgtttacacttattcagaacgatttttttcaggag

SEQ ID NO: 13 - DNA, 54 bp, synthetic construct
  source 1..54: mol_type = other DNA
ggataaaagtgacctgacgcaatatttgtcttttcttgcttaataatgttgtca

SEQ ID NO: 14 - DNA, 35 bp, synthetic construct
  source 1..35: mol_type = other DNA
tgtaagtttatacataggcgagtactctgttatgg

SEQ ID NO: 15 - DNA, 74 bp, synthetic construct
  source 1..74: mol_type = other DNA
ttaaatttcctctcgtcaggccggaataactccctataatgcgccaccacactgatagtgctagtgtagatcac

SEQ ID NO: 16 - DNA, 58 bp, synthetic construct
  source 1..58: mol_type = other DNA
aaaattgatctgaatcaatattttgacaaaaattgatctgaatcaatatttactgagc

SEQ ID NO: 17 - DNA, 44 bp, synthetic construct
  source 1..44: mol_type = other DNA
gttaataaaatgttattgacagttaataaaatgttatactgagc

SEQ ID NO: 18 - DNA, 30 bp, synthetic construct
  source 1..30: mol_type = other DNA
ttagcacgttaattatctatcgtgtatatg

SEQ ID NO: 19 - DNA, 1128 bp, synthetic construct
  source 1..1128: mol_type = other DNA
atgtcgtgcccggttattgagctgacacagcaacttattcgtcgcccctccctgagtccggatgacgcaggctgtcaggcattaatgattgaacgcctgcgtaaaatcggttttaccattgagcatatggattttggcgacacgcaaaatttttgggcatggcgtgggcgtggcgaaacgctggcgttcgccgggcatactgacgtcgtaccggctggcgatgtcgatcgctggatcaatccgccgtttgagcctacgattcgcgacggaatgttgttcggtcgcggcgcggcggatatgaaaggttcactggcggccatggtggtggctgctgaacgttttgttgcgcagcatcctcatcaccggggccgcctcgcatttttgattacctctgatgaggaagccagcgcaaaaaatggcaccgtaaaggtggttgaagcgctgatggcccgtaacgagcggctggattactgtctggtcggcgaaccttccagtactgaaattgtgggcgatgtcgtcaaaaacgggcgtcgcggttctctcacctgtaacctcactatccatggcgttcaggggcacgtcgcctatccgcatctggcggataaccctgttcatcgcgccgcgccttttcttaatgaactggtcgctatcgagtgggatcggggcaatgactttttcccggccaccagtatgcaggtagccaatatccaggcaggcaccggcagcaataatgtcattcccggcgaactgttcgtgcagtttaacttccgtttcagcacggaactgaccgatgagatgatcaaagagcgggtacatgcgctgcttgaaaagcatcagctacgctataccgtagactggtggctttccgggcagccgttcctgaccgcacgcggcaagctggtggacgcggtggtaaacgccattgagcactataatgaaattaaaccgcaattactgacgacgggcggtacgtccgacggacgttttatcgcccgtatgggagcgcaggtggtagaactggggccggtgaacgccaccattcataaaattaatgaatgtgtgaatgccgccgatctccagctactggcccgtatgtatcaacgcattatggaacagctcgtcgcctga

SEQ ID NO: 20 - DNA, 1428 bp, synthetic construct
  source 1..1428: mol_type = other DNA
atgaaaaaaaccacattagcaatgagtgcactggctctgagtttaggtttggcattgtcgcctctgtctgccacggcggctgaaacgtcctcttcagcaatgactgcccagcagatgccaagcctggcaccgatgctcgaaaaagtgatgccatcggtggtcagtattaatgttgaaggtagcaccacggtgaatacgccgcgtatgccgcgtaatttccagcagttctttggcgatgactccccgttctgccaggacggttctccgttccagaattctccgttctgccagggcggcggtaacggcggcaacggcggtcaacaacagaaattcatggcgctgggctccggcgtaattattgacgccgcgaagggctacgtcgtcaccaacaaccacgtggttgataacgccagcgtgattaaagtacagcttagcgatgggcgtaaattcgatgctaaagtggtgggcaaagatccgcgttctgatatcgcgctgattcaaattcagaatccgaagaacctgacggcgattaagctggcggactccgacgcgctgcgcgtgggggattataccgtcgctattggtaacccgtttggtctgggcgaaacggtgacgtcaggtatcgtttcggcgctggggcgtagcggcctgaacgtagaaaattacgagaactttattcagaccgacgccgcgattaaccgtggtaactccggcggcgcgctggtgaacctgaacggtgagctgatcggtattaacaccgcgattctggcgccggacggcggcaacatcggtatcggcttcgctatccccagtaacatggtgaaaaacctgacgtcgcagatggtggaatacggccaggtgaaacgcggcgaactggggatcatggggactgagctgaattccgaattggcgaaagcgatgaaagtcgacgcccagcgaggcgcgttcgtcagccaggtgatgccgaattcgtccgcggcgaaagcgggtatcaaagccggggatgtcattacctcgctgaacggtaaaccgatcagcagctttgcggcgctgcgcgctcaggtcggcactatgccggtcggcagcaaaatcagcctcggtctgctgcgtgaaggtaaagcgattacggtgaatctggaactgcagcagagcagccagagtcaggttgattccagcaccatcttcagcgggattgaaggcgctgaaatgagcaataaaggccaggataaaggcgttgtggtgagcagcgtgaaagcgaactcacccgccgcgcaaattggcctcaaaaaaggcgatgtgattatcggcgctaaccagcagccggtgaaaaatatcgccgagctgcgtaagattctcgacagcaagccgtcggttctggcgctgaatattcagcgtggtgatagttctatttatttgctgatgcagtaa

SEQ ID NO: 21 - DNA, 1590 bp, synthetic construct
  source 1..1590: mol_type = other DNA
atgaaaaaaataatgctagtttttattacacttatattagttagtctaccaattgcgcaacaaactgaagcaaaggatgcatctgcattcaataaagaaaattcaatttcatccatggcaccaccagcatctccgcctgcaagtcctaagacgccaatcgaaaagaaacacgcggatgaaatcgataagtatatacaaggattggactacaataaaaacaatgtattagtataccacggagatgcagtgacaaatgtgccgccaagaaaaggttacaaagatggaaatgaatatattgttgtggagaaaaagaagaaatccatcaatcaaaataatgcagacattcaagttgtgaatgcaatttcgagcctaacctatccaggtgctctcgtaaaagcgaattcggaattagtagaaaatcaaccagatgttctccctgtaaaacgtgattcattaacactcagcattgatttgccaggtatgactaatcaagacaataaaatcgttgtaaaaaatgccactaaatcaaacgttaacaacgcagtaaatacattagtggaaagatggaatgaaaaatatgctcaagcttatccaaatgtaagtgcaaaaattgattatgatgacgaaatggcttacagtgaatcacaattaattgcgaaatttggtacagcatttaaagctgtaaataatagcttgaatgtaaacttcggcgcaatcagtgaagggaaaatgcaagaagaagtcattagttttaaacaaatttactataacgtgaatgttaatgaacctacaagaccttccagatttttcggcaaagctgttactaaagagcagttgcaagcgcttggagtgaatgcagaaaatcctcctgcatatatctcaagtgtggcgtatggccgtcaagtttatttgaaattatcaactaattcccatagtactaaagtaaaagctgcttttgatgctgccgtaagcggaaaatctgtctcaggtgatgtagaactaacaaatatcatcaaaaattcttccttcaaagccgtaatttacggaggttccgcaaaagatgaagttcaaatcatcgacggcaacctcggagacttacgagatattttgaaaaaaggcgctacttttaatcgagaaacaccaggagttcccattgcttatacaacaaacttcctaaaagacaatgaattagctgttattaaaaacaactcagaatatattgaaacaacttcaaaagcttatacagatggaaaaattaacatcgatcactctggaggatacgttgctcaattcaacatttcttgggatgaagtaaattatgatcctgaaggtaacgaaattgttcaacataaaaactggagcgaaaacaataaaagtaagctagctcatttcacatcgtccatctatttgccaggtaacgcgagaaatattaatgtttacgctaaagaatgcactggtttagcttgggaatggtggagaacggtaattgatgaccggaacttaccacttgtgaaaaatagaaatatctccatctggggcaccacgctttatccgaaatatagtaataaagtagataatccaatcgaataa

SEQ ID NO: 22 - DNA, 2118 bp, synthetic construct
  source 1..2118: mol_type = other DNA
tcgagttcatgtgcagctccatcagcaaaaggggatgataagtttatcaccaccgactatttgcaacagtgccgttgatcgtgctatgatcgactgatgtcatcagcggtggagtgcaatgtcatgagggaagcggtgatcgccgaagtatcgactcaactatcagaggtagttggcgtcatcgagcgccatctcgaaccgacgttgctggccgtacatttgtacggctccgcagtggatggcggcctgaagccacacagtgatattgatttgctggttacggtgaccgtaaggcttgatgaaacaacgcggcgagctttgatcaacgaccttttggaaacttcggcttcccctggagagagcgagattctccgcgctgtagaagtcaccattgttgtgcacgacgacatcattccgtggcgttatccagctaagcgcgaactgcaatttggagaatggcagcgcaatgacattcttgcaggtatcttcgagccagccacgatcgacattgatctggctatcttgctgacaaaagcaagagaacatagcgttgccttggtaggtccagcggcggaggaactctttgatccggttcctgaacaggatctatttgaggcgctaaatgaaaccttaacgctatggaactcgccgcccgactgggctggcgatgagcgaaatgtagtgcttacgttgtcccgcatttggtacagcgcagtaaccggcaaaatcgcgccgaaggatgtcgctgccgactgggcaatggagcgcctgccggcccagtatcagcccgtcatacttgaagctagacaggcttatcttggacaagaagaagatcgcttggcctcgcgcgcagatcagttggaagaatttgtccactacgtgaaaggcgagatcaccaaggtagtcggcaaataagatgccgctcgccagtcgattggctgagctcatgaagttcctattccgaagttccgcgaacgcgtaaaggatctaggtgaagatcctttttgataatctcatgaccaaaatcccttaacgtgagttttcgttccactgagcgtcagaccccgtagaaaagatcaaaggatcttcttgagatcctttttttctgcgcgtaatctgctgcttgcaaacaaaaaaaccaccgctaccagcggtggtttgtttgccggatcaagagctaccaactctttttccgaaggtaactggcttcagcagagcgcagataccaaatactgtccttctagtgtagccgtagttaggccaccacttcaagaactctgtagcaccgcctacatacctcgctctgctaatcctgttaccagtggctgctgccagtggcgataagtcgtgtcttaccgggttggactcaagacgatagttaccggataaggcgcagcggtcgggctgaacggggggttcgtgcacacagcccagcttggagcgaacgacctacaccgaactgagatacctacagcgtgagctatgagaaagcgccacgcttcccgaagggagaaaggcggacaggtatccggtaagcggcagggtcggaacaggagagcgcacgagggagcttccagggggaaacgcctggtatctttatagtcctgtcgggtttcgccacctctgacttgagcgtcgatttttgtgatgctcgtcaggggggcggagcctatggaaaaacgccagcaacgcggcctttttacggttcctggccttttgctggccttttgctcacatgttctttcctgcgttatcccctgattctgtggataaccgtattaccgcctttgagtgagctgataccgctcgccgcagccgaacgaccgagcgcagcgagtcagtgagcgaggaagcggaagagcgcctgatgcggtattttctccttacgcatctgtgcggtatttcacaccgcatatgctggatccttgacagctagctcagtcctaggtataatactagtcatcgccgcagcggtttcaggttttagagctagaaatagcaagttaaaataaggctagtccgttatcaacttgaaaaagtggcaccgagtcggtgctttttttgaattctctagagtcgacctgcagaagcttagatctattaccctgttatccctac

SEQ ID NO: 23 - DNA, 3212 bp, synthetic construct
  source 1..3212: mol_type = other DNA
gacgtctgtgtggaattgtgagcgtcatgtccgagtctgcaatgcttcgatcaaaaaacccctcaagacccgtttagaggccccaaggggttatgctaggctagctagagcggtacccctccctatcagtgatagagattgacatccctatcagtgatagagatactgagcacatatgcagcaggacgcactgaccgaattcattaaagaggagaaaggtaccatgtctagattagataaaagtaaagtgattaacagcgcattagagctgcttaatgaggtcggaatcgaaggtttaacaacccgtaaactcgcccagaagctaggtgtagagcagcctacattgtattggcatgtaaaaaataagcgggctttgctcgacgccttagccattgagatgttagataggcaccatactcacttttgccctttagaaggggaaagctggcaagattttttacgtaataacgctaaaagttttagatgtgctttactaagtcatcgcgatggagcaaaagtacatttaggtacacggcctacagaaaaacagtatgaaactctcgaaaatcaattagcctttttatgccaacaaggtttttcactagagaatgcattatatgcactcagcgctgtggggcattttactttaggttgcgtattggaagatcaagagcatcaagtcgctaaagaagaaagggaaacacctactactgatagtatgccgccattattacgacaagctatcgaattatttgatcaccaaggtgcagagccagccttcttattcggccttgaattgatcatatgcggattagaaaaacaacttaaatgtgaaagtgggtcttaactgcagccatgggctagcgtcgaccttaagtctagagaaagaagagactcggcgcgccatgagcgaagcacttaaaattctgaacaacatccgtactcttcgtgcgcaggcaagagaatgtactctggaaacgcttgaagaaatgctggaaaaattagaagttgtcgttaatgagcgtcgtgaagaagaaagcgctgctgctgctgaagtggaagaacgcactcgtaaactgcaacagtatcgtgaaatgttaattgccgacggcattgacccgaatgaactgctgaatagcatggctgccgctaaatccggtaccaaagctaaacgcgcagctcgtccggctaaatatagctatgttgacgaaaacggtgaaactaaaacctggactggccagggtcgtacaccggctgtaatcaaaaaagcaatggaagaacaaggtaagcaactggaagatttcctgatcaaggaataaggatccggctcaccttcacgggtgggcctttcttcgcggtatcagctcactcaaaggcggtaatacggttatccacagaatcaggggataacgcaggaaagaacatgtgagcaaaaggccagcaaaaggccaggaaccgtaaaaaggccgcgttgctggcgtttttccataggctccgcccccctgacgagcatcacaaaaatcgacgctcaagtcagaggtggcgaaacccgacaggactataaagataccaggcgtttccccctggaagctccctcgtgcgctctcctgttccgaccctgccgcttaccggatacctgtccgcctttctcccttcgggaagcgtggcgctttctcaatgctcacgctgtaggtatctcagttcggtgtaggtcgttcgctccaagctgggctgtgtgcacgaaccccccgttcagcccgaccgctgcgccttatccggtaactatcgtcttgagtccaacccggtaagacacgacttatcgccactggcagcagccactggtaacaggattagcagagcgaggtatgtaggcggtgctacagagttcttgaagtggtggcctaactacggctacactagaaggacagtatttggtatctgcgctctgctgaagccagttaccttcggaaaaagagttggtagctcttgatccggcaaacaaaccaccgctggtagcggtggtttttttgtttgcaagcagcagattacgcgcagaaaaaaaggatctcaagaagatcctttgatcttttctacggggtctgacgctcagtggaacgaaaactcacgttaagggattttggtcatgactagtgcttggattctcaccaataaaaaacgcccggcggcaaccgagcgttctgaacaaatccagatggagttctgaggtcattactggatctatcaacaggagtccaagcgagctcgatatcaaacttatttgccgactaccttggtgatctcgcctttcacgtagtggacaaattcttccaactgatctgcgcgcgaggccaagcgatcttcttcttgtccaagataagcctgtctagcttcaagtatgacgggctgatactgggccggcaggcgctccattgcccagtcggcagcgacatccttcggcgcgattttgccggttactgcgctgtaccaaatgcgggacaacgtaagcactacatttcgctcatcgccagcccagtcgggcggcgagttccatagcgttaaggtttcatttagcgcctcaaatagatcctgttcaggaaccggatcaaagagttcctccgccgctggacctaccaaggcaacgctatgttctcttgcttttgtcagcaagatagccagatcaatgtcgatcgtggctggctcgaagatacctgcaagaatgtcattgcgctgccattctccaaattgcagttcgcgcttagctggataacgccacggaatgatgtcgtcgtgcacaacaatggtgacttctacagcgcggagaatctcgctctctccaggggaagccgaagtttccaaaaggtcgttgatcaaagctcgccgcgttgtttcatcaagccttacggtcaccgtaaccagcaaatcaatatcactgtgtggcttcaggccgccatccactgcggagccgtacaaatgtacggccagcaacgtcggttcgagatggcgctcgatgacgccaactacctctgatagttgagtcgatacttcggcgatcaccgcttccctcatgacattgcactccaccgctgatgacatcagtcgatcatagcacgatcaacggcactgttgcaaatagtcggtggtgataaacttatcatccccttttgctgatggagctgcacatgaactcgaacgtctcattttcgccagatatc

SEQ ID NO: 24 - DNA, 5587 bp, synthetic construct
  source 1..5587: mol_type = other DNA
atggtcatagctgtttcctttaatgcccatggcgtttaccaatgcttaatcagtgaggcacctatctcagcgatctgtctatttcgttcatccatagttgcctgactccccgtcgtgtagataactacgatacgggagggcttaccatctggccccagtgctgcaatgataccgcgacttccacgctcaccggctccagatttatcagcaataaaccagccagccggaagggccgagcgcagaagtggtcctgcaactttatccgcctccatccagtctattaattgttgccgggaagctagagtaagtagttcgccagttaatagtttgcgcaacgttgttgccattgctacaggcatcgtggtgtcacgctcgtcgtttggtatggcttcattcagctccggttcccaacgatcaaggcgagttacatgatcccccatgttgtgcaaaaaagcggttagctccttcggtcctccgatcgttgtcagaagtaagttggccgcagtgttatcactcatggttatggcagcactgcataattctcttactgtcatgccatccgtaagatgcttttctgtgactggtgagtactcaaccaagtcattctgagaatagtgtatgcggcgaccgagttgctcttgcccggcgtcaatacgggataataccgcgccacatagcagaactttaaaagtgctcatcattggaaaacgttcttcggggcgaaaactctcaaggatcttaccgctgttgagatccagttcgatgtaacccactcgtgcacccaactgatcttcagcatcttttactttcaccagcgtttctgggtgagcaaaaacaggaaggcaaaatgccgcaaaaaagggaataagggcgacacggaaatgttgaatactcatactcttcctttttcaatattattgaagcatttatcagggttattgtctcatgagcggatacatatttgaatgtatttagaaaaataaacaaataggggttccgcgcacatttccccgaaaagtgccacctgacgtctaagaaaccattattatcatgacattaacctataaaaataggcgtatcacgaggcccttaggccaaataggccgttcagatccttccgtatttagccagtatgttctctagtgtggttcgttgtttttgcgtgagccatgagaacgaaccattgagatcatgcttactttgcatgtcactcaaaaattttgcctcaaaactggtgagctgaatttttgcagttaaagcatcgtgtagtgtttttcttagtccgttacgtaggtaggaatctgatgtaatggttgttggtattttgtcaccattcatttttatctggttgttctcaagttcggttacgagatccatttgtctatctagttcaacttggaaaatcaacgtatcagtcgggcggcctcgcttatcaaccaccaatttcatattgctgtaagtgtttaaatctttacttattggtttcaaaacccattggttaagccttttaaactcatggtagttattttcaagcattaacatgaacttaaattcatcaaggctaatctctatatttgccttgtgagttttcttttgtgttagttcttttaataaccactcataaatcctcatagagtatttgttttcaaaagacttaacatgttccagattatattttatgaatttttttaactggaaaagataaggcaatatctcttcactaaaaactaattctaatttttcgcttgagaacttggcatagtttgtccactggaaaatctcaaagcctttaaccaaaggattcctgatttccacagttctcgtcatcagctctctggttgctttagctaatacaccataagcattttccctactgatgttcatcatctgagcgtattggttataagtgaacgataccgtccgttctttccttgtagggttttcaatcgtggggttgagtagtgccacacagcataaaattagcttggtttcatgctccgttaagtcatagcgactaatcgctagttcatttgctttgaaaacaactaattcagacatacatctcaattggtctaggtgattttaatcactataccaattgagatgggctagtcaatgataattactagtccttttcctttgagttgtgggtatctgtaaattctgctagacctttgctggaaaacttgtaaattctgctagaccctctgtaaattccgctagacctttgtgtgttttttttgtttatattcaagtggttataatttatagaataaagaaagaataaaaaaagataaaaagaatagatcccagccctgtgtataactcactactttagtcagttccgcagtattacaaaaggatgtcgcaaacgctgtttgctcctctacaaaacagaccttaaaaccctaaaggcttaagtagcaccctcgcaagctcgggcaaatcgctgaatattccttttgtctccgaccatcaggcacctgagtcgctgtctttttcgtgacattcagttcgctgcgctcacggctctggcagtgaatgggggtaaatggcactacaggcgccttttatggattcatgcaaggaaactacccataatacaagaaaagcccgtcacgggcttctcagggcgttttatggcgggtctgctatgtggtgctatctgactttttgctgttcagcagttcctgccctctgattttccagtctgaccacttcggattatcccgtgacaggtcattcagactggctaatgcacccagtaaggcagcggtatcatcaacaggcttacccgtcttactgtcaagaggacatccggtcagataaccgtcatcttcggctactgtctagggcggcggatttgtcctactcaggagagcgttcaccgacaaacaacagataaaacgaaaggcccagtctttcgactgagcctttcgttttatttgatgcactagtgccgatcatattcaataacccttaatataacttcgtataatgtatgctatacgaagttattaggtctgaagaggagtttacgtcccatatggagtcccgctcagaagaactcgtcaagaaggcgatagaaggcgatgcgctgcgaatcgggagcggcgataccgtaaagcacgaggaagcggtcagcccattcgccgccaagctcttcagcaatatcacgggtagccaacgctatgtcctgatagcggtccgccacacccagccggccacagtcgatgaatccagaaaagcggccattttccaccatgatattcggcaagcaggcatcgccatgggtcacgacgagatcctcgccgtcgggcatgcgcgccttgagcctggcgaacagttcggccggcgcgagcccctgatgctcttcgtccagatcatcctgatcgacaagaccggcttccatccgagtacgtgctcgctcgatgcgatgtttcgcttggtggtcgaatgggcaggtagccggatcaagcgtatgcagccgccgcattgcatcagccatgatggatactttctcggcaggagcaaggtgagatgacaggagatcctgccccggcacttcgcccaatagcagccagtcccttcccgcttcagtgacaacgtcgagcacagctgcgcaaggaacgcccgtcgtggccagccacgatagccgcgctgcctcgtcctgcagttcattcagggcaccggacaggtcggtcttgacaaaaagaaccgggcgcccctgcgctgacagccggaacacggcggcatcagagcagccgattgtctgttgtgcccagtcatagccgaatagcctctccacccaagcggccggagaacctgcgtgcaatccatcttgttcaatcatgcgaaacgatcctcatcctgtctcttgatcagatcctgatcccctgcgccatcagatccttggcggcaagaaagccatccagtttactttgcagggcttcccaaccttaccagagggcgccccagctggcaattccgacgtcattgcgttgctagccaagcttaggatccggaacccttaatataacttcgtataatgtatgctatacgaagttattaggtccctcgaagaggttcactagctatctagagcttggactcctgttgatagatccagtaatgacctcagaactccatctggatttgttcagaacgctcggttgccgccgggcgttttttattggtgagaatccaagcccgggaaacgggatcctgatcttgatccgccgcaaagtttgagcgaagtcaataaactctctacccattcagggcaatatctctcttgcaggtgaatgcaacgtcaagcgatggcctacttgcggccgcaagaagctgtcaccggatgtgctttccggtctgatgagtccgtgaggacgaaacagcctctacaaataattttgtttaacgcattgcatcacacaggaaagggtacatggaaaccaaaaaaaataatagtgagtatatccctgaattcgaaaaatcctttcgctatccacagtattggggcgcctggttgggcgcggcggcaatggcggggatcgcattaacaccggcatcattccgcgaccctttgctggcgacgctggggcgttttgccggacggctggggaagagttctcgtcgccgggcgctaattaatctgtcgttgtgctttccgcagcgtagcgaagctgagcgcgaagcgattgtcgatgagatgttcgccaccgcgccacaggcaatggcgatgatggctgagttggcgatgcgcggtccgaaaaaaattcaacagcgtgttgactgggaaggtctggagattatcgaggagatgcgtcgtaacgacgaaaaagtcatttttctcgtaccgcatggctggggcgtcgacattccagccatgctgatggcctctcaggggcaaaaaatggcggcgatgtttcataatcagggtaatccggtttttgactatatctggaacacagtgcgtcggcgtttcggcggacgtttgcatgcgcgtaatgacgggattaaaccctttattcagtctgttcgtcagggctactggggttactacctgccggaccaggatcacggcccggagcatagtgaattcgttgatttctttgcgacatacaaagcgacgctgcctgcaattggtcggctgatgaaagtgtgccgcgcacgcgtgataccgcttttcccggtgtataatggtaaaacgcatcgcctgactatccagattcgcccgccaatggacgatctgctcacggctgacgaccacactatcgccagacggatgaacgaagaggtcgaaatttttgtcggcccgcatccggaacagtacacctggatcctgaagctgctcaaaacccgcaagccaggcgagattcagccgtataagcgtaaagatctttatcccatcaaagagcagaaactcatctctgaagaggatctgtaactcgagtaagattacttcgcattgcaatcagctacggactcaagcttacgtcaggtcatacgatgaaggcgataagtcgcgtaagttgctagcccacgcggctcaccttcacgggtgggcctttcttcgcgatccacatgc

SEQ ID NO: 25 - DNA, 5161 bp, synthetic construct
  source 1..5161: mol_type = other DNA
catggtcatagctgtttcctttaatgcccatggcgtttaccaatgcttaatcagtgaggcacctatctcagcgatctgtctatttcgttcatccatagttgcctgactccccgtcgtgtagataactacgatacgggagggcttaccatctggccccagtgctgcaatgataccgcgacttccacgctcaccggctccagatttatcagcaataaaccagccagccggaagggccgagcgcagaagtggtcctgcaactttatccgcctccatccagtctattaattgttgccgggaagctagagtaagtagttcgccagttaatagtttgcgcaacgttgttgccattgctacaggcatcgtggtgtcacgctcgtcgtttggtatggcttcattcagctccggttcccaacgatcaaggcgagttacatgatcccccatgttgtgcaaaaaagcggttagctccttcggtcctccgatcgttgtcagaagtaagttggccgcagtgttatcactcatggttatggcagcactgcataattctcttactgtcatgccatccgtaagatgcttttctgtgactggtgagtactcaaccaagtcattctgagaatagtgtatgcggcgaccgagttgctcttgcccggcgtcaatacgggataataccgcgccacatagcagaactttaaaagtgctcatcattggaaaacgttcttcggggcgaaaactctcaaggatcttaccgctgttgagatccagttcgatgtaacccactcgtgcacccaactgatcttcagcatcttttactttcaccagcgtttctgggtgagcaaaaacaggaaggcaaaatgccgcaaaaaagggaataagggcgacacggaaatgttgaatactcatactcttcctttttcaatattattgaagcatttatcagggttattgtctcatgagcggatacatatttgaatgtatttagaaaaataaacaaataggggttccgcgcacatttccccgaaaagtgccacctgacgtctaagaaaccattattatcatgacattaacctataaaaataggcgtatcacgaggcccttaggccaaataggccgttcagatccttccgtatttagccagtatgttctctagtgtggttcgttgtttttgcgtgagccatgagaacgaaccattgagatcatgcttactttgcatgtcactcaaaaattttgcctcaaaactggtgagctgaatttttgcagttaaagcatcgtgtagtgtttttcttagtccgttacgtaggtaggaatctgatgtaatggttgttggtattttgtcaccattcatttttatctggttgttctcaagttcggttacgagatccatttgtctatctagttcaacttggaaaatcaacgtatcagtcgggcggcctcgcttatcaaccaccaatttcatattgctgtaagtgtttaaatctttacttattggtttcaaaacccattggttaagccttttaaactcatggtagttattttcaagcattaacatgaacttaaattcatcaaggctaatctctatatttgccttgtgagttttcttttgtgttagttcttttaataaccactcataaatcctcatagagtatttgttttcaaaagacttaacatgttccagattatattttatgaatttttttaactggaaaagataaggcaatatctcttcactaaaaactaattctaatttttcgcttgagaacttggcatagtttgtccactggaaaatctcaaagcctttaaccaaaggattcctgatttccacagttctcgtcatcagctctctggttgctttagctaatacaccataagcattttccctactgatgttcatcatctgagcgtattggttataagtgaacgataccgtccgttctttccttgtagggttttcaatcgtggggttgagtagtgccacacagcataaaattagcttggtttcatgctccgttaagtcatagcgactaatcgctagttcatttgctttgaaaacaactaattcagacatacatctcaattggtctaggtgattttaatcactataccaattgagatgggctagtcaatgataattactagtccttttcctttgagttgtgggtatctgtaaattctgctagacctttgctggaaaacttgtaaattctgctagaccctctgtaaattccgctagacctttgtgtgttttttttgtttatattcaagtggttataatttatagaataaagaaagaataaaaaaagataaaaagaatagatcccagccctgtgtataactcactactttagtcagttccgcagtattacaaaaggatgtcgcaaacgctgtttgctcctctacaaaacagaccttaaaaccctaaaggcttaagtagcaccctcgcaagctcgggcaaatcgctgaatattccttttgtctccgaccatcaggcacctgagtcgctgtctttttcgtgacattcagttcgctgcgctcacggctctggcagtgaatgggggtaaatggcactacaggcgccttttatggattcatgcaaggaaactacccataatacaagaaaagcccgtcacgggcttctcagggcgttttatggcgggtctgctatgtggtgctatctgactttttgctgttcagcagttcctgccctctgattttccagtctgaccacttcggattatcccgtgacaggtcattcagactggctaatgcacccagtaaggcagcggtatcatcaacaggcttacccgtcttactgtcaagaggacatccggtcagataaccgtcatcttcggctactgtctagggcggcggatttgtcctactcaggagagcgttcaccgacaaacaacagataaaacgaaaggcccagtctttcgactgagcctttcgttttatttgatgcactagtgccgatcatattcaataacccttaatataacttcgtataatgtatgctatacgaagttattaggtctgaagaggagtttacgtcccatatggagtcccgctcagaagaactcgtcaagaaggcgatagaaggcgatgcgctgcgaatcgggagcggcgataccgtaaagcacgaggaagcggtcagcccattcgccgccaagctcttcagcaatatcacgggtagccaacgctatgtcctgatagcggtccgccacacccagccggccacagtcgatgaatccagaaaagcggccattttccaccatgatattcggcaagcaggcatcgccatgggtcacgacgagatcctcgccgtcgggcatgcgcgccttgagcctggcgaacagttcggccggcgcgagcccctgatgctcttcgtccagatcatcctgatcgacaagaccggcttccatccgagtacgtgctcgctcgatgcgatgtttcgcttggtggtcgaatgggcaggtagccggatcaagcgtatgcagccgccgcattgcatcagccatgatggatactttctcggcaggagcaaggtgagatgacaggagatcctgccccggcacttcgcccaatagcagccagtcccttcccgcttcagtgacaacgtcgagcacagctgcgcaaggaacgcccgtcgtggccagccacgatagccgcgctgcctcgtcctgcagttcattcagggcaccggacaggtcggtcttgacaaaaagaaccgggcgcccctgcgctgacagccggaacacggcggcatcagagcagccgattgtctgttgtgcccagtcatagccgaatagcctctccacccaagcggccggagaacctgcgtgcaatccatcttgttcaatcatgcgaaacgatcctcatcctgtctcttgatcagatcctgatcccctgcgccatcagatccttggcggcaagaaagccatccagtttactttgcagggcttcccaaccttaccagagggcgccccagctggcaattccgacgtcattgcgttgctagccaagcttaggatccggaacccttaatataacttcgtataatgtatgctatacgaagttattaggtccctcgaagaggttcactagctatctagagcttggactcctgttgatagatccagtaatgacctcagaactccatctggatttgttcagaacgctcggttgccgccgggcgttttttattggtgagaatccaagcccgggaaacgggatcctgatcttgatccgccgcaaagtttgagcgaagtcaataaactctctacccattcagggcaatatctctcttgcaggtgaatgcaacgtcaagcgatggcctacttgcggccgcaagaagctgtcaccggatgtgctttccggtctgatgagtccgtgaggacgaaacagcctctacaaataattttgtttaacgcattgcatcacacaggaaagggtaccatgaatcgtactaaactggtactgggcgcggtaatcctgggttctactctgctggctggttgctccagcaacgctaaaatcgatcagctgtcttctgacgttcagactctgaacgctaaagttgaccagctgagcaacgacgtgaacgcaatgcgttccgacgttcaggctgctaaagacgacgcagctcgcgctaaccagcgtctggacaaccaggctactaaataccgtaagcatcaccatcaccatcactaaatcagctacggactcaagcttacgtcaggattaaagaggagaaactcgagatgaaccgtactaaccagctgatcttaggtgcagtagttctgggttccacgttactggcaggttgttcaagcaacgctaaaatcgatcagttgtcttccgatgtacagacgctgagcgctaaagttgagcaactgagtaatgacgtaaatgcaatgcgttccgacgttcaggctgctaaagacgatgctgctcgcgcgaaccaacgtctggacaacaaagtattccgcatctgtaaagagcagaaactcatctctgaagaggatctgtaactcgagtaagattacttcgcattgcaatcagctacggactcaagcttacgtcaggtcatacgatgaaggcgataagtcgcgtaagttgctagcccacgcggctcaccttcacgggtgggcctttcttcgcgatccacatg

SEQ ID NO: 26 - DNA, 945 bp, synthetic construct
  source 1..945: mol_type = other DNA
atgaaaataacattaattattcccacatataatgcagggtcgctttggcctaatgttctggatgcgattaagcagcaaactatatatccggataaattgattgttatagactcaggttctaaagatgaaacggttccgttagcctcagacctgaaaaatatatcaatatttaatattgactctaaagattttaatcatggaggaaccagaaatttagcagttgcaaaaactctggacgctgatgttataatttttctaacgcaagatgcaattctcgcggattcggatgcaattaaaaatttggtttattatttttcagatccattgatagcagcggtttgtggtagacaacttcctcataaagatgctaatccccttgcagtgcatgccagaaattttaattatagttcaaaatctattgttaaaagtaaggcagatatagaaaaattgggtattaaaactgtatttatgtccaattcttttgctgcctatcgccgttccgtttttgaagagttaagtgggtttcctgaacatacaattcttgccgaggatatgtttatggcggctaagatgattcaggcgggttataaggtcgcctactgcgctgaagcggtggtaagacactcccataattataccccgcgagaagagtttcaacgatattttgatactggtgtatttcatgcttgttctccgtggattcagcgtgactttggcggagccggtggtgagggtttccgcttcgtaaaatcagagattcaattcctgcttaaaaatgcaccgttctggattccaagagctttattaacaacctttgctaaattcttgggttacaaattaggcaagcattggcaatctttaccgttgtctacatgtcgctattttagcatgtacaagagttattggaataatatccaatattcttcgtcaaaagagataaaataa

SEQ ID NO: 27 - DNA, 1062 bp, synthetic construct
  source 1..1062: mol_type = other DNA
atgatcgtaaacctatcacgtttaggtaaaagtggtacgggaatgtggcaatactcgattaaatttttaacggcactgcgagaaatagctgatgttgacgcaataatctgtagcaaggtacacgctgattattttgaaaagctcggttatgcagtagttactgttccgaatattgttagcaacacatcaaaaacatcgcgacttagaccattagtatggtatgtatatagttactggcttgcgctgagggttttaattaagtttggtaataaaaaattggtgtgtactacacatcacactatccccttactgagaaaccaaacgataaccgtacatgatataagacctttttattatccagatagttttattcagaaagtgtattttcgctttttattaaaaatgtccgttaagcgatgtaagcatgttttaacggtatcttataccgttaaagatagcattgctaaaacttataatgtagatagtgagaaaatatcagtaatttataatagtgttaataaatctgattttatacaaaaaaaagaaaaagagaattactttttagctgttggtgcaagttggccacataaaaatattcattcattcataaaaaataaaaaagtttggtctgactcttataatttaattattgtatgtggtcgtactgactatgcaatgtctctccaacaaatggtcgttgatctggaactaaaagataaagtgacttttttacatgaagtctcatttaatgaattaaagattttatattctaaagcctacgcgcttgtttatccatctattgatgagggttttggtatacctcctattgaagcgatggcatcaaatactccagttatagtgtccgatataccagtatttcatgaagtgttaaccaatggtgcattatatgtgaatccggatgatgaaaaaagctggcagagtgcaattaaaaatatagagcagttgcctgatgcaatttcccgatttaacaactatgtcgcacggtatgactttgataatatgaagcagatggttggcaattggttggcggaatcaaaataa

SEQ ID NO: 28 - DNA, 1002 bp, synthetic construct
  source 1..1002: mol_type = other DNA
atgcttatatcattttgtattccaacttataatagaaaagaatatcttgaagagttgttgaatagtataaataatcaggaaaaatttaatttagatattgagatatgtatatcagataatgcctctactgatggtacagaggaaatgattgatgtttggaggaacaattataatttcccaataatatatcggcgtaatagcgttaaccttgggccagataggaattttcttgcttcagtatcccttgcgaatggggattattgttggatatttggcagtgatgatgctcttgcgaaagactcgttagcgatattacaaacttatctcgattctcaagcagatatatatttatgtgacagaaaagagaccgggtgtgatttagttgagattagaaaccctcatcgttcttggctcagaacagatgatgaactttatgtgtttaataataatttagatagggaaatctatctcagtagatgcttatctattggtggtgtatttagctatctaagttctttaatagtaaaaaaagaacgatgggatgccattgattttgatgcgtcctatattggcacttcctatcctcatgtatttatcatgatgagcgtatttaatacgccagggtgccttttgcattatatatcaaaaccactcgtaatatgccgaggagataatgatagtttcgagaagaaaggaaaggccagacgaattttaattgattttattgcatatttaaaattagctaatgatttttacagtaaaaatatatctttaaaacgagcatttgaaaatgttttgctaaaagagagaccatggttatatacaactttggctatggcatgttatggcaatagtgatgaaaaaagagatttatctgaattttatgcaaagctaggttgtaataaaaatatgatcaacactgtacttcgatttgggaaactagcatatgcagtgaaaaatattaccgtgcttaagaattttactaaacggataattaagtag

SEQ ID NO: 29 - DNA, 984 bp, synthetic construct
  source 1..984: mol_type = other DNA
atgacagtggatagtaatacgtcttccgggcgtgggaacgatccggaacagattgatttgattgagttattgctacagttatggcgtgggaagatgaccattattgtagccgttattatcgccattttgctggctgtaggctacctgatgatagccaaagaaaaatggacatccacggcgattattacccaacctgatgccgcgcaggttgccacctataccaacgcgctcaacgtcttgtatggtgggaatgcccccaaaatctctgaagtgcaggcgaattttataagccgctttagctctgcgttttccgcattatcggaagtgctggataatcagaaagagcgggaaaagcttaccattgaacagtcggtaaaagggcaggcgctgccactctcggtttcttatgtgagtactaccgctgaaggggcgcagcgtcggctggcggaatatatccaacaggtggatgaagaggtcgctaaggaactggaagttgacctgaaagataacatcacgctgcaaaccaaaacgttgcaggagtcccttgagacgcaggaagttgtggcgcaggagcaaaaagatctgcgtattaagcaaatcgaagaagcgttgcgctatgcggatgaggccaaaatcacgcagccgcagattcagcaaacccaggatgttacccaggacacgatgttcctgttggggagcgatgcgctaaaatcgatgatacagaacgaagcgacgcgtccactggtcttttctccggcctattaccagacgaagcagacactgctggacattaaaaatctgaaagtgactgccgatacggtgcacgtctatcgttatgtgatgaagccgacgctgccggtccgtcgcgatagcccgaaaacagccattacccttgtgctggctgtattgctgggtgggatgatcggtgccgggattgtgctgggacgcaatgcgctacgtagctataagccaaaagccttgtaa

SEQ ID NO: 30 - DNA, 930 bp, synthetic construct
  source 1..930: mol_type = other DNA
atgaaaatttcattagtggttcccgtctttaatgaagaggacgcgatccctattttctataaaacggtcagagaatacagttcacttaaaccttataacgttgagattatcttcgttaatgatgggagtcacgatgcgactgaatcaatcatcagcgcattagctgttgccgatcctcttgttgttccgatctcatttacccgcaattttggtaaagaacctgcactttttgccggattagatcacgcgaccggagatgtggtgatccctatcgatgttgatttacaagatcccatcgaagtaatcccacatttgatcaataaatggcaggctggtgcagaaatggtgctggctaagcgtatcgatcgttcaacggatggccacctgaagcgtaaaagcgctgagtggttctacaggctgcataacaaaatcagtacgccaaagattgaagagaatgtcggtgattttcgattgatgtcgcgcgagattgtagaaaatatcaagctattaccagaacgtaaccttttcatgaaaggtatactttcatgggttggaggtcaaacagatgtggtcgaatatgcccgtgctgaacgtgtcgcaggtaactcaaaatttaatggctggaaactctggaacctggcgctggaggggattacaagtttttctactttccctttgcgtatctggatgtatataggagtgagcgtttctgccctctccctgatatatgccatgtggatgatcattgataaattgatgtggggaaaccctgttcctggttatccttcgcttatgaccgcgattctcttcttaggcggcatccagcttatcggcataggcatcatgggtgaatatatcggacgcgtttacacggaggtgaagcaaagaccccgctatatcgtgaaaaacaaaaaaacaatgatggaataa

SEQ ID NO: 31 - DNA, 927 bp, synthetic construct
  source 1..927: mol_type = other DNA
atgaaaatctcgttagtcgttccggtcttcaatgaagaagccacgatacctattttctataaaacggttcgcgagtttgaagagctaaaaccgtatgaagttgagattgttttcatcaacgatggaagcaaagatgcgactgaatcaataattaacaaaatagctgcatctgatccgctcgttattccgctttcgtttacgcgaaacttcggtaaagaacctgctcttttcgcgggtctcgaccatgcaaccggggatgcggtcattcctattgatgtcgatttacaggatccgatagaagtaatcccccatctcattgagaagtggcaggctggcgcggatatggtgctggctaagcgctcagaccgctcaactgacgggcgcatgaagcgtaagacagctgaatggttttataagctgcataataaaatcagcaatccgaaaattgaagagaacgttggcgactttcggttaatgagtcgtgaggttgtcgaaaatattaaacagatgccagaacgtaatctgtttatgaaaggcgttctgtcatgggtgggcggcaagactgatgtagttgaatacgcccgcgctgagcgtgttgccggcgattcaaaattcaatggctggaaattatggaatctggcgctggaaggaataacttctttctcaacatttccgctccgcatatggacttacattggattgtttattgcaggtatgtcattcctttacggtgcatggatgattattgataaattaatatttggaaataatgttcctggctacccgtctcttcttgtttctgtactttttctgggtggcgttcaattgataggaataggtattcttggggaatatattggcaggatttacatagaaacaaaaaaaaggcctaagtacataattaagaatgagaagaaaaatggttaa

SEQ ID NO: 32 - DNA, 1431 bp, synthetic construct
  source 1..1431: mol_type = other DNA
atggataatattgataataagtataatccacagctatgtaaaatttttttggctatatcggatttgattttttttaatttagccttatggttttcattaggatgtgtctattttatttttgatcaagtacagcgatttattcctcaagaccaattagatacaagagttattacgcattttattttgtcagtagtatgtgtcggttggttttggattcgtttgcgacattatacataccgcaagccattttggtatgagttaaaagaaatttttcgtacgatcgttatttttgctatatttgatttggctctgatagcgtttacaaaatggcagttttcacgctatgtctgggtgttttgttggacttttgccctaatcctggtgcctttttttcgcgcacttacaaagcatttattgaacaagctaggtatctggaagaaaaaaactatcatcctggggagcggacagaatgctcgtggtgcatattctgcgctgcaaagtgaggagatgatggggtttgatgttatcgctttttttgatacggatgcgtcagatgctgaaataaatatgttgccggtgataaaggatactgagattatttgggatttaaatcgtacaggtgatgtccattatatccttgcttatgaatacaccgagttggagaaaacacatttttggctacgtgaactttcaaaacatcattgtcgttctgttactgtagtcccctcgtttagaggattgccattatataatactgatatgtcttttatctttagccatgaagttatgttattaaggatacaaaataacttggctaaaaggtcgtcccgttttctcaaacggacatttgatattgtttgttcaataatgattcttataattgcatcaccacttatgatttatctgtggtataaagttactcgagatggtggtccggctatttatggtcaccagcgagtaggtcggcatggaaaactttttccatgctacaaatttcgttctatggttatgaattctcaagaggtactaaaagaacttttggctaacgatcctattgccagggctgaatgggagaaagattttaaactgaaaaatgatcctcgaatcacagctgtaggtcgatttatacgtaaaactagccttgatgagttgccacaactttttaatgtactaaaaggtgatatgagcctggttggaccacgacctatcgtttcggatgaactggagcgttattgtgatgatgttgattattatttgatggcaaagccgggcatgacaggtctatggcaagtgagtgggcgtaatgatgttgattatgacactcgtgtttattttgattcctggtatgttaaaaactggacgctttggaatgatattgccattctgtttaaaacagcgaaagttgttttgcggcgagatggtgcgtattaa

SEQ ID NO: 33 - DNA, 1104 bp, synthetic construct
  source 1..1104: mol_type = other DNA
ttacttggttaagtttggccggttctcacgttgcctgcgcaggcgacgcttcacacgcttaataaatctcgccaccttccaggcccgcttaatgcagtagccatagaggaagaatgctagcaaaaagagcaccaacataacccattcaggaacaaaatgagagtattctgccgttacgcctactcccgccagaatcgccgctgcgagcgtaataagaacaaatgcctggcgggaagtaaaccctgctcgcataaccaaatgatgaatatgttggcgatcaggggaaaaggggctcatccctttacgcagacggcgatacataatcgccaccatatccatcaatggaatagcgataatccatagcgcggtaaccgggctgatagagtgagttttcccctgcgtcgtttccagtaagagccagatgacggtaaagccaatcagtgtactaccggcatcgcccataaagactttgtaacgccgccccaaaataccgagattaagcataatgtaaggcagaatcgcggcgatcatggcaaagcaccacattgccagactagtctgaccatcaaaccataaaatcagccccatcgccgcaaatgagacgctggataacccacccagcaggccgtcaataccgtccaccatattgaaagcgttgatcgccgcccataccgcaaacagagtaaggaaatagccaaaggggccaagcactaactcccaaggcccaaagatgtaaccaaggctacctaagtgaagttttgcgataaccatcattacaaccgcaataacagcctgaaccacagcacgaatttttacactgatatcaaaacggtcatccatcgcaccaacaaaaaccaatacaccagcgcaaataagatatagcgataagtgcggtatgtagtaatccgagaggccaaacataaagcagattcctgcaaacacagaaatcccgccgactaatgggataacgccctgatgtcgtttacgaaagtttggtttatccactaaaccaatttttatggctacttttcgcgcaagaaaaataaaaatggtcgtgaataaaaaaatactgattagctcagataaagcggtgagtaacttcac

SEQ ID NO: 34 - DNA, 1080 bp, synthetic construct
  source 1..1080: mol_type = other DNA
atgaaaatagcttttattggcgaagcggtatccggttttggagggatggaaaccgttattagcaacgttatccatacgtttgaaaatagctctccgaagatcaactgtgaaatgtttttcttttgtcgtaatgacaaaatggataaagcatggctaaaagagattaaatatgcgcaatcattctcaaatataaaattaagttttcttcgtcgagctaagcatgtttataattttagtcagtggctgaaagaaacgtcaccggatattgtgatatgtattgatgtcatctcatgtctttatgccaataaagcacgaaagaaaagtggtaaacattttactattttctcgtggccgcatttttcgctcgaccataaaaaacatgcagaatgtataacgtacgcggattatcatctggccatcagtagtggtattaaagaacagatcatggcacggggtatctcagcgcaagatattagcgtcgtttataatcctgtctctattaaaacagtcattgtgccgccgcctgagcgcgataaaccagctgtatttctctatgtagggcgtcttaaatttgaagggcagaaaagagttaaagatttatttgatggcttagctcgtacgacaggggaatggcagctacatattattggtgatggctcagattttgaaaagtgccaggcctatagtcgggagcttggtattgagcagcgtgtgatctggtatggttggcaaagcgcgccgtggcaagtcgtacagcaaaaaataaaaaatgtcaccgcgttactacttacctctgcatttgagggatttcctatgaccctgctggaagcaatgtcatatggaattccgtgtattagttctgattgtatgtctggtccgcgcgatatgattaaacccggtttgaatggtgagctttacactccgggtgctatagatgattttgtaggacaccttaatcgcgttatttctggtgaagtaaaatatcagcatgatattattcccggcacgattgagagattttacgatgtgctatattttaaaaattttaataatgcaatattctcgaaattacaaaagtga

SEQ ID NO: 35 - DNA, 954 bp, synthetic construct
  source 1..954: mol_type = other DNA
ttaatgaatctttccaaatacgcttgtggcatctaaattcgccaggttctgttctggtgagcagcatgccatttggttcttcccataacctccaattaacccagggtccgttgggccatatagcgtaatattcggtctgtcgagcgcggcggtgagatggctcaggccggtatcaaccgatacgacaaattttgcgccagccagcactctggcgacctcctccaggctcatgcgcggtaacacatccacatagtcaaagccttcggccagtcgtttagcccgggcctcctcatgaggcgcgccccagggaagctttatccgtaatccggtgttgcccaccaggccgataagctcgcgccagtttgcttccggccagtgtttatcatcgcgggtcgtggcatgtaaaaacaccgcatacggatcgctaaccgcctgctggcaatgcagaaaatgttttgcgatggcataatcgccctgcgactgcggtttatcgtatcccaggcttttggcgaacagctcgcgcgtccgttcaaccgcatgttgttgctttgcgatatggtgtttacggttatagaacaggctggccagcggttcgcgggcggtactccagtccataccgtgctttatcccatgcgccagacgcgtcaccagcgccgcgctttttaccagcccctgcgcatcaatcacagcgtcgtattggtttgcgcataccgcccgacgaaaggctgtgcgttccgctttgatgggcgcggaaaaccaggccttgcgccaacggcgaatagcgacgggaatcacgcgatcgacagcactgtgccaggacggaatttgtgcaaacccttcttcgacagcccaatcaaattgaatccccggaatcgcctgttgcgcgtcggtaagcgcaggcagggtatgtaatacgtcgcccatcgatgatgttttaacgatcaaaacccgcat

SEQ ID NO: 36 - DNA, 1047 bp, synthetic construct
  source 1..1047: mol_type = other DNA
ttaaacgccctcttccgacaacagcgaatgaagctcttccagaacccgctgcggcgtgatatcgatcaggctctggtgatagccttgcgccgtatcacctttacgcactttgtgataacccgtaatgagacgaatcacccgggccttatgagacagcggcggcgtgaaatccgggctacttggaccatacaaggcgaccagcgggcggtcgagcgccgccgcgacgtgcatcagcccggaatcgttagtgacgatggctttacaggcggctatcagaatgacggcctgttccagctgggtttcccccgccaggttgcgacaccatgcctgctgctcgctattcagcgccgccaggatctcatttccggcttcatggtcttttgccgagccaaacagcacgacctgatacccttcgttaatgagctgctttgccagttcggcgtagtgatagtgcggccaacgttttgccgggccaaattctgcgccggggcaaaagccgatcagaggacgttcagaagatagtgaaaagtcgctgcacatcagcgacttttcaccctcgctaacctggagctgtggccagagtagcggctggggcagatctttcgccgtgcgcatcacgcccttgtcataagccagcgccacgtagcgctccaccatcagtggccaggcgtctttatcaaggacgcgcgcatcgttcagcaggccatagcgcatttcgccgcgccagccggtacggtgcgggatattggcaaagaaaggaatcagcgccgatttaaacgaatttggcaacacccaggcgcgatcgtagcgcttctctcgcaggctatggcccaatctgcggcgctcgccgatttccagcgcgccgtggcccaacggcatgggtatcgcctcgttaacttccggcatacgcgataataacggacgacaccaggctggcgccatcacgtcgattatcgcctggggatagcgtgctttaagcgtgcgatagagactttgcgacatcatcatgtcgcccacccaggacgggccaatgaccaaaattttcat

SEQ ID NO: 37 - DNA, 1125 bp, synthetic construct
  source 1..1125: mol_type = other DNA
atgagagttgccttttgcttatataaatattttccttttggcggtctgcagcgtgattttatgcgcattgcccaaaccgtggcggcgcgagggcatcaggttcgtgtttatactcagtcatgggaaggggaatgcccggataactttgaattaatccgcgtgccggttaaatcccggacgaaccacggtcgtaacgcagaatattatgcctgggtgcaacaccatttgcgcgaccaccctgtcgatcgggtggttggattcaataagatgccgggccttgatgtgtattacgccgcagacgtgtgttacgccgaaaaagtcgcacaggaaaaaggatttttctatcgcctgacatcacgctatcggcattatgctgcttttgaacgcgccacgtttgaacacggcaagccgacgcaactattaatgctgacgaataagcagattgctgacttccaaaaacattatcagactgaagcggagcgtttccatattcttcctccggggatttacccggacagaaaatatagccaacagatcccaaacagtcgtcaaatttatcgtcagaaaaatggtatctcagaacagcaaaaattactgttgcaagtagggtctgactttacccgtaaaggtgtggatcgctctattgaagcgctggcatcgctacccgaatctttacggcaaaatacggtgctctatgttgtcgggcaggataagccgaagaagtttgcagcactggctgaaagaagcggcgtcggcacgaatgtgcattttttctccggacgtaatgatatcgcggagttaatggcggcagccgaccttttactgcatccagcctatcaggaagctgctggtattgttttgctggaagccattactgctggtttgccggtgctgacaaccgcggtgtgcggttatgcacattatattgtggatgcaaactgtggcgaagcgatgactgaaccattccgccaggatgcgctaaatgaggttttactcaaagcgctgacacagccttccttacgcaacgcctgggctgaaaatgcgcggtattatgctgatacccaggatttatacagcttaccggagaaggccgcggatattattacaggtgatttagatggttga

SEQ ID NO: 38 - DNA, 1035 bp, synthetic construct
  source 1..1035: mol_type = other DNA
atgaaaaatagtaaaaccaaagtgagtatcattgtcccgttatataatgcgggagcggattttaatgcttgcatggcgtcgttaatcgcgcaaacgtggtcggcgctggaaattattattgtgaatgatggatcgacggatcattccgttgagatagcaaaacattacgcggaacattacccacatgttcgactgcttcatcaggccaatgctggcgcatctgtcgcccgtaatcttggcctgcaagcggcgaccggcgattatgtcgcctttgtcgatgcggatgaccaggtctacccgaagatgtatgaaacgctgatgactatggcgcttaacgatgatctggacgttgcgcagtgtaatgcggactggtgcgtccgaaaaaccgggcacgcctggcaatctattccgaccgatcgtctgcgttccaccggggtattaagcggaccggattggttgcgtatggcgttggcctcgcggcgctggacgcatgttgtctggatgggcgtttatcgacgtgcgttaattaccgataacaatattactttcgttcccggactacatcatcaggacatattatggtcgacggaagttatgtttaatgccacgcgcgtacgttataccgaacaatcattatataaatatttcctgcatgataattcggtaagccgtttgcaaagacaaggcaataaaaatcttaattatcagcggcattatattaaaattacgcgattattagaaaagctcaatcgtgattatgcccgtcgtattccgatttacccggaatttcgccagcaaattacctgggaagcgttacgcgtttgtcatgcggtacgtaaagagcctgatattttgacccgccagcgtatgattgccgaaatttttacttctggcatgtatagacggatgatggctaacgtccgcagcgcgaaagcagcttatcagacgctgctctggtccttccggctgtggcaatggcgcgacaaaaccttgtcgcaccgtcgtatggcccgtaaggcgctcaatctgtcttag

SEQ ID NO: 39 - DNA, 1014 bp, synthetic construct
  source 1..1014: mol_type = other DNA
atgagcagaaaatattttgaagaagaagtcattcaacagactttagattataactatgcacaacatagtgatgctgataaatttaatatagcttatgggattgataaaaactttctttttggctgtggtgtctctattgcatcggttctcctcgctaatccagagaaggcgttagctttccatgtttttaccgatttctttgactctgaagaccagcagcgatttgaggcattagcaaaacagtacgctacgcagattgttgtttacctaatcgactgtgagcgcttaaaatcgctacccagtaccaaaaactggacctatgcaacatactttagattcattatcgccgattatttttcagataaaacagatagagtactttatctggatgcagatattgcatgtaaggggagtattcaggaacttattgatcttaattttgctgaaaatgagattgcggctgtcgttgctgaaggcgagttggaatggtggactaagcgctcggttagcctggcaacgcctgggctggtttctggctattttaatgccggttttattttaattaacatacctctttggactgcagaaaatatctctaagaaagcgattgaaatgctaaaagatccagaggtagtacagcgcataacgcaccttgatcaggatgtattaaatatatttttagtgaataaagcgcgttttgttgataaaaaatttaatacacaatttagtcttaactatgaattaaaagattcagttattaatccagttgatgctgagactgtatttgttcattatatcggaccaacgaagccctggcatagttggggggcttaccccgtgtcacaatattttttacaggctaagagcaactcaccatggtctcattgtgcacttttaaatccagtgactagccatcagttacgttatgcggcaaagcatatgtttaatcagaagcattatacttcgggtataaattattatatagcctactttaaacgtaaacttcttgaataa

SEQ ID NO: 40 - DNA, 1011 bp, synthetic construct
  source 1..1011: mol_type = other DNA
atggattcatttcctgagatagaaatagctgaatataaagtttttgatgaaagtaataataatgatgataacgtattaaacatttcttatggcgttgatgaaaactatcttgatggtgtgggggtatcaatcgcttcagttgtattaaacaataatatcccgctcgcttttcacattatttgtgactcatactccccgtgttttgtaaaatatatagagcgtttagccgtacagcatcacataaaaatttctctttatcttattaaagtagaaagccttgaggtattgcctcaaactaaagtatggtcgagagcaatgtattttcgtttatttgctttcgattatctcagcaagaaggtaaataccttactttatttggatgccgatgttgtatgcaaaggatctttgcaagatcttttacagcttgatctgacagagaagatcgctgcggtcgtaaaagatgttgattccatccagaataaggtaaatgagagattaagcgcttttaatttacaaggtggttattttaactccggcgtggtttttgttaacctgaaattatggaaagagaatgccttaaccaaaaaggcatttttacttttggcaggtaaagaggctgactcttttaaatatcccgatcaggatgttttgaatattctcctacaggataaagtcatttttctaccgcgaccgtataatactatttatactattaaaagtgagttgaaagataagtcacataaaaaatatagcaatataattaatgataatactattttaattcattatacgggcgctacaaaaccatggcatgcctgggcaaattatccttcagttatctattataaaaatgcacgactgaactcgccctggaaagattttcccgcaaaagatgcgcgtaccatagtcgaatttaagaagcgatataaacatcttctcgtgcaaggtcattattttaaaggccttctggctggaagcgcatatctttatcgtaaacttttccacaaataa

SEQ ID NO: 41 - DNA, 1146 bp, synthetic construct
  source 1..1146: mol_type = other DNA
atgattaaaaaaatcatatttactgttactcctatattttcaattcctcctcgtggtgcggctgcggtagaaacctggatttaccaggttgcaaaacgactatcaataccgaatgctattgcttgtataaagaatgctggctatcctgaatataataaaataaacgataactgtgatattcattacatcgggtttagtaaagtttataagcgtctttttcagaaatggactcgtctcgacccactaccctattcccagcgcatccttaatattagagataaagtgactacccaggaagatagcgtcattgttattcataatagtatgaaactgtatcggcagatcagagagcgcaatccgaatgcaaaactggttatgcacatgcataatgcatttgaaccagaacttcctgataatgatgcaaaaattatcgtgcccagtcagtttcttaaagcgttttatgaagaaagattgcccgccgctgctgttagtattgtgcctaatggtttttgtgctgagacttataaaagaaacccacaagataatcttcgtcagcaattaaatattgcggaagatgccaccgttctcttgtatgccgggagaatttcgcctgataaaggcatcctgttgcttttgcaggcgttcaaacaattacgtaccttaagaagtaatattaaacttgtcgttgttggcgacccttatgcaagccgcaagggtgaaaaagcagagtatcaaaagaaagtactggacgccgcaaaagagattggaacggattgtattatggctggggggcaatctcctgaccagatgcataacttctatcatatagccgatctggttattgtgccatctcaggttgaagaagcattttgcatggtggctgtagaagcgatggcagcaggaaaagcggttcttgccagcaaaaaaggggggattagcgaatttgtgttagatggcataacgggctatcacctcgcagaacctatgtcgagcgacagtataattaatgatattaaccgtgcgcttgctgataaggaacgccaccagattgccgaaaaagcaaaatccctggtgttttcaaaatacagttgggaaaatgtagcgcagcgtttcgaggaacaaatgaaaaactggtttgataagtga

SEQ ID NO: 42 - DNA, 1215 bp, synthetic construct
  source 1..1215: mol_type = other DNA
ttatctatttcttagcgccagcagaaaaccggtaatgataccaatttgagcaatatcgacctgttcaaaattgccacgaacgatataaaaaccgacgaaagataaaaatagcaagagatgagcattgtaggggcttatctctactttcctgagggtagagctggctgtttccctgatgatagcgccatataaatagaccaggctcgccagacccaatatgcctgcactaaaccagatgtacagaatggtattatgcggaccgatagattctttaaaggtccacgttggataatcgacaacgcgtttattataaacaccatcatacacatcattaccatagccgtagcccttgatcgggttttcctgaatcagtatccacgcggtgccctgggttccgttagtataacgatatgagctatctgtctgctgtaatttatacagtaaatgttctgggtctggtttgttattatgttgagtgataaccaaagcgccgataatggctaataaaatggcaccaactcctattaacttccattggcggttcagtattgcccacagaacacctactataagcaccgccaaccatgcccctcgcgatagggttcccaggataaagaaaaggtagatggcgctaagcaccaaaaaaaccaacttaattgcattttttctaaacagccaaatattcaataatgctggaaataagaaaaccatggaatcggacatatgtcgatgcgcatagcttatgaatggcataatccctttattatagtcctcgatatacagaatactctctgcaaggcagcgaagtcctaaacttgttaaaaaggagaaaagtactattttcgcaaccgtttcttttgtttcatcttttaatagtacgggaattaataaagtatataataagaagccctccagtaccgtattttcaaattccttgaaactttctttcatatctggcgatatgagtatggaataaacaaggattaatgataatactgctacgctataaaatacgctatttttgaaaagaggggggaaacttttcggtgagcgtgagacctgataaatcgcggtgataaccataagtatgattatcaaatgtttataacgcgtaataccatccagaaaatacgtggcaacaaaaagaaaaaccagcgctttattccagatcggcttccatttctctttatttaacgttaatgatgtggttagcat

SEQ ID NO: 43 - DNA, 798 bp, synthetic construct
  source 1..798: mol_type = other DNA
atggttgagctgaaagcgccgttaaccacactatggcgcggtaaagatgcttttgaggaagtaaaaacgttacagggcgaagtgttcagagagctggagacgcgtcgaacattgcggtttgagctggacggtaaaagctacttcctgaagtggcataaaggtacttcgctgaaagaaattgtgaagaacctgatttcgttacgtatgcctgttctgggcgctgacagagaatggcacgccattcatcgtctacatgagctgggcgttgatacgatgcacggcgttggttttggtgaaaaaggcgtaaacccgctaaccagaacatcatttattatcaccgaagatttaacgcccaccattagccttgaagactactgtgctgactgggctgttaatccaccggacgcgcaggtgaagtggatgatcattaagcgtgttgcgactatggtacgtaaaatgcacgccgggggaattaaccatcgcgactgttatatttgccactttcttctgcatttacctttcactggtcgcgaagaggatttaaaaatctccgtaattgacctgcatcgcgcgcagatacgccagcacgttccccttcgctggcgtgacaaagatttaattgggctttatttttcttcaatgaatattggcctgactcagcgagatatattccggtttatgcgtgagtatttctctctccccctgcgagagattttgcaaaaagaatcggggttgattcatcaggcagatgttaaagccgctcgaattaaagaaaggacaataagaaaaaatctgtaa

SEQ ID NO: 44 - DNA, 1071 bp, synthetic construct
  source 1..1071: mol_type = other DNA
gtggaaaagccatttcgaagaattctgattataaaaatgcgttttcatggagacatgttacttaccacccctgtcatcagcacgctgaagcagaattatcccgatgcaaaaatcgatgtgcttctttaccagaacaccataccgatattgtcggaaaatccggagattaatgcactctacggcatcagtaacaaaggcgcaggaacaaaagagaagatcaaaaacgcgctatcgctaatcaaaaaattgcgtgctaactcgtatgatctggtcgtcaatctcaccgatcagtggagcgtggcgcttattgtgcgttttttaaacgcaaaaataaaaatctcgcaggatttcggtaatcgtcagtctgctctatggaaaaagagctttacgcatttagtaccttatgcgggagaacatgctgttgagcgcacattatccgcgctaaagccgttagcgctaaaacagtatgtcacggaaaccaccatgagctatcgcccggaacattgggaaaacatgcgacaacagctcaaacaacttggtgtgacccgacaatatgttgttattcagcctacggcacggcagctatttaagtgctgggataatgataaattctcgcaggttattgatgccgtgcagcgccgcggttatcaagttgtactgacgtcaggcccggccgcagacgagatggcctgcgtggatgctattgcacgcggctgtgagacaaaaccggttactggtctggcgggtaaaactcgctttcctgaattgggtgcgttgattgaccatgcggatctctttatcggcgttgattcggcccccggtcatattgccgcagcagtcaaaacgccggtcatttgtctttttggcgcgacggatcatgtattctggcgtccctggaccgacgacatcattcagttttgggcaggaaattatcagccgatgcctgaacggcatgagcttgatcgtaataaaaaatacctttccgttattccggctgaagatgttatcgccgcgacggaaaaaatgctgccgcatgaggcacgcaccatagatttggacagcctgctatga

SEQ ID NO: 45 - DNA, 1071 bp, synthetic construct; identical to SEQ ID NO: 44
  source 1..1071: mol_type = other DNA

SEQ ID NO: 46 - DNA, 810 bp, synthetic construct
  source 1..810: mol_type = other DNA
atgggcagcgttaacttcataactcacgccgatgttctgcaacttattgcgaaaagaacggctgaagattgtattatttttctttctggtcctacgtccagaaagacgccgctgtccttgttacgaatgaaagatgtcattgcagtcaatggttctgttcaatatttgctaaacaataacgtcaagccatttttgtaccttctgacggatattcgcttcctccatcgtcggcgcgaagatttttataactttagccgtaacagtcagtttactatcgtcaatcttgatgtgtacgaacaggcttcagtggatgatcaaaaatatattgaagaaaactgtttaattattcgctccttttatcgccgagaaaaagggggctttttaaagaaaattaaatttaatatcctcaagcgggttcataaagcattacttatttcagttcctctttcgaaaagagggcgactggctggattttgcaaggatatcagcatcgggtattgctcttgccatactattgcttataccgctattcaggttgcctattccctcaagtatggccgtattatatgttctgggcttgacttaacagggagttgcccacgtttctatgacgaatctaccagccctatgccatctgagcttagtaaagatctgtttaaaatactgccattttttacttttatgagaaaaaatgtgagtgatttaaatatctttaatttatcagatgatactgcaattcattacgatattattccatatattacagcctcggagcttgaggatgaaatatattacgataaaattgtctag

SEQ ID NO: 47 - DNA, 1734 bp, synthetic construct
  source 1..1734: mol_type = other DNA
atgcaatccacattactccagactaaacccgcgtttagctggaaagccctgggctgggcactgctctacttttggttcttttccaccctcctgcaggccattatttatctcaccggatacagcgggacaaacggtctgcgggattcgctactgtacagctcactgtggctgatcccggtctttctgtttccaggccgcatccgggttattgctgccgttattggcgtcgtactctgggccgcctcgctggcggcgctgagctattacgtaatctacgggcaggagttctcgcaaagcgtgctgtttgtgatgtttgaaaccaacgccaatgaagccagcgaatatttaagccaatatttcagtctgaaaattgttcttgtcgcgctggcttatacggtggcggcgattttgctgtggacacgtctgcgcccggtttatattccatccccctggcgttatctggtgtcgtttgccctgctgtacgggctgatcctccatcccatcgcgatgaatacctttatcaagcataagtcgatggagaaaacgctggatagcctggcatcacgaatggaacccgccgcgccgtggcaatttattactggctactatcagtaccgtttacagctcgcctcgctgaataaactgctgaatgaaaacgatgccctgccgccgctggctaacttccaggaccactccggcgatgcgccgcgcacgctggtactggtgattggcgaatcgacccagcgtggccgtatgagtctgtacggttatccgcgcgaaaccacgccggaactggacgcgctgcataaaaccgaccccgggctgaccgtgtttaataacgtggtaacttcgcgaccgtacaccattgagatcctgcaacaggcgctaacgttcgcggacgaaaagaacccggactggtatctgacgaagccatcgctgatgaatatgatgaaacaggccgggtataaaaccttctggatcactaaccagcagacgatgacggcgcgtaataccatgctgaccgtgttctccaagcagactgataagcagttctatatgaaccagcagcgcactcaaagcgcgcgcgaatatgacagcaacgtgctggcgccgtttaaagcggtgttagccgacccggcgccgaaaaaattcattattgtgcatctgctgggaacgcatattaaatacaagttccgctatccagaaaaccagggcaagtttgatggtaaaaccgaccatgttccgccgggattaagcagtgacgagctggaatcgtataatgattacgacaacgcgaacctgtataacgactatgttgtcgccagcctgattaaggactataaagcgaccgatccgaacggtttcctgctctacttctccgatcacggtgaagaagtgtatgacacgccgccgcataagacgcagggacgaaacgaagattcgccaacccgccatatgtatacggtgccgttcctgctgtggacctcagagaaatggcaggcagcgcatccgcgcgacttctcacaggatgtcgatcgtaagtacagcagttccgagcttatccatacctggtcggacttagcgggcctgacctatgatggctacgacccgacgcgttccatcaccaacccgcagttcaaagagaccacgcgctggattggcaacccgtataagaaaaacgcgctgattgattatgatacgttgccgtatggcgatcaggtcggtaatcaatag

SEQ ID NO: 48 - DNA, 579 bp, synthetic construct
  source 1..579: mol_type = other DNA
ttatttaaccatctctttttcgatcaactgaatcaaaatatgaattactttgatatgaatttcctgaatacgatcggcataaccgaagtgcggtacgcgaatttcaatatccgccgttcccgccattttgccgccgtctttgccggtcaacgtaatcactttcatgcctttttcacgggccgcggcaatcgctttaatcacgttaccagagttacccgacgtcgagatccctaacaggacatcgccttcgcgccctaccgcctcaacgtaacgagagaaaatatagtcatagccaaaatcattactgacgcaggatatatggctaacatcagaaatcgcaattgccgggtagcccggacgattttcacgataacgacctgtcagctcttcagcaaagtgcatcgcatcgcaatgggagccgccgttaccgcaggaaagtaccttaccacccgctttaaaactgtcagccaacaggaccgccgcgcgctgaatggcgtgaatattggcgtcatcttttaaaaaattagccagcgtttccgccgcttcgttcagttcgttacgaataagatcctggtacat

SEQ ID NO: 49 - DNA, 567 bp, synthetic construct
  source 1..567: mol_type = other DNA
ttatttttgctgcttttttatcgctgatggcaggtcagcaaggctgtttaacacccagtccgccgcgttttctgcttctgccgtgaccggtttgcccgtacgcaccagcacttttgtcccgacatttgccgccgctgccgcctgcatatcttccagcttgtctcccaccatataagaagccgccatatcgatatgcaggaaatcacgcgccgagataagcattcctggatgcggcttgcggcaatcacatacctgacggaactcttctatactgccctgcggatggtgaggacaataatagatgccgtccaaatcaacatcgcgatccgccaacgaccagtccatccattcggttaacgtttcaaactgcgcctcagtgaatttgccgcgcgcgattccggactggttcgtcaccaccaccaacgcatagcccattttttttagctcgcgcatagcgtcaataacgccgtctataaactcaaatgcatcgatttcatgtacgtagccgtgatccacattaatggtgccgtcacggtcgagaaaaattgcgggtacaaactttgccac

SEQ ID NO: 50 - DNA, 1434 bp, synthetic construct
  source 1..1434: mol_type = other DNA
atgaaagtaaatctgccagcgtttgaacgtgcaggcgtcatggttgtgggtgatgtaatgctggatcgctattggtatggccccacttgccgtatttcaccggaagcgccggtgcccgtggttaaggtaaataccgttgaggaacgcccgggcggcgcggcgaacgtggcgatgaacattgcgtctctgggagcgaacgcccgtctggtcggcctgacgggtattgatgacgccgcgcgcgcgctgagcaaaacgctggcggaggtcaatgtgaagtgcgacttcgtttctgtgccgacgcatccgacgattaccaaactgcgcgtactatcacgtaatcagcagctcattcgtcttgattttgaagaaggctttgagggcgtggacccgcagccgttgcatgagcgtatcaaccaggcgctgggatcgatcggcgcgctggtattgtccgattatgccaaaggcgctctgaccagcgtgcagactatgatttccctggcgcgccaggcgggcgtgccggtgctcatcgatccgaaaggaacggattttgaacgttaccgcggcgccacgctgctgacgccaaacctttctgaatttgaggcggtcgcggggaaatgtaaaagcgaagacgaactggttgaacgcggcatgaaactcattgctgattacgacctttccgcgctgttggtcacgcgttccgaacagggaatgacgctgctgcaaccgaataaagcgccgctacatatgccgacgcaggcgcaggaagtttatgatgttaccggtgcgggcgatacggtgatcggcgtgctggcggcgacgctggcggcgggaaataccctggaagaggcgtgttatttcgccaatgcggcggcgggcgtagtggtaggtaaactcgggacgtcaacggtttcccctattgagctggaaaacgcagtgcgcggacgcgcggataccggcttcggcgttatgaccgaagaggagttgagacaggccgtcgccagcgcgcgtaagcgtggcgagaaagtggtcatgaccaacggcgttttcgatattctgcacgcgggccatgtctcttatctggcgaacgcgcgcaaactgggcgaccgcctgattgttgcggtcaatagtgacgcctcgactaaacgcctgaagggcgaaagccgtccggttaatccgctcgaacagcgtatgatcgtgctaggcgcgctggagtcggtcgactgggttgtctcttttgaagaggatacgccgcaacgactgattgccggtattctgccggatctgctggtaaaaggcggcgactataagccggaagagatcgcgggcagcgaagaggtctgggccaacggcggtgaagtcatggtgctgaacttcgaagatggttgttccacgaccaatatcatcaaaaagatccagaccgagagcgagaagtaa

SEQ ID NO: 51 - DNA, 933 bp, synthetic construct
  source 1..933: mol_type = other DNA
ttacgcgtcgcggttcagccaggccatatactccgtgacgccttcggcgacggtcttaaagggtttgtcgtagcccgcgttgcgcagattggttaaatccgcctgcgtaaacgcctgatagcgacctttcagcttatccgggaacggaatgtattcaatgctaccttttttatggtatgccagcgtcgcgtcggcgacggcctggaaagattccgcacggcctgtgcccaggttaaagatgccggacttgccgctttccaggaaccacaggttaacggcggccacatcgcccacgtaaacgaagtcgcgcttgaagttttcgctgccttcaaacagtttcgggctttcgccgttgtttaactgtgtattcagatgaaatgccacgcttgccatgctgcctttatggccttcacgtggtccatagacgttgaaatagcggaaaccgacaatctgcgagttcgcttctggcaggatctggcgcacatattcatcaaacaggaatttagaatagccataaacgttaagcggtttttcgtattcgcgcgattcgatgaaatcagacgtgcgaccgccataggtggcggcagaagaggcgtagaggaacgggatttcgcgctcaagacaatagtgcagcagctctttggagtattgatagttattatccatcatatacttgccgtcccactcggtggtggaagagcaggcgccttcatggaaaatagcttcgatatcgccgagctcttctccggacataatctggatcaggaaatcttccttatccatatagtcagcaatgttcagatccaccaggtttacaaacttggtgccgtctttcaggttatccaccaccagaatatcggtgatacctttatcattcagggccttaacgatattgctgccgataaagcccgcgccgccggtaacgatgatcat

SEQ ID NO: 52 - DNA, 789 bp, synthetic construct
  source 1..789: mol_type = other DNA
ttaacgaatcggaccgcgcgttgaacgctcaaagaactcggtaaacgccttcacttccggatgcttttcagcaagttcagcgatttccagcttcgcttcgtcgagcgttttaccactgcggtacaacagtttgtaggcattacgaatcgccaccagcccttcacggctaaagccgcgacgcttcagcccttcgatatttaccccgaacggcgtcgcatggttaccctgcgcaatcacatacggagggacatcctgcgccacgccggagcagccgccgaccatcacatgcgcaccgataatgcagaattgatgaactgccgtcataccgccgatgatcgcaaaatcatcgactgatacgtgccccgccagcgtggcgttgttggcgaggatacagcgattacctaccgtacaatcatgtgcgacatgcgcattgatcatcagcaggttatcgctacccaccttcgtcaacccaccgccctgcactgtaccacgatgaatggtgacgctttcgcggatgcggttacgatcgccaatttccacacgggtcggctcacccgcatatttcagatcctggttcacttcaccgatggaggcaaactgataaatctcgttgtcgcggccgattttggtttgaccattcacgaccacatgagacttcagtacggttccctcaccaatttcgacctgcggcccaacaatacaaaagggaccaatgtgggcattagcgccaattacagcgccgtcttccacaatggcggtaggatgaataaaggcggatttatcaatcac

SEQ ID NO: 53 - DNA, 1149 bp, synthetic construct
  source 1..1149: mol_type = other DNA
tcattgtgctaactccaggacggcatctgccgcctgctcatcggcattacagcggatctgctgatgcaattcacggaaggtgtcgtgcatcgcatggctggttttaccgttcgccagtagcggcaacagcgcttcggcgagtttttgcggttcgcactcttcctgcaacagctctttgactaattctcttcccgccagcaggttaggcaaagacacatactccgttttcaccagacgtttcgccagccagaaagtgaagggcttcatacgatatcccactaccatcgggcattttgccagcatacactccagtgccgccgtacccgaggccagcagagccgcgtcgctggcgatcatcgcctcgcgcgccatgccgtccagcaaatgaacggcgagatccggcgcaacctccgctttaattttttcaaactgctcgcggcgtttcgcgttcaccagcggcactaccacttccagatcgggatagcgctgtcgcagcaattgtgcggttttcaggaaatcggcgctgagcatttccacttccgcgccacggctgcctggcagtagcgccagacaatgggcgtcatgcgggatacccagcacgtcgcgcgccgcatttttatccgggtccagcggcatggcatccgccatggtgtgaccgataaagcggcacgggacgttaaatttatcgtaaaacgctttttcgaaaggcagaaaagccaacaccatatgggtggatctgcctattttgaaaacgcgtttctgtcgccaggcccaaacggacgggctgacataatgaatggtcttaatccctttttttttcagattaccttcgagggtaatattgaaatcaggggcatcaatcccgacaaagacatcgggcttgagttcggtaaaacggcgggtcagatcggcgcggatatgcaacaaacggcgtaaacgtccgagcacttcaacaatgcccatgaccgccagctcttccatctcgtaccaggcttcacacccttcggcctgcatacgcggccccgcaacgcccacaaaacgggcgttgggtacgcgcgctttcagcgcacgaattaagcctgcgccaagaatatcgccggacgtttcaccggcgaccagggcaatcgttaaaggacgctgtgccgccat

SEQ ID NO: 54 - DNA, 918 bp, synthetic construct
  source 1..918: mol_type = other DNA
ttatgccagtaccgtcgaaggcgctttgaaagccaacggcagttctgcgtcgtcctggaaggtcacaaattcccaggcttcctgttttgccaggactgcctgtaacaatttattattcaatgcgtgaccggatttatacgcggtaaacgcaccaataatattgtgaccacacatgaacaagtcaccgatcgcgtcaagcattttgtgacgaacgaattcatcttcaaaacgcaggccgtcttcgttcaatacgcgataatcgtcaacaacgatggcacaatcgaagctgccgcccaggcacaggccgcgggactgcagatattcgatatcacgcataaaaccgaaggtacgcgcacggctgatctggcgcatgaacgcatccgcagagaagttcatcgcgtagcgctggctgctggaatcgatcgccggatggttaaagtcgatggtgaaatccaacgtaaaaccattgtacggtctgaattcagcccatttatcgccatcttcaacccgaacagtctctttgatgcgtacgaattttttggcgcagttcagttcatcaataccggcatcaagcagcaggtagacaaacggagcggcactgccatccatgatcgggatttccggggcattaacctcaataacgatgttatcgatacctaagcccgccagagcagcattcaggtgctcaacggttgaaatccgtacatcatgctcattcaccagacacgtacagagcatggtatcacgcacagatttggcatcggccgggaaatctaccggtggattcaagtcggtgcgacgatagatgaccccggtattggccggcgcagggcgtaatgtcagggtgacttttttgccggtgtgtaaaccgacgccagtcgcctgaacgatacgtttaagtgtcctttgtttgatcat

SEQ ID NO: 55 - DNA, 1026 bp, synthetic construct
  source 1..1026: mol_type = other DNA
ttagtcttgttgattaaccttgcgctcaatcgctttgagacgcttgctcatatcatcaatgttcatcaccagtgcagcagttttacgccatactttgttgggttgcagcggaatgcctgaggagtagacgcccggttccgtgatgggacgcatcaccatacccatgccagttaccgtgactttgtcgcatatttccatatgcccattgatcacgctggcgccgccaatcatgcagtaacggccaatcttcaggctacccgccataatgacgccaccggcaactgccgtattgtcgccaatcacgacgttatgtgcaatctggcactgattatcaataatcacgccattgccaataacagtatcatccaacgcgccacggtcaatggtggtacaagcgccgatctcgacacgatcgccaataatgacccggcccagttgtgggatcttcacccagttgccacgatcgttagcgtagccaaaaccgtccgcgccgatcaccgtactggactggatcaggcaattctcaccgatctgaatgtcgtggtaaatcgttacgttcgcccacaagcgtgaacccgccccgattttgctattttttccgacgaaacagcctgcgccgataaccacgttatcgcccagttgtacgccagattcaatcaccgcattcgcgccgactgaaacattgctacccagcgttgccgtcgcatcaatcacggcgcttggcgcgatattctgcgcgggctgcggcgtagtatctaaaatttgcgccatgcgcgcgtaggtcaggtagggatttttaactaccagcgccgcactcttagcaaaaggaagatcgtcctgcgtcatgacaaccgcagaagcctggcataaacctaagtgttcacggtacttaggattcaccataaacgtaatgtggcctgttgttgcagattgcatggacgcaacgccggtgatgacgatatcgccatcaccgtgtaattctgcatccaactgttctgctaagtcagccagtcgaattgaaggcat

SEQ ID NO: 56 - DNA, 723 bp, synthetic construct
  source 1..723: mol_type = other DNA
gtggcgacactgtttattgcagacttgcatctgcaaacggaagaaccggcgatcgtcgccggttttctgcgttttttagccgtagaagcccgtcaggccgacgcgctgtatattcttggcgatctcttcgaggcctggattggcgacgacgaccccaacccgctacatcgtgaaatggccgttgccattaaatcgctggttgattccggcgtcccctgcttctttattcatggtaatcgcgacttcctgattggcaaacgctttgcccgcgaaagcggcatgattctactgccgcaggaaaaagtgctcgacctgtatggccgcaatgtgttgattatgcacggcgatacgctctgtaccgatgatgccggatatcaggcgtttcgcgccaaagtccataatccgtgggtgcaacgactgttccttaccctgccgctgtttatccgccgccgtatcgccgccagaatgcgcgccggcagtaaagccgccaacagcagcaaatcgctggatattatggacgtcaatgcgcagaccgtcgtcgccgaaatggaaaaacaccgcgtacagtggctgattcacggtcacacccaccgcccggcggtgcatgaactttccgccaacgaccagcccgcattccgcgtggtgttaggcgcatggcatcatgaaggttcaatggtaaaagtcacgccggacaacgttgagttaatcgccttccccctgtaa

SEQ ID NO: 57 - DNA, 978 bp, synthetic construct
  source 1..978: mol_type = other DNA
ctagcgaaccagcgaggtgatatgttgaagcaacttatcaggctgctcaccggacaaacgcgcatcaaccggtaagaaccaccagttatcttcggcaaaagcacggcatttcaccgcgtctttttccgtcattaccagggtctgcccttcaccgaccaacgcctgaacgtcagcaggggcgagcgtttgatgatcggccagcgggacgcacttttgcggatgcgcgccacaggcttccagcgtggcgaaaaagcgcggcggatgaccgatgcccgccatcgccacaatattgctcagttgcgccacatcgcaacgcgctcccgtacgtaagttcaccgccagtccaggcgctagctgcatggggatttcgcccgcccgggcgacgccgccattcacgatagcggcgtctacggttttcaggcgactggcgcgttcgcgcataggaccggcaggaagccaccagccgttgccaaaacggcgcacgccgtcaatcaccacaatttcaatatctcgcgcgagtcggtaatgctgcaacccatcgtcggtgataataatctgcacattatgcgctgccagaatcgctttcaccgccgcggcgcgttcaggcgctaccgcgacaggcgcgccggtccgttgataaatcaataccggttcatctcccgcttctgcggttgtcgtctccggcgtcaggagcagcggataagcggcagctttcccgccgtagccgcgggaaacgacccccacgcgcacgccacgctgttgcagcttttccaccagccaaatgactacgggggttttaccgttaccgccagccgtaagattccctaccacaaccaccggtaccggcgctcgccaggcgcgtttaaaaccaagcttatagctcagacgaatcgccccgctcaccaagccatacagccaggagagcggcagcagtaaccgccatagcggggattcacccgaccagatacgcgcaatcat

SEQ ID NO: 58 - DNA, 921 bp, synthetic construct
  source 1..921: mol_type = other DNA
atgacgaagttgcctaagttctccgtggccttactgcacccgcgctattggttaacctggttgggtataggcgcgctttggttggtcgtgcaactcccctacccggtcatctataaattgggttgcgcattgggccacctggcgcgacgcgtaatgaaacgccgcgcaaaaatcgcctatcgcaaccttgaattatgctttccggaaatgagcgcgcaggaacgccacaccatggtggtcaaaaactttgaatccgtcggtatgggcgtgatggaaaccggcatggcctggttctggcccgatcggcgagtgaaccgctggatggaagcgagcggtctggagcatatccgtgaagttaaggcgcagggactggggttcattctggtaggaatacatttccttacccttgagtttggcgcccgcatgtttggtatgcataacccgggtatcggagtttatcgcccgaatgataatccgttgctcgactggttacagacctggggacgcttacgctccaataaatcaatgttggatcgcaaagatctgaaaggcatggttaaggcattgaaaagcggcgaattgatctggtatgcgccggatcacgattatggcccgcgcgccagcgtttttgtaccattattcgctgtcgaccaggctgccacgacctccggtacctggatgctcgcgcgcatgtctaaagcctgtattatccccttcgtgcctcgccgtaaacccgatgggaaaggctacgaactgatcattcttcctgcggaatattcgcctccgctggagagcgcagaagcgactgccgcatggatgaataagattgttgagcagtgcattatgatggcgccagagcagtatatgtggctgcatcgccgctttaaaactcgccctgaaggcgtaccgtcgcgctattga

SEQ ID NO: 59 - DNA, 972 bp, synthetic construct
  source 1..972: mol_type = other DNA
atggaaaccaaaaaaaataatagtgagtatatccctgaattcgaaaaatcctttcgctatccacagtattggggcgcctggttgggcgcggcggcaatggcggggatcgcattaacaccggcatcattccgcgaccctttgctggcgacgctggggcgttttgccggacggctggggaagagttctcgtcgccgggcgctaattaatctgtcgttgtgctttccgcagcgtagcgaagctgagcgcgaagcgattgtcgatgagatgttcgccaccgcgccacaggcaatggcgatgatggctgagttggcgatgcgcggtccgaaaaaaattcaacagcgtgttgactgggaaggtctggagattatcgaggagatgcgtcgtaacgacgaaaaagtcatttttctcgtaccgcatggctggggcgtcgacattccagccatgctgatggcctctcaggggcaaaaaatggcggcgatgtttcataatcagggtaatccggtttttgactatatctggaacacagtgcgtcggcgtttcggcggacgtttgcatgcgcgtaatgacgggattaaaccctttattcagtctgttcgtcagggctactggggttactacctgccggaccaggatcacggcccggagcatagtgaattcgttgatttctttgcgacatacaaagcgacgctgcctgcaattggtcggctgatgaaagtgtgccgcgcacgcgtgataccgcttttcccggtgtataatggtaaaacgcatcgcctgactatccagattcgcccgccaatggacgatctgctcacggctgacgaccacactatcgccagacggatgaacgaagaggtcgaaatttttgtcggcccgcatccggaacagtacacctggatcctgaagctgctcaaaacccgcaagccaggcgagattcagccgtataagcgtaaagatctttatcccatcaaataa

SEQ ID NO: 60 - DNA, 909 bp, synthetic construct
  source 1..909: mol_type = other DNA
atgttcgcagcaatcattatcggtatttttattatcagcgtcatttatgcgcattcacgcggggtggaaaaacaaaaactttcccgtcagctctttgaccactcgacgtttatggcgccgatcaatatgttcatgactcgcttctcaacgttaccggcaaagcagccgtactttgataccacggcatttccagagctgcagaagctgacggaaaactggcaggtgattcgtgaagaggcactacagcttcagcatcacataaaagccgcgcaggccaataacgacgccggattcaatacctttttcaagcgcggctggaaacggttttaccttaaatggtattccgatgcccacccgtcggcggaaacgttatgcccgataacgacaaagctggtcaacagcatcccctctattaaagcggcgatgttcgccgagttgcctcccggggcctatctgggaaaacatcgcgacccctatgccggttcagtacgttaccatcttggattaagcacaccgaatgacgaccgctgttttattgaagttgatcgacagcgccatagctggcgcgacggcaaagccgtcatcttcgacgaaacctacgttcattgggcggaaaataaaactgagcagacgcgtattatcctcttttgcgatattgagcgcccaatgaaatggcgctgggcgcagagcgtaaaccactgggtcggcgcatcgttgatgtccgccgccagttcgccaaacgacgagaacgatcgcaccggtgcgattaatcgcatctttaaatacgttcacgcagcacgcgatgccgggcaacgtctgaaaaagaaaaaccgcactctctattacgcgctgaaatatctcgttattgctgctatttttgccgcgataatccttttcagcctcctctga

SEQ ID NO: 61 - DNA, 921 bp, synthetic construct
  source 1..921: mol_type = other DNA
tcagatgtagagtgacgcttcccccaacgggcgagtcttgaaacggcgatggatccagagatattgctccggggcgcgcatgatctctttctcaataattttattcatataggcagcggcttgattttcatctgccgggtaaccttccatttcaggggtaatatacagacgataacccgagttatcggatttccttaccattgtaacggtcaacatggcggcgccagacagcctggacagtacataggtgccgttggtggtggcgacgttttcaaccgcgaaaaatggcgcaaaggagctgcctttagggccgtagtcctggtcgggagcaaaccaaacggcttcccctttttttagcgcgcccacaatgccgcgcagattgtttctgccgatcatcgctttatttgagcgcatacgaccgcgcgtctgcacccactccatgagcggattgttatgcggacgataggtcgccatcatcggctggcagagacccattacccggcctcccaattccagcgacataaaatgcacgccaacgaccattacgccgcgattttgcgcctgcgcacgggtaaggttgtccagcccgtccacatcaaaccatttgcgaacccggctatcaggccagaaccaggccatgcccgtttcaagcagcgccatgccaagagagtggaaattctcggcgatcagtttttccctttcttcccgggagagggtcggaaaacagagttcaatatttttctgggcgattgactcacgtcgcttcaggaaggggcgcgccagtttaccggtgcgggtgcccagaaaacgcaaaaccgggtagggaagctgcaccagtaaccagaggatgccaacgccaaaccacgtcagccagtagcgcgggtgcaaaaacgcgcgtgaaaatttgctttgaggaaacat

SEQ ID NO: 62 - DNA, 720 bp, synthetic construct
  source 1..720: mol_type = other DNA
ttatttgtttaaaatttgtttatttccgcccgggagataattctcaaaaagcgctatcgcccggtcgctgagcggggtcatcagccaccaggggaggccaatcaaaataaccgtgagcgacccgaccacaatatcggtgaaccagtgagcgccaatcataacgcgcggaaacgcgaaaaccacaaatataataagggcgataatccccgcagttttgccgaaataacgcagcataaaggcggaaaatatcagcagcatcataccgtgatcgcctgggaaactgtcttttgacgcgtcttttgtcgggatgtgcagcaactcgctgacgcgataaatatgctcaaaagagagcgttgggctggcgcgcttgacggggatcagcgcctgaccgagttggttaagcaccaccgctgttagtagcatgaccaatccgattatcacaatgcgccgccggcccgatgcgttttcttttagccagaaactgagcatcagtccgcccatcgccagcagcgaacagccgtcaaacgcccgattattggtaatagcgacccaccagaggaacgcgtggctttccaccagtttctggttaaagaagtggaatatgccggaatcaatggtgaaccagaagccgtgattgacgggaagataccatgacaaaaacagcgccagaccggcggcattaagcagaattatcaaggaatagcgggttttcatcgtcat

SEQ ID NO: 63 - DNA, 1278 bp, synthetic construct
  source 1..1278: mol_type = other DNA
tcaatgcgttttcggtggcagataaggttccagcagttgcagcagacgctggagcgcgccctgattttgatacagcacttcaactgcgtgacgtccgtagaaattacgataatcagcgtcggtcagtaaagaggaaacttcttttgccagcgtagccgcatcggtaatcgtgataagtccgctcgcctgatccagacgggcgcaaatatctttaaagttaaaggtatgcggacccatcagtaccggaatcgcatgagcggcggcctccagcgggttatgaccgccgcgttcaaccagcgaaccaccaacaaaggcgagatcggcaatgccatagagcaacattaattcgcccatggtatcgcctaccacgacctgggtgctggcggacggtacttcgcccgaagaacgagtgatgtagcttaaccctgcctgacgcacaagattgatagcatccgggaaacgctccggatggcggggcaccagaatcagtaataaattcgggaattgatgtaataacgcctggtgagcggcgataacgatactctcttcgccatcgtgggtgctggtggcaatccagaccggacggtgcggcgcccactggcggcgtagcgtaacggctttagccgccagctgcggcgtaactgaaatatcaaatttcagactgccggtgaccgtgacctgattgttcttcgcgcccaatgccacaaagcgttcgccatcttcttcgttttgcgcggcaatcagggtgatacggcgcaagagcgtacggacaaacttgccaagcttcgcataacccgcggcggagcgggcggaaagccgcgcattagcgataaccaggggaatatgacgtttgtgcagcgcagcaatcagatttggccagagctcagtctccatgatcaataccagcttaggatcaatcttattgaggaaacgattgagcgcatcgggcaaatcataaggcaagtaaacgtgctgaacatcgttgccaaaggcggactggacgcgctccgagccggtcggcgtcatggtcgttacggtaataggcagatcgggatagcgatgacgtagagcgcggaccaatgggatggccgccagagtttcgcccaccgagacggaatgcagcatgattccgcccggtttcaacggacggcggtagaatccgtagcgttcaccccagcgcttacgataggccggcgctttacgtccacgcacccaaagccgtatccagatcagaggctgaataaggtagagaagagcggtgtaaagcaattcgagcat

SEQ ID NO: 64 - DNA, 1647 bp, synthetic construct
  source 1..1647: mol_type = other DNA
tcatttaggccgatactgaattaacaccagacgcccctgataatcaatattgtccgcagggggaagggaaagagcgctgatgtcttcatctttggctattgaaagtactagcgtaataatgccctcctgacgatgctggttgagccaggcgttaaaatcgtcggctttaacgaatttatcctgcacatcaggatagctaagaccatacctgagttcgcccgcgtgtccgtagagcataatatcgtctcgtttcagactccaggccagcccggcggcgacgcccacgttgtcggcaagaatatagcggcttgatgccaaaggcgcctgggtcatttcgacaaaaaactgtggctgtttggactccatcaccctgtcggggatggaaaagccgaacagcagcgccagtcccagcggacaaaacgcgggtaataggtatttttggctatgacagaggctataccagcccacaaacgcccaaacagtaaagacgccccagacgcaaaaaactttataggtttcgatatgcgtccacaccggcgatttcagcgggccccatgaggagacgacaaacgctgcgacgatcccgactaacccgaacaccaggttgatcccgccgttgacacgtagcgcggcgacgccttcttttacgttatgcaggacgaagcgcgccatgagtatcgctatcggtgcgaaacaggaaagaacataggtgggcagtttccctttcgcaatgctgaaaaagagaagcggcatgatcgtccatccgagcaaatagaatgcgccgtttcgctcgcgccagcccagtttaagcgcgccaggcagtaaccccagccacggtaaacttcccgcgagcagtaccggcagatagtaccagaaaggggccttatgctgggcatcgctcatggcgaatcgctggatatgctccacccagaaaaagtaatgccagaaatcggcttcgcgccgcgcaatggcgatcgcccagggaaggacaaccacaaagcagctcaagaccgccagccagccgtaaagcaaaaagtccttccagcgtttctggacaatgacccacggcagcacgctcaccacaggtacggccagggcgaggaagcctttagttaatacacccagaccgcaggttgcgcccagtagcaaaaacatcccaatcttgcccattcgggtcgtggcctgcatcccctgccagaaacaacacatcccggccgtaagccaaagggcgatcatcgggtcgagtaccgcatacgtcccgatactgtaaacggcaaagagggagagaaagataacggaggcgagcaacgcggtacgtttatcccgccataagcggaacgtcagccatgccaccagcgctgcggccagcaatgtcgttaaaatagcgccagcccgcacgccaaaattggtagcgccaaaaagccactgacccagactgtttatccagtaaccggctatcggtttttcaaaataacgtaatcccagaaaatgcggcacgatccagtcgccagacgccagcatctcccgacttatttcggcatagcgcgtttcatccggctgccagagcaggcggctgttgacaggaataacatagtagagcgcgataaacgcggcgaaagccagataatagcgtatcgatttcatcat

SEQ ID NO: 65 - DNA, 573 bp, synthetic construct
  source 1..573: mol_type = other DNA
tcaaaactggaaacgcatccaggcgaaatagacgtttccgttgttatacgaacccggaatgtaggtcatctgaaaggtagcgggaccatagcctatcgacgctaaaggcaacagcacagggatgggaatataattccagttgtcgcgcgcggtaacgcctgcggtaaagcccagtccaaggcgaaaattatcgtcttccagcggtcgccaggttttttcccagccataaccgcctatgggttcccatttgttaaatgaatctttaaaggccatcatatagaggccatgccagttgcctttgtcgtcccagcgggactgaccaaaaccaacgccccacggccgctcgttatagcgatccgttttctctttatcgtaggcaaagcgcgcatgccaggtaatggcggggacatacaaatcataatgctcaggctgtcgccacgtttctgcgacgttatcggtaaacgtgttaaacccccctttatccgccgcagagactgaaggaatagccagccatggcatcaaaaggagagcaataataagaaaatactttctgatgatcatcgcaacatacat

SEQ ID NO: 66 - DNA, 1644 bp, synthetic construct
  source 1..1644: mol_type = other DNA
atgttaaagcgctttcttaaaagacctgttcttgggcaaatcgcctggcttctgcttttttccttttatattgccgtctgcctgaacattgcgttctacaagcaggtactacaagacctaccgttaaactcgctgcgcaatgtgctggtgtttatttccatgccggtcgtcgcgtttagcgtggtcaatagtgtgctgacgctggcctcatttatttggctaaaccgactgctggcctgcgtttttattctggtcggcgctgccgcgcagtattttattttgacttacggcatcatcatcgatcgctccatgatcgccaatatgatggataccacgcccgcggaaacctttgcgctgatgacgccgcaaatggtgctgacgctgggattaagcggcgttctggcagccgtgattgccttctgggtcaaaatccgtccggcgacgccgcgcttacgtagcgggctttaccgcctggccagcgtcctgatctctattttattagttattctggtcgccgcctttttctataaagattacgcctcgttatttcgaaataataaacagttgatcaaagcattaagcccatcgaacagtattgtcgccagttggtcatggtattcacatcaacggctggcgaatttgccgctggtacgcattggcgaggatgcccatcgcaatccattaatgctgaaaggcgatcgcaaaaacctgacgattctcatcgttggcgaaacctcgcgcggcgatgatttctctcttggcggctatccgcgcgacaccaatccgcggctggcgaaagacgatgtgatctacttcccgcataccacctcttgcggtacggcgaccgcgatctccgttccctgcatgttttctgatatgccgcgcaaacattatgacgaagagctggcgcatcaccaggaagggctgctggatattatccagcgcgcggggattaacgtactgtggaatgataatgacggcggctgtaaaggcgcatgcgatcgcgttccgcatcaaaatgtcaccgagctaaacctgcccggacaatgtatcgacggcgagtgctacgatgaagtgttatttcacggtctggaagactatatcgaccatttgaaaggcgatggcgttattgtattacataccatcggcagccacggcccaacctattacaaccgttatccaccgcagtttaaaaaatttaccccaacctgtgacactaacgaaattcagaactgttcccaagagcagttgatcaacacctatgataataccgtgctgtacgtggactatattgtagataaagccattaacctgctgaaatctcatcaggataaattcaccaccagcctggtctatctttccgatcacggcgaatcattgggtgaaaatggcgtttatttacacggtttgccgtattccattgcgccggatacgcaaaaacatgtcccgatgctcatttggctttctaaagattatcaacagcgttatcaggtggatcaggcctgcctgcaaaaacgggcgagcacgctggattattcacaggacaatcttttctcaaccatgctgggattaaccggcgtacaaacgacgtattaccaggccgcagatgatattctgcaaccgtgcaggagactaagcgaatga

SEQ ID NO: 67 - DNA, 1692 bp, synthetic construct
  source 1..1692: mol_type = other DNA
atgagatacattaaatcgatgacgcaacagaaacttagtttcttgcttgcgctctatatcggtctgtttatgaattgcgccgtgttttaccgccgtttcggcagttatgcacaagaatttaccatttggaaaggcctctccgcagttgtcgaactgggcgccacggtgctggtcactttcttcttacttcgtcttctttcactgtttggccgacgcgtctggcgtgtgctggccacgctggtggtgctgttttccgctggcgccagttattacatgaccttcctgaacgtggtgattggctacggcattattgcgtctgttatgaccaccgatatcgatctctcgaaagaggtggtggggctgcactttgtattgtggctgattgccgtgagcgtgcttccgctcatctttatctggagtaaccactgtcgctacacgttgttgcgccagctacgtacgccggggcagcgttttcgcagcgccgctgtagtggtactcgcaggcgtaatggtgtgggcgcctattcgcctgctggatatacagcaaaaaaaggttgaacgggcgacaggcatcgacttacccagctatggcggcgtggtggcgaactcctacctgccctcaaactggttatctgcgttagggctgtatgcctgggcgcaggtagatgagtcgtcggacaataattcgttaataaacccggccaggaaatttacctatgttgcgccgaaagatggggatgacacctacgtcgttttcattatcggtgagacgacccgttgggatcacatggggattttcggctacgagcgtaataccacgccgaagctggcgcaggaaaaaaatctggcggcgttccgcggctattcctgcgataccgcgacgaagctttctttacgctgtatgtttgtacgggaaggcggggcggataataacccgcagcgtaccttaaaagagcagaatgtttttgccgtactcaaacagctcggattcagttccgatctgtacgccatgcagagcgagatgtggttctatagcaataccatggcggataatatctcttaccgcgagcagattggcgccgagccgcgtaaccgcggtaaaacggtggatgacatgctgttgattgatgagatgcagaactcgcttgcccagaatccggagggtaagcatctgattatcctgcataccaagggatcgcattttaactatacgcagcgttatccgcgcagctacgctcagtggaagcccgaatgtattggggtcgatagcggctgcacgaaagcgcagatgatcaactcttacgataactccgtgacctatgtggatcactttattaccagtgtgttcgatcagctacgtgataaaaaagcgattgtgttctacgcggctgaccacggcgagtcgattaacgaacgcgaacatttgcacggtacgccgcgcaatatggcgccgccggagcaattccgtgttccgatgctggtatggatgtcggataaatatcttgccagtccgcaacatgcgcagatgttcgctcacctgaaacagcaggcggagatcaaagtgccgcgtcgtcatgtggagctatacgatacgataatgggctgcctggggtatacatcgccgaatggcggcattaaccagaacaacaactggtgccatattcccgatgtgcagaaagtcgccgcgaagtag

SEQ ID NO: 68 - DNA, 855 bp, synthetic construct
  source 1..855: mol_type = other DNA
atgaaacaaaaagtggttaacattggcgacattaaggtggcaaatgacctgccgtttgtgctgtttggcggtatgaacgtgctggagtcacgcgatctggcaatgcgcatttgtgagcactacgtaaccgttacccagaagctgggtattccttacgtgttcaaggcctcttttgataaagccaaccgttcctctattcactcttaccgtgggccgggtctggaagaagggatgaaaatcttccaggaactcaagcagacatttggcgtaaaagtgatcactgacgtccatgaagccagccaggcgcagcctgttgctgatgtggttgacgtgattcagctcccggcgtttctggcgcgccagaccgacctggtggaagcgatggcgaaaaccggcgctgtgattaacgtgaaaaagccgcagttcgtaagcccgggtcagatgggcaatattgtggataagttccatgagggcggtaacgataaggtgattctgtgcgaccgcggcgcgaacttcggctatgacaacctggtggtggatatgctgggctttagcgtgatgaaaaaggtctccggcaactcgccagtgattttcgacgtcacccacgcgctgcaatgccgcgacccatttggcgccgcctctggcggtcgtcgtggtcaggtgaccgagctggcgcgcgccggtatggctgtcggtctggcgggcctgttcctggagtcgcatccggacccggctaacgcgaagtgcgacggtccttccgcgctgccgctggcgaaactggagcagttcctgacccagataaaagcgattgatgatttggtgaaaagcttcgacgagctggataccgagaactga

SEQ ID NO: 69 - DNA, 747 bp, synthetic construct
  source 1..747: mol_type = other DNA
ttaacgcatttcagcgcgcacgcgctccaggtcgtcggcggtgtctacgcccgtgccgggcaccgctttggcgacggcgacatgaattttttcgccgtaccacagcacacggagttgctccagcatttcaatatgttccagcgggctgggttgccagctcacgtaacggcggataaaccccgcgcgatagccataaatgcccaggtgacgaaggcaagtatcccctaccgtttccagactttttgcaaagcgatcgcgatcccagggaatcgtcgcccgggaaaagtaaagcgcatagccttcagcatccagcacgacttttaccgcattcgggttaaacgcttcttcggcgctgtgaatcggcaccgccagcgtcgccatgccaacctggcgctgcgccagattttccgcgacctggcgaataataaccgccgggatcatcggctcatcgccctgaacgttcacaataacggtatcgtcgctgaatccgcacttctctaccacttccgccaaccgttcggtgccggactggtgatcggcgcgcgtcatgcacacttcgccgccagccgcttctaccgcacgagccacgtcttcatgatcggtcgcgacaataatgcgttccgcgccagattcgcgcgcccgctccaggacatgaacaatcatgggcttaccattaatatccactaatggtttgcctggcagtcgggtagatgaaaaacgggccggaatgatgacgacgaaactcat

SEQ ID NO: 70 - DNA, 567 bp, synthetic construct
  source 1..567: mol_type = other DNA
tcatatcgattgccctttggcctcatccagcttgccctgcgccagcagcagcaaatcgcacacctcacgtaccgcgccgcgcccgccggcaatgtgcgtcacatagtcagcgcgggggatcagcagtggatgcgcatccgcaacggcaacgcttaaccccactttttccatcactggccagtcaatcagatcatcgccgacataggcaacattttccggcgcaatggccagtttttccagcagatcgctaaaggcgatcaacttattcgactgtccctgataaagatggacaatccccagcgtggcgcagcgatcttctacaagtttagcctttcgtccggtaataatggcaacctcgatattggaggtcaaagcacagcgaataccatagccgtcacgaacgttgaaagccttcagctcttcgccgttattgcccatataaatcaggccgtcagacaatacgccatccacgtccaggatgagcaggcggatattctccgctttggtcatgacatgggggctgacggggccataacaggtcggaagcgacgcacctgctttactcat

SEQ ID NO: 71 - DNA, 987 bp, synthetic construct
  source 1..987: mol_type = other DNA
ctacacgacgcctgcacgcaggagatcatgcatatgtaacacaccgagtaactggtcgccatcagcaaccagtacggaggtgatatggcgggactgcattaaattcagcgcatcgacagcgagaataccgggacgcacgcgaatgccccctggcgtcatcacctcggcgatccccaactggcgcatatcgccgcccatatcgaatacgcgacgtaaatcgccgtcggtgaagataccgtcgatcttcatggattcatcgcaaatgacggtcataccgagatttttacgcgtaatttctaatagcgcatcacgcagggtggcatgtttattaacatgcgggatctcatcgccagtatgcataatatcgcttacgcgcagcagtagcttacgtcccagcgcgccgccaggatgcgacagagcgaaatcctcggcggtaaagccgcgcgcttttaacaacgccacagcgagcgcgtcgcccatcaccagcgttgcggtggtactactggtaggcgccagtcctaacggacacgcttctttgggcactttaacacacagatgcacatctgccgcacgcgccatgctgctttccggtcgcccggtaatgcaaattaacggcacgtgcagacgtttaagtaccggtattagcgccgcgatctcgctggattcgccggagttggagatagcgataaccacatcctgcggcgtaaccatccccaaatcgccgtgcgcggcttcgcccggatgtacaaaaaaggaagaggtgccggtactggcgaacgtggcggccattttccgtccgatatggccggatttccccatccccatgaccaccacttttccggtgcagttgaacattttttcacaggccagcgtgaaatgctggttgatatattgatcaagctccgccaggccttcacgttcaatttccaggacctctttgcctgcctgctgaaagtcaaaccccggttgcaacgctaaatgcgacat

SEQ ID NO: 72 - DNA, 987 bp, synthetic construct; identical to SEQ ID NO: 71
  source 1..987: mol_type = other DNA

SEQ ID NO: 73 - DNA, 1224 bp, synthetic construct
  source 1..1224: mol_type = other DNA
atgcttataatttcatacattgcattatgcttattatttatagtttatctctatactctttccgtaagaattgaggggaaaataataaatgtaatggtcccatacctgataataacagtccctacactgtacgtgtttgaaggtatatttgtatacctctcagaggtgcggaattatacagtggaatatttgtttttctatacttgctatataacatacatagcatcatttgttatttcttatctttacacacaaagaaaacccatatacaacaaatcaaacacgaaaaataaaccaaggtatgtgtttacttcattgttattcaccttccttgcttttatcatttaccttccagtgttgatggagttcagagagtatatacttagcccaagaagaatatacgaattaaccagaacagggtatggtatatacttctatccttcattaatgttttctcttgtcgcttctatttgcgcgttctttacatacaaaaaatcaaagttattttgtatttccatagttttatttaactgtatacttattttcttgcatggtaacaaaggaccaatatttagtatatttatagcattcatcctttacctttcatatattgaaaataaaaaaattaaatttatgttcctggtaaaatcgtttgctgttatagcagtcattgtaacggcattctttgcatatacgtttactgatgggaatccgatagaaaatatggcgaattactcggattatacccgtaatgctgttcttgttgcttcctcaaactttgactttatgtacggaaaattactaatggaaagcgaggtttactcgaggattccgagggctatttggcctgataagcctgaagattttggcgcattgtatctggcaaaagtatttttccctgatgcattctacagaaatcagggcgctcctgctttcgggtatggtgaactatacgcagatttcgggctttttacaccagtttggttagttatatctggagtatttaaaggcgtcctagctaagtatttctccaataaaactcaggaaacaaagtcagcgcattatttcataatgttcctattttgcattggaataagtgtgattcctgttagcatgggatggttgttccctgagcatttgatgattgcttttatggtatacattgcatcttcctttgttttttcagagcatataagattcgttttactaagaaacaataaataa

SEQ ID NO: 74 - DNA, 1251 bp, synthetic construct
  source 1..1251: mol_type = other DNA
tcatgctcgcctacgccagagtaaaaatacgccgcaacaaagtgaaaaatagacaatataggtggccatataagcctgtgccgcacccagcgcgccgtgagcgggaatcagccagtgagcgaacgccgttaacagaatgaactggctaatttcagccagaatgtaaaatcgcaacgacgctttggcaatcaccagataaccgaaaacataggcgccgactttcagcacgtcgcccactaactgccaggcgaacagatcgcgcatcgcggtgaatttagcggaaaaaagcagccagatagcaaaatcgcgcagtagccagacggtaaaactcgccgccgcaaccgccggtaaaacaaatttcagcgcttttaccacttcacgcgtaatgtcctgtttttccgtcaggcgtgagagcgtgggtaacaggtaaacgctgaaggaggcggtgataaattgcagataggcgtcagaaatactgcttacgccctgccagatcccgacatcgctccagctatagtgcgcggccagttggtttcgcatcatcacataggcaaccggcatcgtaacggaggtaatcagcgccatcagggtaaatttactgagctgccctgccagaccgttgtcccaggagggcttgagatagcgtagcgggacggtgccgcgcttaatcagtattataccggctggcactaccaccagcgccggcaccagcgccaggccaagcagagcgccttcatagccgccgacacggtagcagagataccaggcggcgacgcccaaaaagctgccgacaattaacgataaggcattacccgacgcgtcacgaaagcccttcattagcgccagcagcaggttcgcccaggcgatccccatttgtaccagcgcaaccagacgcaccagcccttgatagtccgtatgaccgaacaatccctggctaatcggcgccgccgccagcaagaagaccagcgccagcagcgtagagaaccccaataccatcgcggaggaggttcccaccacggtacgtaactgcgccgggttatcatgatgttgtgcgacaagtttggtaacgccgttaaatatcccggcgccagccaatacgcccagcacggtaatcatctggcggaagttacccgcttgtccgacgcccgccggaccaaaagagacggccagtagtttcaccaccagcagtccggcgccaatttttaccagcgtactgaccgccgtccacagggaggctttagcaagcgacat

SEQ ID NO: 75 - DNA, 555 bp, synthetic construct
  source 1..555: mol_type = other DNA
ttagttactcttcttttgcgccggagtctggcctttgtttttgtcttgcaactgcgacggcaccagaacggtggtgacgcgtttgcctttctcgctgaaggcctgcattttctgctctttcaccaggtaggtgattttgtcgccggtaatgttgctgtcaagctgctccagataagcgttgccggtcagcaccacaaaatctttcgccagctcgtagtgcatatgggaagcgtggcctttcaccggcttaccgttgtcctgcatctggtagaaggtggccggattgccgtaaccgtcgatcacctctttcccctgttcgccgccagggcgggtaaccacgactttatcggcgttgatcttaatcgtgccctgggtcatcaccacgttgcccgtaaaggtcacgacgttgccttgcatatccagcgactgttgatccgagtcaatatgaataggctgttcggtatcgcccgtgacggcgaaagccggaatgctggcggccagcagcgagccggcaagcataagattaaggctgagtttgtttgttttgaatttcat

SEQ ID NO: 76 - DNA, 726 bp, synthetic construct
  source 1..726: mol_type = other DNA
tcagagtctgaagtcttccccaagatatacacgcttaacgtgttcgtcttgcaggatttctgtcggcgtaccgtgggcaataaggtggccctggctcacgatataggcgcgttcacagactgccagcgtctcacggacgttatgatcggtgatcagcacgccgagcccgctatcgcgcagatgctcgataatgcgtttgatgtcgataacggaaatcgggtcaacgccggcaaagggttcatccagcaggataaatttgggattagcggccaacgcgcgggctatttctacacgacggcgttcaccaccggacagcgcctgtcccatgctgtcgcgcagatgctcgatatgaaactcttccatcagctcgttggcgcggtcttctcgctgttctgcggtcaaatcgtcacgaatttgcagtaccgccatcaggttatcaaatacgctgagacggcggaaaatagaggcttcctgcggcaaatagccgataccgcggcgcgcgcgcgcgtgcagcggcagcagactgatatcttcatcatcgatgatgatattgcctgcgtcacgcggcacgataccgacgaccatataaaaggtggtggttttacccgcgccgtttggaccgagcagcccgacaatctccccggagttaacggtcagactgacatcttccactacgcgacggcctttataggccttcgccagattctttgcagttaatgttgccat

SEQ ID NO: 77 - DNA, 576 bp, synthetic construct
  source 1..576: mol_type = other DNA
ttaaggctgagtttgtttgttttgaatttcataagaggttctaaccttttcaatcagctcggcgttcttgctgcgtaagttaccgcgcattttcagtccgctggagttaaatgttgtgccgtataacgtcaccagatcgttcgaggtaacatcctgcgtcaccagattaatctgcgcgttatcggtggtaattctgcgtaattgagcgtcaggcaccagggcgttgacttcaacatggccatacagatagagcatccgatcgttagtcaatttggctttatcggccttgatcgaccatgtcggcactttatccttatcaaaggtggttaataccggttgcgtaaaccatgagaccgcctgatcggaaaaatattcaacgtgctgcgcgatcagacgatagctcaacgcgccttccggactgtacacgacggtatccgtatgctcgcttttatacgtgggatcgttgctgttgaccatcacggcagcaggatcgtctttatccgccagattgataccaatcagtaccagaatggccagcgacagtagaatgataacccaacgtctggttttactcat

SEQ ID NO: 78 - DNA, 2361 bp, synthetic construct
  source 1..2361: mol_type = other DNA
atgaaaaaacgtattcccactcttctggccaccatgatcgccagcgccctttatagtcatcaggggctggcagccgatctcgcctcacagtgtatgttgggcgtgccgagctacgatcgtcctctggtaaaaggcgataccaacgatctgccggttactatcaatgccgataacgctaaaggtaactacccggacgatgccgtttttaccggcaacgtggacattatgcaggggaatagccgcctgcaagcggatgaagtgcagcttcatcagaagcaggcggaaggtcagccggaacctgtacgcaccgtcgatgcgctgggtaatgtgcattatgatgacaatcaggtcatccttaaagggccgaagggctgggcgaacctgaacaccaaagacacgaacgtctgggaaggcgattaccagatggtgggccgtcaggggcgcggtaaagccgatctcatgaagcagcgcggcgaaaaccgctataccattctggaaaacggcagctttacctcctgtctgcctggctccgatacctggagcgtggtggggagtgaagtcatccatgaccgcgaagaacaggttgcggagatctggaacgcccggtttaaagtaggtccggttccgatcttttatagcccctatttacagctacccgtcggtgacaagcgtcgctcaggtttcctgatcccgaacgcgaaatacacgaccaagaactatttcgagttctacttaccgtattactggaacatcgcgcccaatatggacgccaccatcaccccgcactatatgcaccgccgcggcaatattatgtgggagaacgaattccgttatctcacgcaggcaggcgagggagtgatggaattagattatctgccttctgataaagtctacgaggacgatcaccccaaagagggcgataagcaccgctggttattcaactggcagcactcaggcgtgatggatcaggtgtggcgttttaacgtcgattacaccaaagtcagcgactccagctactttaacgatttcgacagtaagtacggttccagtaccgacggctacgcaacgcagaaattcagcgtcggctacgccgtacaaaactttgacgctacggtgtcgaccaaacaattccaggtctttaacgatcaaaacaccagcagctattcagcggagccgcagttagacgttaactactaccataacgatctcggcccgtttgatacccggatttacggccaggcggtgcactttgttaacaccaaagacaatatgccggaagcgacccgcgtccacctggagccaaccatcaatttgccgctctccaaccgctggggcagcctgaacaccgaagcgaagctgatggcgacgcactatcagcaaacgaatctggacagctataacagcgatccaaacaataaaaataagctggaagattcggttaaccgcgtcatgccgcagtttaaagtcgacggtaagctcatcttcgaacgcgatatggcgatgctggcgccggggtatacccagacgctggaaccacgcgtgcagtacctgtatgtgccgtaccgcgaccagagcggcatctataactacgattcttctttgctgcaatccgactataacggcctgttccgcgaccgcacttatggcggtctcgaccgtattgcttccgccaaccaggtcacaaccggcgtcacaacacgcatttatgatgatgccgccgttgaacgttttaacgtttctgttggtcaaatctactatttcacggagtctcgcaccggcgatgacaacattaaatgggagaatgacgacaaaaccggttcgctggtttgggcaggcgacacttactggcgtatttcagaacgctgggggctgcgtagcggagtgcagtacgatacccgtctggatagcgtcgctaccagcagcagcagcctcgaataccgtcgggatcaggatcgtctggtacagttgaactaccgctatgccagcccggaatatattcaggctacgttgccttcgtattattccacggcagagcagtataaaaacggcatcaatcaggtgggcgcggtggcaagttggccgattgccgatcgctggtcgattgtcggcgcgtactacttcgataccaattcgagcaaacctgcagaccagatgctcggcttgcagtacaactcttgctgctatgcgatccgcgtcggatacgaacgtaagctgaacggttgggataacgataaacaacacgcgatttatgataacgcgattggcttcaacattgagctgcgcggtttgagctctaactacggcctcggcacgcaagaaatgttgcgttcgaacattctgccgtaccaaagctctatgtaa

SEQ ID NO: 79 - DNA, 1083 bp, synthetic construct
  source 1..1083: mol_type = other DNA
ttacgacttacgcagcattagccagaggctaatcaggaagaaagacgcgctcggcagcagcgcgccgacaatcggcggaatgccgtataccagcgtcagcgggccaaaaatctggtcgagaacgtaaaagacgaagccgaagctaatccccgtcaccacgcgcacgcccatcggcacactacgcagcggtccaaagataaacgacagcgccatcagcatcatcaccgccacggagagcggctggaagattttactccacatattgagctgataacgtccggcgtcctgtccgctcgacttcagatatttaacgtagttatgcagaccgctgatggaaagcgcatccgggtccagcgccaccacgcctaacttatccggcgtcagattcgttttccaggtgccgctcaccgtctgcgaaccggtgatctgtttcgggttttgcagatcggactcatccacctgcgacaaacgccagaccttatgctccgggtcgaattttgccgaagcggcgtaacgcactgactgcaaacgacgctgatcgttgaaagcgtaaatactaatgccggccagctcctcgtcgcccttcacccgttcaatatagacaaagttattcccgtctttcgcccacagaccttgctgggtggaaagcagcgaaccgccatacatcgcctgcgcacgatagttacgcgccatctgctcgccctgcggggcgacccattcgccgatcgccatggttaacagcaccagggggatagccgttttcatcaccgacagcgccacctgcatacgggtgaaacccgatgcctgcatcaccaccagttcgctacgctgcgccagcatccccagtcccagcagcgcgccaagcagcgccgccataggaaagaagatctggatatccttaggtacgctgagcagggtgtacatacccgcgcccagcgcgtcgtagttaccctgccccgcttttttcagctgatcgacaaacttgatgatcccggagagcgacaccagcatgaacaacgtcatcatgatggtggtaaaaatggttttaccgatatagcggtcaagtacaccaaatggctgcat

SEQ ID NO: 80 - DNA, 69 bp, synthetic construct
  source 1..69: mol_type = other DNA
tcgctacactattcacaattccttttcgcgtcagcagaccctggaaaagctcgagttcatgtgcagctc

SEQ ID NO: 81 - DNA, 70 bp, synthetic construct
  source 1..70: mol_type = other DNA
aggtagtacagggtttgtcagcataaagcctctcttacgagaggctttattagatcctttacgcgttcgc

SEQ ID NO: 82 - DNA, 69 bp, synthetic construct
  source 1..69: mol_type = other DNA
aatacttgtaacgctacatggagattaactcaatctagagggtattaatatcgagttcatgtgcagctc

SEQ ID NO: 83 - DNA, 70 bp, synthetic construct
  source 1..70: mol_type = other DNA
cggacaaaaaaatggcgcacgatgtgcgccattttatattgtgcgtcaaatagatcctttacgcgttcgc

SEQ ID NO: 84 - DNA, 74 bp, synthetic construct
  source 1..74: mol_type = other DNA
tttatggctacactgtctccagcttcatcctttttttagttagggtatctatgattgaacaagatggattgcac

SEQ ID NO: 85 - DNA, 72 bp, synthetic construct
  source 1..72: mol_type = other DNA
ttaatgagaaattttacctgtcgtagccgaccaccatccggcaaagaagctcagaagaactcgtcaagaagg

SEQ ID NO: 86 - DNA, 74 bp, synthetic construct
  source 1..74: mol_type = other DNA
cttatttgcggatttttatattccagattcattgttttcaggaatgagaaatgattgaacaagatggattgcac

SEQ ID NO: 87 - DNA, 72 bp, synthetic construct
  source 1..72: mol_type = other DNA
agccagtagtatcatcgccgttttcggtaatatcttgagcatagtgttcatcagaagaactcgtcaagaagg

SEQ ID NO: 88 - DNA, 74 bp, synthetic construct
  source 1..74: mol_type = other DNA
gtaacgcattatactttaaggaaatgatatatgctgagagcacatacactatgattgaacaagatggattgcac

SEQ ID NO: 89 - DNA, 72 bp, synthetic construct
  source 1..72: mol_type = other DNA
agcgctcaccgcgcgtgcccccggtaatggttgtgtcatcgtatcctcattcagaagaactcgtcaagaagg

SEQ ID NO: 90 - DNA, 74 bp, synthetic construct
  source 1..74: mol_type = other DNA
ctatttaatatctaaagtctttagattaaggttttaactctggggtatatatgattgaacaagatggattgcac

SEQ ID NO: 91 - DNA, 72 bp, synthetic construct
  source 1..72: mol_type = other DNA
taaagtctgttgaatgacttcttcttcaaaatattttctgctcatagtgatcagaagaactcgtcaagaagg

SEQ ID NO: 92 - DNA, 74 bp, synthetic construct
  source 1..74: mol_type = other DNA
agagccacagtataaaggcagggtaaattaaggtttttctggtaatcgttatgattgaacaagatggattgcac

SEQ ID NO: 93 - DNA, 72 bp, synthetic construct
  source 1..72: mol_type = other DNA
gcaccagtggcaaggctgggggaaaatcgccgcgcctaaaaacgtgagcgtcagaagaactcgtcaagaagg

SEQ ID NO: 94 - DNA, 74 bp, synthetic construct
  source 1..74: mol_type = other DNA
tttaaaaattttaataatgcaatattctcgaaattacaaaagtgatcactatgattgaacaagatggattgcac

SEQ ID NO: 95 - DNA, 72 bp, synthetic construct
  source 1..72: mol_type = other DNA
ttcagctatttctatctcaggaaatgaatccattacatcacctatgggtttcagaagaactcgtcaagaagg

SEQ ID NO: 96 - DNA, 74 bp, synthetic construct
  source 1..74: mol_type = other DNA
atagcctactttaaacgtaaacttcttgaataaaacccataggtgatgtaatgattgaacaagatggattgcac

SEQ ID NO: 97 - DNA, 72 bp, synthetic construct
  source 1..72: mol_type = other DNA
agtttttaatctttttttcaataatcataatggagatttagggaggggaatcagaagaactcgtcaagaagg

SEQ ID NO: 98 - DNA, 74 bp, synthetic construct
  source 1..74: mol_type = other DNA
ttataacatttctttttctataaagttaactattctggattatagctattatgattgaacaagatggattgcac

SEQ ID NO: 99 - DNA, 72 bp, synthetic construct
  source 1..72: mol_type = other DNA
gcgctgatacttattacggtatcagcgcgttttccatcatcaggactcaatcagaagaactcgtcaagaagg

SEQ ID NO: 100 - DNA, 74 bp, synthetic construct
  source 1..74: mol_type = other DNA
agattcattaaagagactctgtctcatcccaaacctattgtggagaaaagatgattgaacaagatggattgcac

SEQ ID NO: 101 - DNA, 72 bp, synthetic construct
  source 1..72: mol_type = other DNA
cctgatgatggaaaacgcgctgataccgtaataagtatcagcgcgttttttcagaagaactcgtcaagaagg

SEQ ID NO: 102 - DNA, 74 bp, synthetic construct
  source 1..74: mol_type = other DNA
tttatacagcttaccggagaaggccgcggatattattacaggtgatttagatgattgaacaagatggattgcac

SEQ ID NO: 103 - DNA, 72 bp, synthetic construct
  source 1..72: mol_type = other DNA
ctatccttgtctcactcataaattactcactgagtgcataattattataatcagaagaactcgtcaagaagg

SEQ ID NO: 104 - DNA, 74 bp, synthetic construct
  source 1..74: mol_type = other DNA
gtgcttttttctgcttatttatccggacaatttcaaccaaagagtcgcttatgattgaacaagatggattgcac

SEQ ID NO: 105 - DNA, 72 bp, synthetic construct
  source 1..72: mol_type = other DNA
acgctgcagaccgccaaaaggaaaatatttatataagcaaaaggcaactctcagaagaactcgtcaagaagg

SEQ ID NO: 106 - DNA, 74 bp, synthetic construct
  source 1..74: mol_type = other DNA
ttgaatataacatttatttataggttgcatgataaacatacgagttttttatgattgaacaagatggattgcac

SEQ ID NO: 107 - DNA, 72 bp, synthetic construct
  source 1..72: mol_type = other DNA
aaaaaagaaatgcgtgccgaagcaacgaaaaataatgatttatctagtgttcagaagaactcgtcaagaagg

SEQ ID NO: 108 - DNA, 74 bp, synthetic construct
  source 1..74: mol_type = other DNA
taaggttcaggcgttacgtttggcgctacgattaaagacaggctctcattatgattgaacaagatggattgcac

SEQ ID NO: 109 - DNA, 72 bp, synthetic construct
  source 1..72: mol_type = other DNA
agaagcacgccaggcccgataagcgttagcgttatcgggcaacatacaggtcagaagaactcgtcaagaagg

SEQ ID NO: 110 - DNA, 74 bp, synthetic construct
  source 1..74: mol_type = other DNA
atccggtacactgcatactgtcatttacattcatgctgaaggatatcctcatgattgaacaagatggattgcac

SEQ ID NO: 111 - DNA, 72 bp, synthetic construct
  source 1..72: mol_type = other DNA
gtttctgagcgcaaccaacgcacctgcagcttgaagtatgacgggtatagtcagaagaactcgtcaagaagg

SEQ ID NO: 112 - DNA, 74 bp, synthetic construct
  source 1..74: mol_type = other DNA
ctgaaacatgcgatactagcgccacttgctttactcaggagctataaaagatgattgaacaagatggattgcac

SEQ ID NO: 113 - DNA, 72 bp, synthetic construct
  source 1..72: mol_type = other DNA
agcggaaaaatgcatttttgttttaaccgctcatcttttatccataacgctcagaagaactcgtcaagaagg

SEQ ID NO: 114 - DNA, 74 bp, synthetic construct
  source 1..74: mol_type = other DNA
tgaattatgctattatcgcgcgcaaattttgaatctctcaggagacaggaatgattgaacaagatggattgcac

SEQ ID NO: 115 - DNA, 72 bp, synthetic construct
  source 1..72: mol_type = other DNA
cgccttcaaaatcagcgcccgccgcgtctgtaacgcctgatgacgcggtttcagaagaactcgtcaagaagg

SEQ ID NO: 116 - DNA, 74 bp, synthetic construct
  source 1..74: mol_type = other DNA
gcattcatgtctgagacagtctctgacaccataattcaaaggttacagttatgattgaacaagatggattgcac

SEQ ID NO: 117 - DNA, 72 bp, synthetic construct
  source 1..72: mol_type = other DNA
catcatcatgtcgcccacccaggacgggccaatgaccaaaattttcatactcagaagaactcgtcaagaagg

SEQ ID NO: 118 - DNA, 74 bp, synthetic construct
  source 1..74: mol_type = other DNA
gaaaacttcatcacctctccagattacatctgaatatgaggacaagagaaatgattgaacaagatggattgcac

SEQ ID NO: 119 - DNA, 72 bp, synthetic construct
  source 1..72: mol_type = other DNA
agcaaaaagtcgtcatcggccggttatgaccgatgacatcccgatgtggttcagaagaactcgtcaagaagg

SEQ ID NO: 120 - DNA, 72 bp, synthetic construct
  source 1..72: mol_type = other DNA
gaatattatgacaatgcgaaatgccaaaataaaaggccttgcggcctttttcagaagaactcgtcaagaagg

SEQ ID NO: 121 - DNA, 74 bp, synthetic construct
  source 1..74: mol_type = other DNA
ataatgactcttctgcgatacattattttcgtatctacagaaggtattttatgattgaacaagatggattgcac

SEQ ID NO: 122 - DNA, 72 bp, synthetic construct
  source 1..72: mol_type = other DNA
gagctgaccgccaacgctgagcagactggcaagcaccagaacgacgccgatcagaagaactcgtcaagaagg

SEQ ID NO: 123 - DNA, 74 bp, synthetic construct
  source 1..74: mol_type = other DNA
atccctggccgtgaaggttggctggggtgtcaacaggcagcgagcgcctcatgattgaacaagatggattgcac

SEQ ID NO: 124 - DNA, 74 bp, synthetic construct
  source 1..74: mol_type = other DNA
taattttactttgtcacgattagcgtcaccgaatcgatggacgcatcaacatgattgaacaagatggattgcac

SEQ ID NO: 125 - DNA, 72 bp, synthetic construct
  source 1..72: mol_type = other DNA
gagtattaacccctgtaataatagcgtgtcgtcttcaacaatcagtatcttcagaagaactcgtcaagaagg

SEQ ID NO: 126 - DNA, 72 bp, synthetic construct
  source 1..72: mol_type = other DNA
taccagaatggccagcgacagtagaatgataacccaacgtctggttttactcagaagaactcgtcaagaagg

SEQ ID NO: 127 - DNA, 74 bp, synthetic construct
  source 1..74: mol_type = other DNA
catgatctcctgcgtgcaggcgtcgtgtagaaactcaaggataattaacgatgattgaacaagatggattgcac

SEQ ID NO: 128 - DNA, 72 bp, synthetic construct
  source 1..72: mol_type = other DNA
ggtcggaagcgacgcacctgctttactcatcgttaattatccttgagttttcagaagaactcgtcaagaagg

SEQ ID NO: 129 - DNA, 74 bp, synthetic construct
  source 1..74: mol_type = other DNA
gatgctctattggctatcgccacttcttgttggataactggaaacggattatgattgaacaagatggattgcac

SEQ ID NO: 130 - DNA, 72 bp, synthetic construct
  source 1..72: mol_type = other DNA
ggacgtttcaccggcgaccagggcaatcgttaaaggacgctgtgccgccatcagaagaactcgtcaagaagg

SEQ ID NO: 131 - DNA, 74 bp, synthetic construct
  source 1..74: mol_type = other DNA
tcgtgtgcgaagcaaccatgatgtgtgctcgtagccgggaggcctgattcatgattgaacaagatggattgcac

SEQ ID NO: 132 - DNA, 72 bp, synthetic construct
  source 1..72: mol_type = other DNA
ggagagagtgccaggttaaccagtcgaattttatacgacagcgtatgtcgtcagaagaactcgtcaagaagg

SEQ ID NO: 133 - DNA, 74 bp, synthetic construct
  source 1..74: mol_type = other DNA
cgaatgtatagtacacttcggttggataggtaatttggcgagattatacgatgattgaacaagatggattgcac

SEQ ID NO: 134 - DNA, 72 bp, synthetic construct
  source 1..72: mol_type = other DNA
tcgtatgaatgtgacaggccggaaaagaatggcaactacaaggcggaacgtcagaagaactcgtcaagaagg

SEQ ID NO: 135 - DNA, 74 bp, synthetic construct
  source 1..74: mol_type = other DNA
gcgatgtgaaagacatcaccgctgacgtactgaaacaggttaaataagtaatgattgaacaagatggattgcac

SEQ ID NO: 136 - DNA, 74 bp, synthetic construct
  source 1..74: mol_type = other DNA
gtaccaaaagaagacgtcatcattgaaaacgtgaccgtcagcgagtaatcatgattgaacaagatggattgcac

SEQ ID NO: 137 - DNA, 72 bp, synthetic construct
  source 1..72: mol_type = other DNA
ggcaaggaaaacggttgcgtgcgcgccgtaacggacgattcgacgaacattcagaagaactcgtcaagaagg

SEQ ID NO: 138 - DNA, 74 bp, synthetic construct
  source 1..74: mol_type = other DNA
ggttgcctgaaaatcccgggatgaggttttcttagaaggacagtgacgttatgattgaacaagatggattgcac

SEQ ID NO: 139 - DNA, 72 bp, synthetic construct
  source 1..72: mol_type = other DNA
cgccaggatagaacaggccgcggcaggcagttccataccgcggcccggcttcagaagaactcgtcaagaagg

SEQ ID NO: 140 - DNA, 72 bp, synthetic construct
  source 1..72: mol_type = other DNA
tcataccgcgctgttcatgaccgtctaagacgatcatgaacaggatcatgtcagaagaactcgtcaagaagg

SEQ ID NO: 141 - DNA, 74 bp, synthetic construct
  source 1..74: mol_type = other DNA
gtattgctggaaaatgaagctcgcgccctgacatctgatgagagtaaatcatgattgaacaagatggattgcac

SEQ ID NO: 142 - DNA, 74 bp, synthetic construct
  source 1..74: mol_type = other DNA
cttatgattattgctttaaagatgcgtatggaaaaacggagagctattcaatgattgaacaagatggattgcac

SEQ ID NO: 143 - DNA, 72 bp, synthetic construct
  source 1..72: mol_type = other DNA
ggccaaagcgaccctgcattatatgtgggaataattaatgttattttcattcagaagaactcgtcaagaagg

SEQ ID NO: 144 - DNA, 74 bp, synthetic construct
  source 1..74: mol_type = other DNA
ctgatatgcggattcatttattcaaagttcattgtctttagggatgcgaaatgattgaacaagatggattgcac

SEQ ID NO: 145 - DNA, 72 bp, synthetic construct
  source 1..72: mol_type = other DNA
acaccaacgagaaaactataaggatagcgattaccatttttaatctattgtcagaagaactcgtcaagaagg

SEQ ID NO: 146 - DNA, 74 bp, synthetic construct
  source 1..74: mol_type = other DNA
taatatgcctattttatttacattatgcacggtcagagggtgaggattaaatgattgaacaagatggattgcac

SEQ ID NO: 147 - DNA, 72 bp, synthetic construct
  source 1..72: mol_type = other DNA
ttttacgcaggctaatttatacaattattattcagtacttctcggtaagctcagaagaactcgtcaagaagg

SEQ ID NO: 148 - DNA, 72 bp, synthetic construct
  source 1..72: mol_type = other DNA
cggcagcagtaaccgccatagcggggattcacccgaccagatacgcgcaatcagaagaactcgtcaagaagg

SEQ ID NO: 149 - DNA, 74 bp, synthetic construct
  source 1..74: mol_type = other DNA
aggataacgggtagaatatgcggctatttcaacaaatgctggttttttgaatgattgaacaagatggattgcac

SEQ ID NO: 150 - DNA, 74 bp, synthetic construct
  source 1..74: mol_type = other DNA
tgcctgatggtaatatttttaatactaagcattttttctaaaggctctatatgattgaacaagatggattgcac

SEQ ID NO: 151 - DNA, 72 bp, synthetic construct
  source 1..72: mol_type = other DNA
atttttacgcttcagagccaaataaaacggcggcattgccgccgtataactcagaagaactcgtcaagaagg

SEQ ID NO: 152 - DNA, 72 bp, synthetic construct
  source 1..72: mol_type = other DNA
cctttataggccttcgccagattctttgcagttaatgttgccataacgaatcagaagaactcgtcaagaagg

SEQ ID NO: 153 - DNA, 74 bp, synthetic construct
  source 1..74: mol_type = other DNA
taacttacgcagcaagaacgccgagctgattgaaaaggttagaacctcttatgattgaacaagatggattgcac

SEQ ID NO: 154 - DNA, 72 bp, synthetic construct
  source 1..72: mol_type = other DNA
catattcagagtcgttttctcccgctagagcagcatagccctctaccctatcagaagaactcgtcaagaagg

SEQ ID NO: 155 - DNA, 74 bp, synthetic construct
  source 1..74: mol_type = other DNA
acaaaaacaaaggccagactccggcgcaaaagaagagtaactaattcgttatgattgaacaagatggattgcac

SEQ ID NO: 156 - DNA, 74 bp, synthetic construct
  source 1..74: mol_type = other DNA
accgtttgtcacgcgcaacgctaccgatgatggaacaataaatacaacgtatgattgaacaagatggattgcac

SEQ ID NO: 157 - DNA, 72 bp, synthetic construct
  source 1..72: mol_type = other DNA
ttttccatttcaattaaccgcaatgcggattacgttgtaaatcaatcagatcagaagaactcgtcaagaagg

SEQ ID NO: 158 - DNA, 72 bp, synthetic construct
  source 1..72: mol_type = other DNA
tcatggtaggcctgataagcgcagcgccatcaggcctacgattactgtgatcagaagaactcgtcaagaagg

SEQ ID NO: 159 - DNA, 74 bp, synthetic construct
  source 1..74: mol_type = other DNA
gtgccggtccgccgcctgcgtgcccgttttctgcgtaaaggagcggtataatgattgaacaagatggattgcac

SEQ ID NO: 160 - DNA, 18 bp, synthetic construct
  source 1..18: mol_type = other DNA
ggcgcgccgagtctcttc

SEQ ID NO: 161 - DNA, 21 bp, synthetic construct
  source 1..21: mol_type = other DNA
ctcactcaaaggcggtaatac

SEQ ID NO: 162 - DNA, 74 bp, synthetic construct
  source 1..74: mol_type = other DNA
cagcgggttctggaagagcttcattcgctgttgtcggaagagggcgtttaatgattgaacaagatggattgcac

SEQ ID NO: 163 - DNA, 72 bp, synthetic construct
  source 1..72: mol_type = other DNA
gtggttagcatcttttctccacaataggtttgggatgagacagagtctcttcagaagaactcgtcaagaagg

SEQ ID NO: 164 - DNA, 74 bp, synthetic construct
  source 1..74: mol_type = other DNA
gccgaaggcgtcacggagtatatggcctggctgaaccgcgacgcgtaagtatgattgaacaagatggattgcac

SEQ ID NO: 165 - DNA, 72 bp, synthetic construct
  source 1..72: mol_type = other DNA
ggtatgtaatacgtcgcccatcgatgatgttttaacgatcaaaacccgcatcagaagaactcgtcaagaagg

SEQ ID NO: 166 - DNA, 74 bp, synthetic construct
  source 1..74: mol_type = other DNA
gaaaaaatgctgccgcatgaggcacgcaccatagatttggacagcctgctatgattgaacaagatggattgcac

SEQ ID NO: 167 - DNA, 72 bp, synthetic construct
  source 1..72: mol_type = other DNA
cctcaaaagcatctttaccgcgccatagtgtggttaacggcgctttcagctcagaagaactcgtcaagaagg

SEQ ID NO: 168 - DNA, 74 bp, synthetic construct
  source 1..74: mol_type = other DNA
tctttatcgtaaacttttccacaaataattcccctccctaaatctccattatgattgaacaagatggattgcac

SEQ ID NO: 169 - DNA, 72 bp, synthetic construct
  source 1..72: mol_type = other DNA
caaataaaagtcagtcagccccttaaattaaaccaaacgtgctacattgatcagaagaactcgtcaagaagg

SEQ ID NO: 170 - DNA, 74 bp, synthetic construct
  source 1..74: mol_type = other DNA
caaaaagatgcgagaatacggggaattgttcgttgaaagacaggatagaaatgattgaacaagatggattgcac

SEQ ID NO: 171 - DNA, 72 bp, synthetic construct
  source 1..72: mol_type = other DNA
ttttaaagctaaaagaggggaaaaattgcagcctgacggctgcaatcctgtcagaagaactcgtcaagaagg

SEQ ID NO: 172 - DNA, 72 bp, synthetic construct
  source 1..72: mol_type = other DNA
taccttcaacgatgtaaaactatcgctgaaggtaatgttaattacataggtcagaagaactcgtcaagaagg

SEQ ID NO: 173 - DNA, 74 bp, synthetic construct
  source 1..74: mol_type = other DNA
cgtttagcgacgcacgcgtaaggttgccaccgtttaaaaactatggcgaaatgattgaacaagatggattgcac

SEQ ID NO: 174 - DNA, 72 bp, synthetic construct
  source 1..72: mol_type = other DNA
tattgttttttaagactttttaattcacaactgaagcatacccttccccatcagaagaactcgtcaagaagg

SEQ ID NO: 175 - DNA, 74 bp, synthetic construct
  source 1..74: mol_type = other DNA
attttattcaggttaatgttgttattatcacagtcgaatttttgaacggtatgattgaacaagatggattgcac

SEQ ID NO: 176 - DNA, 74 bp, synthetic construct
  source 1..74: mol_type = other DNA
aagaatcgttgtacaggtcgtttttatcccgattcccagggtttgtttgcatgattgaacaagatggattgcac

SEQ ID NO: 177 - DNA, 72 bp, synthetic construct
  source 1..72: mol_type = other DNA
tcccttagtcgcaaaatacaattcaatcggcgagaaagtcggcagacaactcagaagaactcgtcaagaagg

SEQ ID NO: 178 - DNA, 74 bp, synthetic construct
  source 1..74: mol_type = other DNA
tgttctacattaattaaccgacattttacctataagtgtaaggcgatcctatgattgaacaagatggattgcac

SEQ ID NO: 179 - DNA, 72 bp, synthetic construct
  source 1..72: mol_type = other DNA
aaaaaagccggatagtatcttatccggcctacacaagctaaaaaccgcaatcagaagaactcgtcaagaagg

SEQ ID NO: 180 - DNA, 72 bp, synthetic construct
  source 1..72: mol_type = other DNA
cacttcatccacacccgccactaaatgggtgtgtggataaacaaattcgatcagaagaactcgtcaagaagg

SEQ ID NO: 181 - DNA, 74 bp, synthetic construct
  source 1..74: mol_type = other DNA
aaggcgtttaccgagttctttgagcgttcaacgcgcggtccgattcgttaatgattgaacaagatggattgcac

SEQ ID NO: 182 - DNA, 72 bp, synthetic construct
  source 1..72: mol_type = other DNA
atgacattcatgactccataaattcatcactgccgctgcattgggggacgtcagaagaactcgtcaagaagg

SEQ ID NO: 183 - DNA, 74 bp, synthetic construct
  source 1..74: mol_type = other DNA
ctggcgcaacacggcgtttacgcccagctacataagatgcaatttggccaatgattgaacaagatggattgcac

SEQ ID NO: 184 - DNA, 72 bp, synthetic construct
  source 1..72: mol_type = other DNA
aatcggatcaaacgtacctggataaatcgcccgtttttgcatgacagtcctcagaagaactcgtcaagaagg

SEQ ID NO: 185 - DNA, 74 bp, synthetic construct
  source 1..74: mol_type = other DNA
caggctaaatacatagaatccccagcacatccataagtcagctatttactatgattgaacaagatggattgcac

SEQ ID NO: 186 - DNA, 74 bp, synthetic construct
  source 1..74: mol_type = other DNA
ttgataatatgaagcagatggttggcaattggttggcggaatcaaaataaatgattgaacaagatggattgcac

SEQ ID NO: 187 - DNA, 72 bp, synthetic construct
  source 1..72: mol_type = other DNA
cataaacggctacctgtgccgccagccataattacgggaagaaaagacattcagaagaactcgtcaagaagg

SEQ ID NO: 188 - DNA, 74 bp, synthetic construct
  source 1..74: mol_type = other DNA
ttgggggcttccactaacttacttaattaaggcaaataagggataatcatatgattgaacaagatggattgcac

SEQ ID NO: 189 - DNA, 72 bp, synthetic construct
  source 1..72: mol_type = other DNA
gaatccagaaaggttaaatctacatttaatctcaatataataacttactatcagaagaactcgtcaagaagg

SEQ ID NO: 190 - DNA, 72 bp, synthetic construct
  source 1..72: mol_type = other DNA
ggtgtggttatggtgagggatatccgatcccaggacgtgaatcagtacagtcagaagaactcgtcaagaagg

SEQ ID NO: 191 - DNA, 74 bp, synthetic construct
  source 1..74: mol_type = other DNA
cgtcgatcaacgaacggtgattactaccttgctaaattatttctcctgatatgattgaacaagatggattgcac

SEQ ID NO: 192 - DNA, 72 bp, synthetic construct
  source 1..72: mol_type = other DNA
cggcgaaagccggaatgctggcggccagcagcgagccggcaagcataagatcagaagaactcgtcaagaagg

SEQ ID NO: 193 - DNA, 74 bp, synthetic construct
  source 1..74: mol_type = other DNA
ttgctgctgctggcgcagggcaagctggatgaggccaaagggcaatcgatatgattgaacaagatggattgcac

SEQ ID NO: 194 - DNA, 70 bp, synthetic construct
  source 1..70: mol_type = other DNA
tcgctacactattcacaattccttttcgcgtcagcagaccctggaaaagccgaagaaaggcccacccgtg

SEQ ID NO: 195 - DNA, 75 bp, synthetic construct
  source 1..75: mol_type = other DNA
aggtagtacagggtttgtcagcataaagcctctcttacgagaggctttatatttgtcctactcaggagagcgttc

SEQ ID NO: 196 - DNA, 70 bp, synthetic construct
  source 1..70: mol_type = other DNA
aatacttgtaacgctacatggagattaactcaatctagagggtattaatacgaagaaaggcccacccgtg

SEQ ID NO: 197 - DNA, 75 bp, synthetic construct
  source 1..75: mol_type = other DNA
cggacaaaaaaatggcgcacgatgtgcgccattttatattgtgcgtcaaaatttgtcctactcaggagagcgttc

SEQ ID NO: 198 - DNA, 19 bp, synthetic construct
  source 1..19: mol_type = other DNA
cgttccacagtatgatgcg

SEQ ID NO: 199 - DNA, 19 bp, synthetic construct
  source 1..19: mol_type = other DNA
cggttcaaccaataccacg

SEQ ID NO: 200 - DNA, 23 bp, synthetic construct
  source 1..23: mol_type = other DNA
cctgatgagcttactcaagtaag

SEQ ID NO: 201 - DNA, 21 bp, synthetic construct
  source 1..21: mol_type = other DNA
cacagaaaccgactggaatac

SEQ ID NO: 202 - DNA, 20 bp, synthetic construct
  source 1..20: mol_type = other DNA
cttttgtcctctgggcgaac

SEQ ID NO: 203 - DNA, 21 bp, synthetic construct
  source 1..21: mol_type = other DNA
cggttctgagtgctaaatcaa

SEQ ID NO: 204 - DNA, 20 bp, synthetic construct
  source 1..20: mol_type = other DNA
cagactccagactatgctcg

SEQ ID NO: 205 - DNA, 21 bp, synthetic construct
  source 1..21: mol_type = other DNA
cattgagcagggtttctgaat

SEQ ID NO: 206 - DNA, 22 bp, synthetic construct
  source 1..22: mol_type = other DNA
catatttcgttctctaccggac

SEQ ID NO: 207 - DNA, 21 bp, synthetic construct
  source 1..21: mol_type = other DNA
catatcacctccgtactggtt

SEQ ID NO: 208 - DNA, 22 bp, synthetic construct
  source 1..22: mol_type = other DNA
cgtgattatagcgtgatgttgc

SEQ ID NO: 209 - DNA, 24 bp, synthetic construct
  source 1..24: mol_type = other DNA
cgacatagttgttaaatcgggaaa

SEQ ID NO: 210 - DNA, 25 bp, synthetic construct
  source 1..25: mol_type = other DNA
catctttatgaggaagttgtctacc

SEQ ID NO: 211 - DNA, 22 bp, synthetic construct
  source 1..22: mol_type = other DNA
ctgcttgagaatcgagataagt

SEQ ID NO: 212 - DNA, 21 bp, synthetic construct
  source 1..21: mol_type = other DNA
ctcaatgagatgggggattac

SEQ ID NO: 213 - DNA, 20 bp, synthetic construct
  source 1..20: mol_type = other DNA
ctaccgtacaatcatgtgcg

SEQ ID NO: 214 - DNA, 20 bp, synthetic construct
  source 1..20: mol_type = other DNA
cgggctgacataatgaatgg

SEQ ID NO: 215 - DNA, 19 bp, synthetic construct
  source 1..19: mol_type = other DNA
cagcattcaggtgctcaac

SEQ ID NO: 216 - DNA, 22 bp, synthetic construct
  source 1..22: mol_type = other DNA
cgtagtatctaaaatttgcgcc

SEQ ID NO: 217 - DNA, 19 bp, synthetic construct
  source 1..19: mol_type = other DNA
caacacattgcggccatac

SEQ ID NO: 218 - DNA, 23 bp, synthetic construct
  source 1..23: mol_type = other DNA
catcgtcggtgataataatctgc

SEQ ID NO: 219 - DNA, 24 bp, synthetic construct
  source 1..24: mol_type = other DNA
cttgaaaaaggtattgaatccggc

SEQ ID NO: 220 - DNA, 21 bp, synthetic construct
  source 1..21: mol_type = other DNA
caagtaaacgtgctgaacatc

SEQ ID NO: 221 - DNA, 20 bp, synthetic construct
  source 1..20: mol_type = other DNA
cgcacttctctaccacttcc

SEQ ID NO: 222 - DNA, 21 bp, synthetic construct
  source 1..21: mol_type = other DNA
caaggtgagatgacaggagat

SEQ ID NO: 223 - DNA, 20 bp, synthetic construct
  source 1..20: mol_type = other DNA
ctgttgcaggatcaggatct

SEQ ID NO: 224 - DNA, 21 bp, synthetic construct
  source 1..21: mol_type = other DNA
ctataatcctgccactccatg

SEQ ID NO: 225 - DNA, 21 bp, synthetic construct
  source 1..21: mol_type = other DNA
cagagtaacaccatgcacaat

SEQ ID NO: 226 - DNA, 20 bp, synthetic construct
  source 1..20: mol_type = other DNA
caatagagacaccacagcca

SEQ ID NO: 227 - DNA, 22 bp, synthetic construct
  source 1..22: mol_type = other DNA
cattacgggttatcacaaagtg

SEQ ID NO: 228 - DNA, 20 bp, synthetic construct
  source 1..20: mol_type = other DNA
cgacaaaccctttaagaccg

SEQ ID NO: 229 - DNA, 20 bp, synthetic construct
  source 1..20: mol_type = other DNA
caggaagtagcttttaccgt

SEQ ID NO: 230 - DNA, 20 bp, synthetic construct
  source 1..20: mol_type = other DNA
cgagagcattacgcaaagtt

SEQ ID NO: 231 - DNA, 22 bp, synthetic construct
  source 1..22: mol_type = other DNA
catcaacgccataagaaatgtt

SEQ ID NO: 232 - DNA, 28 bp, synthetic construct
  source 1..28: mol_type = other DNA
ccgtagtctgtattaatcaatacaactt

SEQ ID NO: 233 - DNA, 24 bp, synthetic construct
  source 1..24: mol_type = other DNA
cgatattgctcaaattggtatcat

SEQ ID NO: 234 - DNA, 22 bp, synthetic construct
  source 1..22: mol_type = other DNA
ctgggttaattggaggttatgg

SEQ ID NO: 235 - DNA, 23 bp, synthetic construct
  source 1..23: mol_type = other DNA
ccagtcttcttccaaaaaaatca

SEQ ID NO: 236 - DNA, 24 bp, synthetic construct
  source 1..24: mol_type = other DNA
catgactgagtataaacacgaacc

SEQ ID NO: 237 - DNA, 20 bp, synthetic construct
  source 1..20: mol_type = other DNA
cagaacatcggcgtgagtta

SEQ ID NO: 238 - DNA, 21 bp, synthetic construct
  source 1..21: mol_type = other DNA
cggtattgatagtcgttttgc

SEQ ID NO: 239 - DNA, 21 bp, synthetic construct
  source 1..21: mol_type = other DNA
cgtgatacatgataatcccct

SEQ ID NO: 240 - DNA, 22 bp, synthetic construct
  source 1..22: mol_type = other DNA
ctgaccacttgtgatgattagg

SEQ ID NO: 241 - DNA, 20 bp, synthetic construct
  source 1..20: mol_type = other DNA
cgtaatgaaatgagcggagg

SEQ ID NO: 242 - DNA, 24 bp, synthetic construct
  source 1..24: mol_type = other DNA
cagcttactaacagacaatcagag

SEQ ID NO: 243 - DNA, 22 bp, synthetic construct
  source 1..22: mol_type = other DNA
cttctttaaacaatccttccgc

SEQ ID NO: 244 - DNA, 22 bp, synthetic construct
  source 1..22: mol_type = other DNA
cgctttatagtattttgcagca

SEQ ID NO: 245 - DNA, 21 bp, synthetic construct
  source 1..21: mol_type = other DNA
ctgcttaatcgcatccagaac

SEQ ID NO: 246 - DNA, 22 bp, synthetic construct
  source 1..22: mol_type = other DNA
ccatacgcatctttaaagcaat

SEQ ID NO: 247 - DNA, 19 bp, synthetic construct
  source 1..19: mol_type = other DNA
cgaaagctctcttagggca

SEQ ID NO: 248 - DNA, 21 bp, synthetic construct
  source 1..21: mol_type = other DNA
catggaagtcactttcgagaa

SEQ ID NO: 249 - DNA, 19 bp, synthetic construct
  source 1..19: mol_type = other DNA
cagtggtaaaacgctcgac

SEQ ID NO: 250 - DNA, 21 bp, synthetic construct
  source 1..21: mol_type = other DNA
ccggattatctggatatcccc

SEQ ID NO: 251 - DNA, 19 bp, synthetic construct
  source 1..19: mol_type = other DNA
cgaagaacgcaacaaactg

SEQ ID NO: 252 - DNA, 20 bp, synthetic construct
  source 1..20: mol_type = other DNA
catgcgtcttaaaactcctg

SEQ ID NO: 253 - DNA, 19 bp, synthetic construct
  source 1..19: mol_type = other DNA
ccttgatgaagctacgtcc

SEQ ID NO: 254 - DNA, 22 bp, synthetic construct
  source 1..22: mol_type = other DNA
catttattatggggagaaacgc

SEQ ID NO: 255 - DNA, 22 bp, synthetic construct
  source 1..22: mol_type = other DNA
cgcaaaaatgggaaaagtaatg

SEQ ID NO: 256 - DNA, 23 bp, synthetic construct
  source 1..23: mol_type = other DNA
caaactctggtataaccaggaac

SEQ ID NO: 257 - DNA, 22 bp, synthetic construct
  source 1..22: mol_type = other DNA
cattacatactcctgtcaggtg

SEQ ID NO: 258 - DNA, 20 bp, synthetic construct
  source 1..20: mol_type = other DNA
cagtggtttgatacacccca

SEQ ID NO: 259 - DNA, 20 bp, synthetic construct
  source 1..20: mol_type = other DNA
ctcagcaaacccaacaagct

SEQ ID NO: 260 - DNA, 20 bp, synthetic construct
  source 1..20: mol_type = other DNA
ctacaccacaaaagagagcg

SEQ ID NO: 261 - DNA, 21 bp, synthetic construct
  source 1..21: mol_type = other DNA
caggatgttacctcgaacgat

SEQ ID NO: 262 - DNA, 22 bp, synthetic construct
  source 1..22: mol_type = other DNA
ctggtgaaagagcagaaaatgc

SEQ ID NO: 263 - DNA, 20 bp, synthetic construct
  source 1..20: mol_type = other DNA
ctgactatgtgacgcacatt

SEQ ID NO: 264 - DNA, 20 bp, synthetic construct
  source 1..20: mol_type = other DNA
ctgcgactttatcgactacc

SEQ ID NO: 265 - DNA, 20 bp, synthetic construct
  source 1..20: mol_type = other DNA
cctgatctatctggcgttgg

SEQ ID NO: 266 - DNA, 18 bp, synthetic construct
  source 1..18: mol_type = other DNA
caagtaggccatcgcttg

SEQ ID NO: 267 - DNA, 21 bp, synthetic construct
  source 1..21: mol_type = other DNA
catacgatgaaggcgataagt

SEQ ID NO: 268 - DNA, 47 bp, synthetic construct
  source 1..47: mol_type = other DNA
gtcaagcgatggcctacttgatgaaaataacattaattattcccaca

SEQ ID NO: 269 - DNA, 46 bp, synthetic construct
  source 1..46: mol_type = other DNA
cttatcgccttcatcgtatgttattttatctcttttgacgaagaat

SEQ ID NO: 270 - DNA, 41 bp, synthetic construct
  source 1..41: mol_type = other DNA
gtcaagcgatggcctacttgtattttgattccgccaaccaa

SEQ ID NO: 271 - DNA, 43 bp, synthetic construct
  source 1..43: mol_type = other DNA
cttatcgccttcatcgtatgatgatcgtaaacctatcacgttt

SEQ ID NO: 272 - DNA, 46 bp, synthetic construct
  source 1..46: mol_type = other DNA
gtcaagcgatggcctacttgatgcttatatcattttgtattccaac

SEQ ID NO: 273 - DNA, 48 bp, synthetic construct
  source 1..48: mol_type = other DNA
cttatcgccttcatcgtatgctacttaattatccgtttagtaaaattc

SEQ ID NO: 274 - DNA, 44 bp, synthetic construct
  source 1..44: mol_type = other DNA
gtcaagcgatggcctacttgatgacagtggatagtaatacgtct

SEQ ID NO: 275 - DNA, 43 bp, synthetic construct
  source 1..43: mol_type = other DNA
cttatcgccttcatcgtatgttacaaggcttttggcttatagc

SEQ ID NO: 276 - DNA, 44 bp, synthetic construct
  source 1..44: mol_type = other DNA
gtcaagcgatggcctacttgatgaaaatttcattagtggttccc

SEQ ID NO: 277 - DNA, 50 bp, synthetic construct
  source 1..50: mol_type = other DNA
cttatcgccttcatcgtatgttattccatcattgtttttttgtttttcac

SEQ ID NO: 278 - DNA, 43 bp, synthetic construct
  source 1..43: mol_type = other DNA
gtcaagcgatggcctacttgatgaaaatctcgttagtcgttcc

SEQ ID NO: 279 - DNA, 47 bp, synthetic construct
  source 1..47: mol_type = other DNA
cttatcgccttcatcgtatgttaaccatttttcttctcattcttaat

SEQ ID NO: 280 - DNA, 53 bp, synthetic construct
  source 1..53: mol_type = other DNA
gtcaagcgatggcctacttgatggataatattgataataagtataatccacag

SEQ ID NO: 281 - DNA, 40 bp, synthetic construct
  source 1..40: mol_type = other DNA
cttatcgccttcatcgtatgttaatacgcaccatctcgcc

SEQ ID NO: 282 - DNA, 40 bp, synthetic construct
  source 1..40: mol_type = other DNA
gtcaagcgatggcctacttggtgaagttactcaccgcttt

SEQ ID NO: 283 - DNA, 41 bp, synthetic construct
  source 1..41: mol_type = other DNA
cttatcgccttcatcgtatgttacttggttaagtttggccg

SEQ ID NO: 284 - DNA, 44 bp, synthetic construct
  source 1..44: mol_type = other DNA
gtcaagcgatggcctacttgatgaaaatagcttttattggcgaa

SEQ ID NO: 285 - DNA, 42 bp, synthetic construct
  source 1..42: mol_type = other DNA
cttatcgccttcatcgtatgtcacttttgtaatttcgagaat

SEQ ID NO: 286 - DNA, 39 bp, synthetic construct
  source 1..39: mol_type = other DNA
gtcaagcgatggcctacttgatgcgggttttgatcgtta

SEQ ID NO: 287 - DNA, 46 bp, synthetic construct
  source 1..46: mol_type = other DNA
cttatcgccttcatcgtatgttaatgaatctttccaaatacgcttg

SEQ ID NO: 288 - DNA, 42 bp, synthetic construct
  source 1..42: mol_type = other DNA
gtcaagcgatggcctacttgatgaaaattttggtcattggcc

SEQ ID NO: 289 - DNA, 41 bp, synthetic construct
  source 1..41: mol_type = other DNA
cttatcgccttcatcgtatgttaaacgccctcttccgacaa

SEQ ID NO: 290 - DNA, 40 bp, synthetic construct
  source 1..40: mol_type = other DNA
gtcaagcgatggcctacttgatgagagttgccttttgctt

SEQ ID NO: 291 - DNA, 47 bp, synthetic construct
  source 1..47: mol_type = other DNA
cttatcgccttcatcgtatgtcaaccatctaaatcacctgtaataat

SEQ ID NO: 292 - DNA, 47 bp, synthetic construct
  source 1..47: mol_type = other DNA
gtcaagcgatggcctacttgatgaaaaatagtaaaaccaaagtgagt

SEQ ID NO: 293 - DNA, 39 bp, synthetic construct
  source 1..39: mol_type = other DNA
cttatcgccttcatcgtatgctaagacagattgagcgcc

SEQ ID NO: 294 - DNA, 46 bp, synthetic construct
  source 1..46: mol_type = other DNA
gtcaagcgatggcctacttgatgagcagaaaatattttgaagaaga

SEQ ID NO: 295 - DNA, 49 bp, synthetic construct
  source 1..49: mol_type = other DNA
cttatcgccttcatcgtatgttattcaagaagtttacgtttaaagtagg

SEQ ID NO: 296 - DNA, 46 bp, synthetic construct
  source 1..46: mol_type = other DNA
gtcaagcgatggcctacttgatggattcatttcctgagatagaaat

SEQ ID NO: 297 - DNA, 50 bp, synthetic construct
  source 1..50: mol_type = other DNA
cttatcgccttcatcgtatgttatttgtggaaaagtttacgataaagata

SEQ ID NO: 298 - DNA, 46 bp, synthetic construct
  source 1..46: mol_type = other DNA
gtcaagcgatggcctacttgatgattaaaaaaatcatatttactgt

SEQ ID NO: 299 - DNA, 47 bp, synthetic construct
  source 1..47: mol_type = other DNA
cttatcgccttcatcgtatgtcacttatcaaaccagtttttcatttg

SEQ ID NO: 300 - DNA, 42 bp, synthetic construct
  source 1..42: mol_type = other DNA
gtcaagcgatggcctacttgatgctaaccacatcattaacgt

SEQ ID NO: 301 - DNA, 42 bp, synthetic construct
  source 1..42: mol_type = other DNA
cttatcgccttcatcgtatgttatctatttcttagcgccagc

SEQ ID NO: 302 - DNA, 38 bp, synthetic construct
  source 1..38: mol_type = other DNA
gtcaagcgatggcctacttgatggttgagctgaaagcg

SEQ ID NO: 303 - DNA, 47 bp, synthetic construct
  source 1..47: mol_type = other DNA
cttatcgccttcatcgtatgttacagattttttcttattgtcctttc

SEQ ID NO: 304 - DNA, 40 bp, synthetic construct
  source 1..40: mol_type = other DNA
gtcaagcgatggcctacttggtggaaaagccatttcgaag

SEQ ID NO: 305 - DNA, 40 bp, synthetic construct
  source 1..40: mol_type = other DNA
cttatcgccttcatcgtatgtcatagcaggctgtccaaat

SEQ ID NO: 306 - DNA, 54 bp, synthetic construct
  source 1..54: mol_type = other DNA
gtcaagcgatggcctacttgatgattattgaaaaaaagattaaaaactataccg

SEQ ID NO: 307 - DNA, 39 bp, synthetic construct
  source 1..39: mol_type = other DNA
cttatcgccttcatcgtatgtcagcgtttttccttaccc

SEQ ID NO: 308 - DNA, 41 bp, synthetic construct
  source 1..41: mol_type = other DNA
gtcaagcgatggcctacttgatgggcagcgttaacttcata

SEQ ID NO: 309 - DNA, 53 bp, synthetic construct
  source 1..53: mol_type = other DNA
cttatcgccttcatcgtatgctagacaattttatcgtaatatatttcatcctc

SEQ ID NO: 310 - DNA, 42 bp, synthetic construct
  source 1..42: mol_type = other DNA
gtcaagcgatggcctacttgtatgcaatccacattactccag

SEQ ID NO: 311 - DNA, 42 bp, synthetic construct
  source 1..42: mol_type = other DNA
cttatcgccttcatcgtatgctattgattaccgacctgatcg

SEQ ID NO: 312 - DNA, 44 bp, synthetic construct
  source 1..44: mol_type = other DNA
gtcaagcgatggcctacttgatgtaccaggatcttattcgtaac

SEQ ID NO: 313 - DNA, 46 bp, synthetic construct
  source 1..46: mol_type = other DNA
cttatcgccttcatcgtatgttatttaaccatctctttttcgatca

SEQ ID NO: 314 - DNA, 39 bp, synthetic construct
  source 1..39: mol_type = other DNA
gtcaagcgatggcctacttggtggcaaagtttgtacccg

SEQ ID NO: 315 - DNA, 44 bp, synthetic construct
  source 1..44: mol_type = other DNA
cttatcgccttcatcgtatgttatttttgctgcttttttatcgc

SEQ ID NO: 316 - DNA, 40 bp, synthetic construct
  source 1..40: mol_type = other DNA
gtcaagcgatggcctacttgatgaaagtaaatctgccagc

SEQ ID NO: 317 - DNA, 39 bp, synthetic construct
  source 1..39: mol_type = other DNA
cttatcgccttcatcgtatgttacttctcgctctcggtc

SEQ ID NO: 318 - DNA, 40 bp, synthetic construct
  source 1..40: mol_type = other DNA
gtcaagcgatggcctacttgatgatcatcgttaccggcgg

SEQ ID NO: 319 - DNA, 40 bp, synthetic construct
  source 1..40: mol_type = other DNA
cttatcgccttcatcgtatgttacgcgtcgcggttcagcc

SEQ ID NO: 320 - DNA, 43 bp, synthetic construct
  source 1..43: mol_type = other DNA
gtcaagcgatggcctacttggtgattgataaatccgcctttat

SEQ ID NO: 321 - DNA, 40 bp, synthetic construct
  source 1..40: mol_type = other DNA
cttatcgccttcatcgtatgttaacgaatcggaccgcgcg

SEQ ID NO: 322 - DNA, 43 bp, synthetic construct
  source 1..43: mol_type = other DNA
gtcaagcgatggcctacttgtcattgtgctaactccaggacgg

SEQ ID NO: 323 - DNA, 40 bp, synthetic construct
  source 1..40: mol_type = other DNA
cttatcgccttcatcgtatgatggcggcacagcgtccttt

SEQ ID NO: 324 - DNA, 41 bp, synthetic construct
  source 1..41: mol_type = other DNA
gtcaagcgatggcctacttgatgatcaaacaaaggacactt

SEQ ID NO: 325 - DNA, 40 bp, synthetic construct
  source 1..40: mol_type = other DNA
cttatcgccttcatcgtatgttatgccagtaccgtcgaag

SEQ ID NO: 326 - DNA, 39 bp, synthetic construct
  source 1..39: mol_type = other DNA
gtcaagcgatggcctacttgatgccttcaattcgactgg

SEQ ID NO: 327 - DNA, 44 bp, synthetic construct
  source 1..44: mol_type = other DNA
cttatcgccttcatcgtatgttagtcttgttgattaaccttgcg

SEQ ID NO: 328 - DNA, 40 bp, synthetic construct
  source 1..40: mol_type = other DNA
gtcaagcgatggcctacttggtggcgacactgtttattgc

SEQ ID NO: 329 - DNA, 40 bp, synthetic construct
  source 1..40: mol_type = other DNA
cttatcgccttcatcgtatgttacagggggaaggcgatta

SEQ ID NO: 330 - DNA, 41 bp, synthetic construct
  source 1..41: mol_type = other DNA
gtcaagcgatggcctacttgatgattgcgcgtatctggtcg

SEQ ID NO: 331 - DNA, 40 bp, synthetic construct
  source 1..40: mol_type = other DNA
cttatcgccttcatcgtatgctagcgaaccagcgaggtga

SEQ ID NO: 332 - DNA, 40 bp, synthetic construct
  source 1..40: mol_type = other DNA
gtcaagcgatggcctacttgtcaatagcgcgacggtacgc

SEQ ID NO: 333 - DNA, 41 bp, synthetic construct
  source 1..41: mol_type = other DNA
cttatcgccttcatcgtatgatgacgaagttgcctaagttc

SEQ ID NO: 334 - DNA, 48 bp, synthetic construct
  source 1..48: mol_type = other DNA
gtcaagcgatggcctacttgatggaaaccaaaaaaaataatagtgagt

SEQ ID NO: 335 - DNA, 48 bp, synthetic construct
  source 1..48: mol_type = other DNA
cttatcgccttcatcgtatgttatttgatgggataaagatctttacgc

SEQ ID NO: 336 - DNA, 42 bp, synthetic construct
  source 1..42: mol_type = other DNA
gtcaagcgatggcctacttgatgttcgcagcaatcattatcg

SEQ ID NO: 337 - DNA, 40 bp, synthetic construct
  source 1..40: mol_type = other DNA
cttatcgccttcatcgtatgtcagaggaggctgaaaagga

SEQ ID NO: 338 - DNA, 44 bp, synthetic construct
  source 1..44: mol_type = other DNA
gtcaagcgatggcctacttgatgtttcctcaaagcaaattttca

SEQ ID NO: 339 - DNA, 40 bp, synthetic construct
  source 1..40: mol_type = other DNA
cttatcgccttcatcgtatgtcagatgtagagtgacgctt

SEQ ID NO: 340 - DNA, 40 bp, synthetic construct
  source 1..40: mol_type = other DNA
gtcaagcgatggcctacttgatgacgatgaaaacccgcta

SEQ ID NO: 341 - DNA, 50 bp, synthetic construct
  source 1..50: mol_type = other DNA
cttatcgccttcatcgtatgttatttgtttaaaatttgtttatttccgcc

SEQ ID NO: 342 - DNA, 41 bp, synthetic construct
  source 1..41: mol_type = other DNA
gtcaagcgatggcctacttgatgctcgaattgctttacacc

SEQ ID NO: 343 - DNA, 38 bp, synthetic construct
  source 1..38: mol_type = other DNA
cttatcgccttcatcgtatgtcaatgcgttttcggtgg

SEQ ID NO: 344 - DNA, 46 bp, synthetic construct
  source 1..46: mol_type = other DNA
gtcaagcgatggcctacttgatgatgaaatcgatacgctattatct

SEQ ID NO: 345 - DNA, 41 bp, synthetic construct
  source 1..41: mol_type = other DNA
cttatcgccttcatcgtatgtcatttaggccgatactgaat

SEQ ID NO: 346 - DNA, 42 bp, synthetic construct
  source 1..42: mol_type = other DNA
gtcaagcgatggcctacttgatgtatgttgcgatgatcatca

SEQ ID NO: 347 - DNA, 40 bp, synthetic construct
  source 1..40: mol_type = other DNA
cttatcgccttcatcgtatgtcaaaactggaaacgcatcc

SEQ ID NO: 348 - DNA, 44 bp, synthetic construct
  source 1..44: mol_type = other DNA
gtcaagcgatggcctacttgatgttaaagcgctttcttaaaaga

SEQ ID NO: 349 - DNA, 40 bp, synthetic construct
  source 1..40: mol_type = other DNA
cttatcgccttcatcgtatgtcattcgcttagtctcctgc

SEQ ID NO: 350 - DNA, 45 bp, synthetic construct
  source 1..45: mol_type = other DNA
gtcaagcgatggcctacttgatgagatacattaaatcgatgacgc

SEQ ID NO: 351 - DNA, 39 bp, synthetic construct
  source 1..39: mol_type = other DNA
cttatcgccttcatcgtatgctacttcgcggcgactttc

SEQ ID NO: 352 - DNA, 45 bp, synthetic construct
  source 1..45: mol_type = other DNA
gtcaagcgatggcctacttgatgaaacaaaaagtggttaacattg

SEQ ID NO: 353 - DNA, 39 bp, synthetic construct
  source 1..39: mol_type = other DNA
cttatcgccttcatcgtatgtcagttctcggtatccagc

SEQ ID NO: 354 - DNA, 41 bp, synthetic construct
  source 1..41: mol_type = other DNA
gtcaagcgatggcctacttgatgagtttcgtcgtcatcatt

SEQ ID NO: 355 - DNA, 38 bp, synthetic construct
  source 1..38: mol_type = other DNA
cttatcgccttcatcgtatgttaacgcatttcagcgcg

SEQ ID NO: 356 - DNA, 40 bp, synthetic construct
  source 1..40: mol_type = other DNA
gtcaagcgatggcctacttgatgagtaaagcaggtgcgtc

SEQ ID NO: 357 - DNA, 40 bp, synthetic construct
  source 1..40: mol_type = other DNA
cttatcgccttcatcgtatgtcatatcgattgccctttgg

SEQ ID NO: 358 - DNA, 39 bp, synthetic construct
  source 1..39: mol_type = other DNA
gtcaagcgatggcctacttgatgtcgcatttagcgttgc

SEQ ID NO: 359 - DNA, 38 bp, synthetic construct
  source 1..38: mol_type = other DNA
cttatcgccttcatcgtatgctacacgacgcctgcacg

SEQ ID NO: 360 - DNA, 43 bp, synthetic construct
  source 1..43: mol_type = other DNA
gtcaagcgatggcctacttgatgcataacgataaagatctctc

SEQ ID NO: 361 - DNA, 40 bp, synthetic construct
  source 1..40: mol_type = other DNA
cttatcgccttcatcgtatgtcattggccaaattgcatct

SEQ ID NO: 362 - DNA, 46 bp, synthetic construct
  source 1..46: mol_type = other DNA
gtcaagcgatggcctacttgatgcttataatttcatacattgcatt

SEQ ID NO: 363 - DNA, 50 bp, synthetic construct
  source 1..50: mol_type = other DNA
cttatcgccttcatcgtatgttatttattgtttcttagtaaaacgaatct

SEQ ID NO: 364 - DNA, 38 bp, synthetic construct
  source 1..38: mol_type = other DNA
gtcaagcgatggcctacttgatgtcgcttgctaaagcc

SEQ ID NO: 365 - DNA, 40 bp, synthetic construct
  source 1..40: mol_type = other DNA
cttatcgccttcatcgtatgtcatgctcgcctacgccaga

SEQ ID NO: 366 - DNA, 45 bp, synthetic construct
  source 1..45: mol_type = other DNA
gtcaagcgatggcctacttgatgaaattcaaaacaaacaaactca

SEQ ID NO: 367 - DNA, 41 bp, synthetic construct
  source 1..41: mol_type = other DNA
cttatcgccttcatcgtatgttagttactcttcttttgcgc

SEQ ID NO: 368 - DNA, 41 bp, synthetic construct
  source 1..41: mol_type = other DNA
gtcaagcgatggcctacttgatggcaacattaactgcaaag

SEQ ID NO: 369 - DNA, 40 bp, synthetic construct
  source 1..40: mol_type = other DNA
cttatcgccttcatcgtatgtcagagtctgaagtcttccc

SEQ ID NO: 370 - DNA, 41 bp, synthetic construct
  source 1..41: mol_type = other DNA
gtcaagcgatggcctacttgatgagtaaaaccagacgttgg

SEQ ID NO: 371 - DNA, 43 bp, synthetic construct
  source 1..43: mol_type = other DNA
cttatcgccttcatcgtatgttaaggctgagtttgtttgtttt

SEQ ID NO: 372 - DNA, 41 bp, synthetic construct
  source 1..41: mol_type = other DNA
gtcaagcgatggcctacttgttacatagagctttggtacgg

SEQ ID NO: 373 - DNA, 45 bp, synthetic construct
  source 1..45: mol_type = other DNA
cttatcgccttcatcgtatgatgaaaaaacgtattcccactcttc

SEQ ID NO: 374 - DNA, 40 bp, synthetic construct
  source 1..40: mol_type = other DNA
gtcaagcgatggcctacttgatgcagccatttggtgtact

SEQ ID NO: 375 - DNA, 41 bp, synthetic construct
  source 1..41: mol_type = other DNA
cttatcgccttcatcgtatgttacgacttacgcagcattag

SEQ ID NO: 376 - DNA, 76 bp, synthetic construct
  source 1..76: mol_type = other DNA
cataaacggctacctgtgccgccagccataattacgggaagaaaagacatctagtgccgatcatattcaataaccc

SEQ ID NO: 377 - DNA, 70 bp, synthetic construct
  source 1..70: mol_type = other DNA
ttgataatatgaagcagatggttggcaattggttggcggaatcaaaataacttatcgccttcatcgtatg

SEQ ID NO: 378 - DNA, 76 bp, synthetic construct
  source 1..76: mol_type = other DNA
cttatgattattgctttaaagatgcgtatggaaaaacggagagctattcactagtgccgatcatattcaataaccc

SEQ ID NO: 379 - DNA, 70 bp, synthetic construct
  source 1..70: mol_type = other DNA
ggccaaagcgaccctgcattatatgtgggaataattaatgttattttcatcttatcgccttcatcgtatg

SEQ ID NO: 380 - DNA, 76 bp, synthetic construct
  source 1..76: mol_type = other DNA
ttgggggcttccactaacttacttaattaaggcaaataagggataatcatctagtgccgatcatattcaataaccc

SEQ ID NO: 381 - DNA, 70 bp, synthetic construct
  source 1..70: mol_type = other DNA
gaatccagaaaggttaaatctacatttaatctcaatataataacttactacttatcgccttcatcgtatg

SEQ ID NO: 382 - DNA, 76 bp, synthetic construct
  source 1..76: mol_type = other DNA
tttatggctacactgtctccagcttcatcctttttttagttagggtatctctagtgccgatcatattcaataaccc

SEQ ID NO: 383 - DNA, 70 bp, synthetic construct
  source 1..70: mol_type = other DNA
ttaatgagaaattttacctgtcgtagccgaccaccatccggcaaagaagccttatcgccttcatcgtatg

SEQ ID NO: 384 - DNA, 76 bp, synthetic construct
  source 1..76: mol_type = other DNA
cttatttgcggatttttatattccagattcattgttttcaggaatgagaactagtgccgatcatattcaataaccc

SEQ ID NO: 385 - DNA, 70 bp, synthetic construct
  source 1..70: mol_type = other DNA
agccagtagtatcatcgccgttttcggtaatatcttgagcatagtgttcacttatcgccttcatcgtatg

SEQ ID NO: 386 - DNA, 76 bp, synthetic construct
  source 1..76: mol_type = other DNA
ctgatatgcggattcatttattcaaagttcattgtctttagggatgcgaactagtgccgatcatattcaataaccc

SEQ ID NO: 387 - DNA, 70 bp, synthetic construct
  source 1..70: mol_type = other DNA
acaccaacgagaaaactataaggatagcgattaccatttttaatctattgcttatcgccttcatcgtatg

SEQ ID NO: 388 - DNA, 76 bp, synthetic construct
  source 1..76: mol_type = other DNA
taatatgcctattttatttacattatgcacggtcagagggtgaggattaactagtgccgatcatattcaataaccc

SEQ ID NO: 389 - DNA, 70 bp, synthetic construct
  source 1..70: mol_type = other DNA
ttttacgcaggctaatttatacaattattattcagtacttctcggtaagccttatcgccttcatcgtatg

SEQ ID NO: 390 - DNA, 76 bp, synthetic construct
  source 1..76: mol_type = other DNA
gtaacgcattatactttaaggaaatgatatatgctgagagcacatacactctagtgccgatcatattcaataaccc

SEQ ID NO: 391 - DNA, 70 bp, synthetic construct
  source 1..70: mol_type = other DNA
agcgctcaccgcgcgtgcccccggtaatggttgtgtcatcgtatcctcatcttatcgccttcatcgtatg

SEQ ID NO: 392 - DNA, 76 bp, synthetic construct
  source 1..76: mol_type = other DNA
ctatttaatatctaaagtctttagattaaggttttaactctggggtatatctagtgccgatcatattcaataaccc

SEQ ID NO: 393 - DNA, 70 bp, synthetic construct
  source 1..70: mol_type = other DNA
taaagtctgttgaatgacttcttcttcaaaatattttctgctcatagtgacttatcgccttcatcgtatg

SEQ ID NO: 394 - DNA, 76 bp, synthetic construct
  source 1..76: mol_type = other DNA
cagcgggttctggaagagcttcattcgctgttgtcggaagagggcgtttactagtgccgatcatattcaataaccc

SEQ ID NO: 395 - DNA, 70 bp, synthetic construct
  source 1..70: mol_type = other DNA
gtggttagcatcttttctccacaataggtttgggatgagacagagtctctcttatcgccttcatcgtatg

SEQ ID NO: 396 - DNA, 76 bp, synthetic construct
  source 1..76: mol_type = other DNA
gccgaaggcgtcacggagtatatggcctggctgaaccgcgacgcgtaagtctagtgccgatcatattcaataaccc

SEQ ID NO: 397 - DNA, 70 bp, synthetic construct
  source 1..70: mol_type = other DNA
ggtatgtaatacgtcgcccatcgatgatgttttaacgatcaaaacccgcacttatcgccttcatcgtatg

SEQ ID NO: 398 - DNA, 76 bp, synthetic construct
  source 1..76: mol_type = other DNA
gaaaaaatgctgccgcatgaggcacgcaccatagatttggacagcctgctctagtgccgatcatattcaataaccc

SEQ ID NO: 399 - DNA, 70 bp, synthetic construct
  source 1..70: mol_type = other DNA
cctcaaaagcatctttaccgcgccatagtgtggttaacggcgctttcagccttatcgccttcatcgtatg

SEQ ID NO: 400 - DNA, 76 bp, synthetic construct
  source 1..76: mol_type = other DNA
agagccacagtataaaggcagggtaaattaaggtttttctggtaatcgttctagtgccgatcatattcaataaccc

SEQ ID NO: 401 - DNA, 70 bp, synthetic construct
  source 1..70: mol_type = other DNA
gcaccagtggcaaggctgggggaaaatcgccgcgcctaaaaacgtgagcgcttatcgccttcatcgtatg

SEQ ID NO: 402 - DNA, 76 bp, synthetic construct
  source 1..76: mol_type = other DNA
tttaaaaattttaataatgcaatattctcgaaattacaaaagtgatcactctagtgccgatcatattcaataaccc

SEQ ID NO: 403 - DNA, 70 bp, synthetic construct
  source 1..70: mol_type = other DNA
ttcagctatttctatctcaggaaatgaatccattacatcacctatgggttcttatcgccttcatcgtatg

SEQ ID NO: 404 - DNA, 76 bp, synthetic construct
  source 1..76: mol_type = other DNA
atagcctactttaaacgtaaacttcttgaataaaacccataggtgatgtactagtgccgatcatattcaataaccc

SEQ ID NO: 405 - DNA, 70 bp, synthetic construct
  source 1..70: mol_type = other DNA
agtttttaatctttttttcaataatcataatggagatttagggaggggaacttatcgccttcatcgtatg

SEQ ID NO: 406 - DNA, 76 bp, synthetic construct
  source 1..76: mol_type = other DNA
ttataacatttctttttctataaagttaactattctggattatagctattctagtgccgatcatattcaataaccc

SEQ ID NO: 407 - DNA, 70 bp, synthetic construct
  source 1..70: mol_type = other DNA
gcgctgatacttattacggtatcagcgcgttttccatcatcaggactcaacttatcgccttcatcgtatg

SEQ ID NO: 408 - DNA, 76 bp, synthetic construct
  source 1..76: mol_type = other DNA
agattcattaaagagactctgtctcatcccaaacctattgtggagaaaagctagtgccgatcatattcaataaccc

SEQ ID NO: 409 - DNA, 70 bp, synthetic construct
  source 1..70: mol_type = other DNA
cctgatgatggaaaacgcgctgataccgtaataagtatcagcgcgtttttcttatcgccttcatcgtatg

SEQ ID NO: 410 - DNA, 76 bp, synthetic construct
  source 1..76: mol_type = other DNA
tttatacagcttaccggagaaggccgcggatattattacaggtgatttagctagtgccgatcatattcaataaccc

SEQ ID NO: 411 - DNA, 70 bp, synthetic construct
  source 1..70: mol_type = other DNA
ctatccttgtctcactcataaattactcactgagtgcataattattataacttatcgccttcatcgtatg

SEQ ID NO: 412 - DNA, 76 bp, synthetic construct
  source 1..76: mol_type = other DNA
gtgcttttttctgcttatttatccggacaatttcaaccaaagagtcgcttctagtgccgatcatattcaataaccc

SEQ ID NO: 413 - DNA, 70 bp, synthetic construct
  source 1..70: mol_type = other DNA
acgctgcagaccgccaaaaggaaaatatttatataagcaaaaggcaactccttatcgccttcatcgtatg

SEQ ID NO: 414 - DNA, 76 bp, synthetic construct
  source 1..76: mol_type = other DNA
tctttatcgtaaacttttccacaaataattcccctccctaaatctccattctagtgccgatcatattcaataaccc

SEQ ID NO: 415 - DNA, 70 bp, synthetic construct
  source 1..70: mol_type = other DNA
caaataaaagtcagtcagccccttaaattaaaccaaacgtgctacattgacttatcgccttcatcgtatg

SEQ ID NO: 416 - DNA, 76 bp, synthetic construct
  source 1..76: mol_type = other DNA
ttgaatataacatttatttataggttgcatgataaacatacgagttttttctagtgccgatcatattcaataaccc

SEQ ID NO: 417 - DNA, 70 bp, synthetic construct
  source 1..70: mol_type = other DNA
aaaaaagaaatgcgtgccgaagcaacgaaaaataatgatttatctagtgtcttatcgccttcatcgtatg

SEQ ID NO: 418 - DNA, 76 bp, synthetic construct
  source 1..76: mol_type = other DNA
taaggttcaggcgttacgtttggcgctacgattaaagacaggctctcattctagtgccgatcatattcaataaccc

SEQ ID NO: 419 - DNA, 70 bp, synthetic construct
  source 1..70: mol_type = other DNA
agaagcacgccaggcccgataagcgttagcgttatcgggcaacatacaggcttatcgccttcatcgtatg

SEQ ID NO: 420 - DNA, 76 bp, synthetic construct
  source 1..76: mol_type = other DNA
atccggtacactgcatactgtcatttacattcatgctgaaggatatcctcctagtgccgatcatattcaataaccc

SEQ ID NO: 421 - DNA, 70 bp, synthetic construct
  source 1..70: mol_type = other DNA
gtttctgagcgcaaccaacgcacctgcagcttgaagtatgacgggtatagcttatcgccttcatcgtatg

SEQ ID NO: 422 - DNA, 76 bp, synthetic construct
  source 1..76: mol_type = other DNA
ctgaaacatgcgatactagcgccacttgctttactcaggagctataaaagctagtgccgatcatattcaataaccc

SEQ ID NO: 423 - DNA, 70 bp, synthetic construct
  source 1..70: mol_type = other DNA
agcggaaaaatgcatttttgttttaaccgctcatcttttatccataacgccttatcgccttcatcgtatg

SEQ ID NO: 424 - DNA, 76 bp, synthetic construct
  source 1..76: mol_type = other DNA
tgaattatgctattatcgcgcgcaaattttgaatctctcaggagacaggactagtgccgatcatattcaataaccc

SEQ ID NO: 425 - DNA, 70 bp, synthetic construct
  source 1..70: mol_type = other DNA
cgccttcaaaatcagcgcccgccgcgtctgtaacgcctgatgacgcggttcttatcgccttcatcgtatg

SEQ ID NO: 426 - DNA, 76 bp, synthetic construct
  source 1..76: mol_type = other DNA
gcattcatgtctgagacagtctctgacaccataattcaaaggttacagttctagtgccgatcatattcaataaccc

SEQ ID NO: 427 - DNA, 70 bp, synthetic construct
  source 1..70: mol_type = other DNA
catcatcatgtcgcccacccaggacgggccaatgaccaaaattttcataccttatcgccttcatcgtatg

SEQ ID NO: 428 - DNA, 76 bp, synthetic construct
  source 1..76: mol_type = other DNA
tcgtgtgcgaagcaaccatgatgtgtgctcgtagccgggaggcctgattcctagtgccgatcatattcaataaccc

SEQ ID NO: 429 - DNA, 70 bp, synthetic construct
  source 1..70: mol_type = other DNA
ggacgtttcaccggcgaccagggcaatcgttaaaggacgctgtgccgccacttatcgccttcatcgtatg

SEQ ID NO: 430 - DNA, 76 bp, synthetic construct
  source 1..76: mol_type = other DNA
aaggcgtttaccgagttctttgagcgttcaacgcgcggtccgattcgttactagtgccgatcatattcaataaccc

SEQ ID NO: 431 - DNA, 70 bp, synthetic construct
  source 1..70: mol_type = other DNA
cacttcatccacacccgccactaaatgggtgtgtggataaacaaattcgacttatcgccttcatcgtatg

SEQ ID NO: 432 - DNA, 76 bp, synthetic construct
  source 1..76: mol_type = other DNA
cgaatgtatagtacacttcggttggataggtaatttggcgagattatacgctagtgccgatcatattcaataaccc

SEQ ID NO: 433 - DNA, 70 bp, synthetic construct
  source 1..70: mol_type = other DNA
ggagagagtgccaggttaaccagtcgaattttatacgacagcgtatgtcgcttatcgccttcatcgtatg

SEQ ID NO: 434 - DNA, 76 bp, synthetic construct
  source 1..76: mol_type = other DNA
gcgatgtgaaagacatcaccgctgacgtactgaaacaggttaaataagtactagtgccgatcatattcaataaccc

SEQ ID NO: 435 - DNA, 70 bp, synthetic construct
  source 1..70: mol_type = other DNA
tcgtatgaatgtgacaggccggaaaagaatggcaactacaaggcggaacgcttatcgccttcatcgtatg

SEQ ID NO: 436 - DNA, 76 bp, synthetic construct
  source 1..76: mol_type = other DNA
gtaccaaaagaagacgtcatcattgaaaacgtgaccgtcagcgagtaatcctagtgccgatcatattcaataaccc

SEQ ID NO: 437 - DNA, 70 bp, synthetic construct
  source 1..70: mol_type = other DNA
ggcaaggaaaacggttgcgtgcgcgccgtaacggacgattcgacgaacatcttatcgccttcatcgtatg

SEQ ID NO: 438 - DNA, 76 bp, synthetic construct
  source 1..76: mol_type = other DNA
ctggcgcaacacggcgtttacgcccagctacataagatgcaatttggccactagtgccgatcatattcaataaccc

SEQ ID NO: 439 - DNA, 70 bp, synthetic construct
  source 1..70: mol_type = other DNA
atgacattcatgactccataaattcatcactgccgctgcattgggggacgcttatcgccttcatcgtatg

SEQ ID NO: 440 - DNA, 76 bp, synthetic construct
  source 1..76: mol_type = other DNA
caaaaagatgcgagaatacggggaattgttcgttgaaagacaggatagaactagtgccgatcatattcaataaccc

SEQ ID NO: 441 - DNA, 70 bp, synthetic construct
  source 1..70: mol_type = other DNA
ttttaaagctaaaagaggggaaaaattgcagcctgacggctgcaatcctgcttatcgccttcatcgtatg

SEQ ID NO: 442 - DNA, 76 bp, synthetic construct
  source 1..76: mol_type = other DNA
tcgctacactattcacaattccttttcgcgtcagcagaccctggaaaagcctagtgccgatcatattcaataaccc

SEQ ID NO: 443 - DNA, 70 bp, synthetic construct
  source 1..70: mol_type = other DNA
aggtagtacagggtttgtcagcataaagcctctcttacgagaggctttatcttatcgccttcatcgtatg

SEQ ID NO: 444 - DNA, 76 bp, synthetic construct
  source 1..76: mol_type = other DNA
ggttgcctgaaaatcccgggatgaggttttcttagaaggacagtgacgttctagtgccgatcatattcaataaccc

SEQ ID NO: 445 - DNA, 70 bp, synthetic construct
  source 1..70: mol_type = other DNA
cgccaggatagaacaggccgcggcaggcagttccataccgcggcccggctcttatcgccttcatcgtatg

SEQ ID NO: 446 - DNA, 76 bp, synthetic construct
  source 1..76: mol_type = other DNA
ataatgactcttctgcgatacattattttcgtatctacagaaggtattttctagtgccgatcatattcaataaccc

SEQ ID NO: 447 - DNA, 70 bp, synthetic construct
  source 1..70: mol_type = other DNA
gaatattatgacaatgcgaaatgccaaaataaaaggccttgcggccttttcttatcgccttcatcgtatg

SEQ ID NO: 448 - DNA, 76 bp, synthetic construct
  source 1..76: mol_type = other DNA
cgtttagcgacgcacgcgtaaggttgccaccgtttaaaaactatggcgaactagtgccgatcatattcaataaccc

SEQ ID NO: 449 - DNA, 70 bp, synthetic construct
  source 1..70: mol_type = other DNA
taccttcaacgatgtaaaactatcgctgaaggtaatgttaattacataggcttatcgccttcatcgtatg

SEQ ID NO: 450 - DNA, 76 bp, synthetic construct
  source 1..76: mol_type = other DNA
caggctaaatacatagaatccccagcacatccataagtcagctatttactctagtgccgatcatattcaataaccc

SEQ ID NO: 451 - DNA, 70 bp, synthetic construct
  source 1..70: mol_type = other DNA
aatcggatcaaacgtacctggataaatcgcccgtttttgcatgacagtcccttatcgccttcatcgtatg

SEQ ID NO: 452 - DNA, 76 bp, synthetic construct
  source 1..76: mol_type = other DNA
atccctggccgtgaaggttggctggggtgtcaacaggcagcgagcgcctcctagtgccgatcatattcaataaccc

SEQ ID NO: 453 - DNA, 70 bp, synthetic construct
  source 1..70: mol_type = other DNA
gagctgaccgccaacgctgagcagactggcaagcaccagaacgacgccgacttatcgccttcatcgtatg

SEQ ID NO: 454 - DNA, 76 bp, synthetic construct
  source 1..76: mol_type = other DNA
attttattcaggttaatgttgttattatcacagtcgaatttttgaacggtctagtgccgatcatattcaataaccc

SEQ ID NO: 455 - DNA, 70 bp, synthetic construct
  source 1..70: mol_type = other DNA
tattgttttttaagactttttaattcacaactgaagcatacccttccccacttatcgccttcatcgtatg

SEQ ID NO: 456 - DNA, 76 bp, synthetic construct
  source 1..76: mol_type = other DNA
taattttactttgtcacgattagcgtcaccgaatcgatggacgcatcaacctagtgccgatcatattcaataaccc

SEQ ID NO: 457 - DNA, 70 bp, synthetic construct
  source 1..70: mol_type = other DNA
gagtattaacccctgtaataatagcgtgtcgtcttcaacaatcagtatctcttatcgccttcatcgtatg

SEQ ID NO: 458 - DNA, 76 bp, synthetic construct
  source 1..76: mol_type = other DNA
aagaatcgttgtacaggtcgtttttatcccgattcccagggtttgtttgcctagtgccgatcatattcaataaccc

SEQ ID NO: 459 - DNA, 70 bp, synthetic construct
  source 1..70: mol_type = other DNA
tcccttagtcgcaaaatacaattcaatcggcgagaaagtcggcagacaaccttatcgccttcatcgtatg

SEQ ID NO: 460 - DNA, 76 bp, synthetic construct
  source 1..76: mol_type = other DNA
tgttctacattaattaaccgacattttacctataagtgtaaggcgatcctctagtgccgatcatattcaataaccc

SEQ ID NO: 461 - DNA, 70 bp, synthetic construct
  source 1..70: mol_type = other DNA
aaaaaagccggatagtatcttatccggcctacacaagctaaaaaccgcaacttatcgccttcatcgtatg

SEQ ID NO: 462 - DNA, 76 bp, synthetic construct
  source 1..76: mol_type = other DNA
gtattgctggaaaatgaagctcgcgccctgacatctgatgagagtaaatcctagtgccgatcatattcaataaccc

SEQ ID NO: 463 - DNA, 70 bp, synthetic construct
  source 1..70: mol_type = other DNA
tcataccgcgctgttcatgaccgtctaagacgatcatgaacaggatcatgcttatcgccttcatcgtatg

SEQ ID NO: 464 - DNA, 76 bp, synthetic construct
  source 1..76: mol_type = other DNA
catgatctcctgcgtgcaggcgtcgtgtagaaactcaaggataattaacgctagtgccgatcatattcaataaccc

SEQ ID NO: 465 - DNA, 70 bp, synthetic construct
  source 1..70: mol_type = other DNA
taccagaatggccagcgacagtagaatgataacccaacgtctggttttaccttatcgccttcatcgtatg

SEQ ID NO: 466 - DNA, 76 bp, synthetic construct
  source 1..76: mol_type = other DNA
gatgctctattggctatcgccacttcttgttggataactggaaacggattctagtgccgatcatattcaataaccc

SEQ ID NO: 467 - DNA, 70 bp, synthetic construct
  source 1..70: mol_type = other DNA
ggtcggaagcgacgcacctgctttactcatcgttaattatccttgagtttcttatcgccttcatcgtatg

SEQ ID NO: 468 - DNA, 76 bp, synthetic construct
  source 1..76: mol_type = other DNA
aggataacgggtagaatatgcggctatttcaacaaatgctggttttttgactagtgccgatcatattcaataaccc

SEQ ID NO: 469 - DNA, 70 bp, synthetic construct
  source 1..70: mol_type = other DNA
cggcagcagtaaccgccatagcggggattcacccgaccagatacgcgcaacttatcgccttcatcgtatg

SEQ ID NO: 470 - DNA, 76 bp, synthetic construct
  source 1..76: mol_type = other DNA
tgcctgatggtaatatttttaatactaagcattttttctaaaggctctatctagtgccgatcatattcaataaccc

SEQ ID NO: 471 - DNA, 70 bp, synthetic construct
  source 1..70: mol_type = other DNA
atttttacgcttcagagccaaataaaacggcggcattgccgccgtataaccttatcgccttcatcgtatg

SEQ ID NO: 472 - DNA, 76 bp, synthetic construct
  source 1..76: mol_type = other DNA
cgtcgatcaacgaacggtgattactaccttgctaaattatttctcctgatctagtgccgatcatattcaataaccc

SEQ ID NO: 473 - DNA, 70 bp, synthetic construct
  source 1..70: mol_type = other DNA
ggtgtggttatggtgagggatatccgatcccaggacgtgaatcagtacagcttatcgccttcatcgtatg

SEQ ID NO: 474 - DNA, 76 bp, synthetic construct
  source 1..76: mol_type = other DNA
taacttacgcagcaagaacgccgagctgattgaaaaggttagaacctcttctagtgccgatcatattcaataaccc

SEQ ID NO: 475 - DNA, 70 bp, synthetic construct
  source 1..70: mol_type = other DNA
cctttataggccttcgccagattctttgcagttaatgttgccataacgaacttatcgccttcatcgtatg

SEQ ID NO: 476 - DNA, 76 bp, synthetic construct
  source 1..76: mol_type = other DNA
acaaaaacaaaggccagactccggcgcaaaagaagagtaactaattcgttctagtgccgatcatattcaataaccc

SEQ ID NO: 477 - DNA, 70 bp, synthetic construct
  source 1..70: mol_type = other DNA
catattcagagtcgttttctcccgctagagcagcatagccctctaccctacttatcgccttcatcgtatg

SEQ ID NO: 478 - DNA, 76 bp, synthetic construct
  source 1..76: mol_type = other DNA
ttgctgctgctggcgcagggcaagctggatgaggccaaagggcaatcgatctagtgccgatcatattcaataaccc

SEQ ID NO: 479 - DNA, 70 bp, synthetic construct
  source 1..70: mol_type = other DNA
cggcgaaagccggaatgctggcggccagcagcgagccggcaagcataagacttatcgccttcatcgtatg

SEQ ID NO: 480 - DNA, 76 bp, synthetic construct
  source 1..76: mol_type = other DNA
accgtttgtcacgcgcaacgctaccgatgatggaacaataaatacaacgtctagtgccgatcatattcaataaccc

SEQ ID NO: 481 - DNA, 70 bp, synthetic construct
  source 1..70: mol_type = other DNA
ttttccatttcaattaaccgcaatgcggattacgttgtaaatcaatcagacttatcgccttcatcgtatg

SEQ ID NO: 482 - DNA, 76 bp, synthetic construct
  source 1..76: mol_type = other DNA
gtgccggtccgccgcctgcgtgcccgttttctgcgtaaaggagcggtatactagtgccgatcatattcaataaccc

SEQ ID NO: 483 - DNA, 70 bp, synthetic construct
  source 1..70: mol_type = other DNA
tcatggtaggcctgataagcgcagcgccatcaggcctacgattactgtgacttatcgccttcatcgtatg